European Patent Specification EP 3 827 015 B1, published February 18, 2026. Title: GIP/GLP1 CO-AGONIST COMPOUNDS. Applicant: Eli Lilly and Company. The sequence listing filed with the application follows.

SEQUENCE LISTING (396 sequences)

SEQ ID NO: 1 - protein, 42 aa, Homo sapiens
YAEGTFISDYSIAMDKIHQQDFVNWLLAQKGKKNDWKHNITQ

SEQ ID NO: 2 - protein, 30 aa, Homo sapiens
  MOD_RES (30)..(30): AMIDATION
HAEGTFTSDVSSYLEGQAAKEFIAWLVKGR

SEQ ID NO: 3 - protein, 31 aa, Artificial Sequence
  Synthetic construct; Formula I
  VARIANT (1)..(1): Xaa at position 1 is selected from the group consisting of Y, H, D-Tyr, F, desH, and desY, or Xaa at position 1 and Xaa at position 2 combine to form desH-psi[NHCO]-Aib
  MOD_RES (1)..(1): The N-terminus of Xaa at position 1 is modified with R1, wherein the modification is selected from the group consisting of Ac and absent.
  VARIANT (2)..(2): Xaa at position 2 is selected from the group consisting of Aib, alpha-MeP, A, P, and D-Ala, or Xaa at position 1 combines with Xaa at position 2 to form desH-psi[NHCO]-Aib
  VARIANT (3)..(3): Xaa at position 3 is selected from the group of E, N, Aad, and cTA
  VARIANT (6)..(6): Xaa at position 6 is selected from the group consisting of F, alpha-MeF, and alpha-MeF(2F)
  VARIANT (10)..(10): Xaa at position 10 is selected from the group consisting of A, L, H, 3Pal, 4Pal, V, Y, E, alpha-MeF, alpha-MeF(2F), I, alpha-MeY, Q, D-His, D-Tyr, cTA, and K
  VARIANT (10)..(10): when Xaa at position 10 is K, then K is chemically modified by conjugation of the epsilon-amino group of the K side chain with (2-[2-(2-amino-ethoxy)-ethoxy]-acetyl)2-(gamma-Glu)-CO-(CH2)q-CO2 H
  MISC_FEATURE (10)..(31): When Xaa is K(2-[2-(2-amino-ethoxy)-ethoxy]-acetyl)2-(gamma-Glu)-CO-(CH2)q-CO 2H at positions 10, 12, 13, 14, 16, 17, 19, 20, 21, 23, 24, 26, 27, 28, 29, 30 or 31, q is 14, 15, 16, 17, 18, 19 or 20.
  VARIANT (11)..(11): Xaa at position 11 is selected from the group consisting of S, alpha-MeS, or D-Ser
  VARIANT (12)..(12): Xaa at position 12 is selected from the group consisting of I, S, D-Ile, and K
  MOD_RES (12)..(12): when Xaa at position 12 is K, then K is chemically modified by conjugation of the epsilon-amino group of the K side chain with (2-[2-(2-amino-ethoxy)-ethoxy]-acetyl)2-(gamma-Glu)-CO-(CH2)q-CO2 H
  VARIANT (13)..(13): Xaa at position 13 is selected from the group consisting of Nle, Aib, L, alpha-MeL, and K
  MOD_RES (13)..(13): when Xaa at position 13 is K, then K is chemically modified by conjugation of the epsilon-amino group of the K side chain with (2-[2-(2-amino-ethoxy)-ethoxy]-acetyl)2-(gamma-Glu)-CO-(CH2)q-CO2 H
  VARIANT (14)..(14): Xaa at position 14 is selected from the group consisting of L and K, wherein K is conjugated to a C16-C22 fatty acid wherein said fatty acid is optionally conjugated to said K via a linker
  VARIANT (16)..(16): Xaa at position 16 is selected from the group consisting of E, Orn, Dab, Dap, S, T, H, Aib, alpha-MeK, R, and K
  MOD_RES (16)..(16): when Xaa at position 16 is K, then K is optionally chemically modified by conjugation of the epsilon-amino group of the K side chain with (2-[2-(2-amino-ethoxy)-ethoxy]-acetyl)2 -(gamma-Glu)-CO-(CH2)q-CO2H
  VARIANT (17)..(17): Xaa at position 17 is selected from the group consisting of K, Q, I, and an amino acid conjugated to a C16-C22 fatty acid wherein said fatty acid is optionally conjugated to said amino acid via a linker
  VARIANT (19)..(19): Xaa at position 19 is selected from the group consisting of Q, A, and K
  MOD_RES (19)..(19): when Xaa at position 19 is K, then K is chemically modified by conjugation of the epsilon-amino group of the K side chain with (2-[2-(2-amino-ethoxy)-ethoxy]-acetyl)2 -(gamma-Glu)-CO-(CH2)q-CO2H
  VARIANT (20)..(20): Xaa at position 20 is selected from the group consisting of Aib, Q, H, R, K, and alpha-MeK
  MOD_RES (20)..(20): when Xaa at position 20 is K, then K  is optionally chemically modified by conjugation of the epsilon-amino group of the K side chain with (2-[2-(2-amino-ethoxy)-ethoxy]-acetyl)2 -(gamma-Glu)-CO-(CH2)q-CO2H
  VARIANT (21)..(21): Xaa at position 21 is selected from the group consisting of H, Aad, D, Aib, T, A, E, I, and K
  MOD_RES (21)..(21): when Xaa at position 21 is K, then K is chemically modified by conjugation of the epsilon-amino group of the K side chain with K(2-[2-(2-amino-ethoxy)-ethoxy]-acetyl)2-(gamma-Glu)-CO-(CH2)q-CO 2H
  VARIANT (22)..(22): Xaa at position 22 is selected from the group consisting of F and alpha-MeF
  VARIANT (23)..(23): Xaa at position 23 is selected from the group consisting of I, L, A, G, F, H, E, V, and  K
  MOD_RES (23)..(23): when Xaa at position 23 is K, then K is chemically modified by conjugation of the epsilon-amino group of the K side chain with K(2-[2-(2-amino-ethoxy)-ethoxy]-acetyl)2-(gamma-Glu)-CO-(CH2)q-CO 2H
  VARIANT (24)..(24): Xaa at position 24 is selected from the group consisting of S, Aad, D-Glu, E, Aib, H, V, A, Q, D, P, and K
  MOD_RES (24)..(24): when Xaa at position 24 is K, then K is chemically modified by conjugation of the epsilon-amino group of the K side chain with K(2-[2-(2-amino-ethoxy)-ethoxy]-acetyl)2-(gamma-Glu)-CO-(CH2)q-CO 2H
  VARIANT (25)..(25): Xaa at position 25 is selected from the group consisting of Y or alpha-MeY
  VARIANT (26)..(26): Xaa at position 26 is selected from the group consisting of L, alpha-MeL, and K
  MOD_RES (26)..(26): when Xaa at position 26 is K, then K is chemically modified by conjugation of the epsilon-amino group of the K side chain with (2-[2-(2-amino-ethoxy)-ethoxy]-acetyl)2-(gamma-Glu)-CO-(CH2)q-CO2 H
  VARIANT (27)..(27): Xaa at position 27 is selected from the group consisting of L, I, and K
  MOD_RES (27)..(27): when Xaa at position 27 is K, then K is chemically modified by conjugation of the epsilon-amino group of the K side chain with (2-[2-(2-amino-ethoxy)-ethoxy]-acetyl)2-(gamma-Glu)-CO-(CH2)q-CO2 H
  VARIANT (28)..(28): Xaa at position 28 is selected from the group consisting of E, A, S, D-Glu, and K
  MOD_RES (28)..(28): when Xaa at position 28 is K, then K is chemically modified by conjugation of the epsilon-amino group of the K side chain with (2-[2-(2-amino-ethoxy)-ethoxy]-acetyl)2-(gamma-Glu)-CO-(CH2)q-CO2 H
  VARIANT (29)..(29): Xaa at position 29 is selected from the group consisting of Aib, G, A, and K
  MOD_RES (29)..(29): when Xaa at position 29 is K, then K is chemically modified by conjugation of the epsilon-amino group of the K side chain with (2-[2-(2-amino-ethoxy)-ethoxy]-acetyl)2-(gamma-Glu)-CO-(CH2)q-CO2 H
  VARIANT (30)..(30): Xaa at position 30 is selected from the group consisting of C, G, G-R2, and K, wherein R2 is a modification of the C-terminal group, wherein the modification is NH2 or absent, wherein if X30 is G-R2, then X31 is absent.
  MOD_RES (30)..(30): when Xaa at position 30 is K, then K is chemically modified by conjugation of the epsilon-amino group of the K side chain with (2-[2-(2-amino-ethoxy)-ethoxy]-acetyl)2-(gamma-Glu)-CO-(CH2)q-CO2 H
  VARIANT (31)..(31): Xaa at position 31 is absent or is selected from the group consisting of SEQ ID NO:4, SEQ ID NO:5, SEQ ID:6, SEQ ID NO:7, SEQ ID NO:8, and SEQ ID NO:9
  MISC_FEATURE (31)..(31): wherein no more than one of X10, X12, X13, X14, X16, X17, X19, X20, X21, X23, X24, X26, X27, X28, X29, X30, X31, X32, X33, X34, X35, X36, X37, X38, X39, and X40 may be a substituent that contains a fatty acid
  MISC_FEATURE (31)..(31): wherein no more than one of X30, X34, X39, and X40 may be C
  MISC_FEATURE (31)..(31): wherein if one of X30, X34, X39, and X40 is C, then none of X10, X12, X13, X14, X16, X17, X19, X20, X21, X23, X24, X26, X27, X28, X29, X30, X31, X32, X33, X34, X35, X36, X37, X38, X39, and X40 is a substituent that contains a fatty acid
  MOD_RES (31)..(31): Xaa at position 31 is modified with R2, wherein the modification is NH2 to form a C-terminal amide or absent
XXXGTXTSDXXXXXDXXAXXXXXXXXXXXXX

SEQ ID NO: 4 - protein, 4 aa, Artificial Sequence
  Synthetic construct; SEQ ID NO:4 is PX32X33X34
  VARIANT (2)..(2): Xaa at position 2 is S or K, wherein K is chemically modified by conjugation of the epsilon-amino group of the K side chain with (2-[2-(2-amino-ethoxy)-ethoxy]-acetyl)2-(gamma-Glu)-CO-(CH2)q-CO2 H
  MISC_FEATURE (2)..(4): wherein q is selected from the group consisting of 14, 15, 16, 17, 18, 19, and 20.
  VARIANT (3)..(3): Xaa at position 3 is S or K, wherein K is chemically modified by conjugation of the epsilon-amino group of the K side chain with (2-[2-(2-amino-ethoxy)-ethoxy]-acetyl)2-(gamma-Glu)-CO-(CH2)q-CO2 H
  VARIANT (4)..(4): Xaa at position 4 is G, C or K, wherein K is chemically modified by conjugation of the epsilon-amino group of the K side chain with (2-[2-(2-amino-ethoxy)-ethoxy]-acetyl)2 -(gamma-Glu)-CO-(CH2)q-CO2H
  MOD_RES (4)..(4): The C-terminal group of Xaa at position 4 is modified with R2, wherein the modification is NH2 to form a C-terminal amide or absent
PXXX

SEQ ID NO: 5 - protein, 9 aa, Artificial Sequence
  Synthetic Construct; SEQ ID NO:5 is PX32X33X34X35X36X37X38X39
  VARIANT (2)..(2): Xaa at position 2 is S or K, wherein K is chemically modified by conjugation of the epsilon-amino group of the K side chain with (2-[2-(2-amino-ethoxy)-ethoxy]-acetyl)2-(gamma-Glu)-CO-(CH2)q-CO2 H
  MISC_FEATURE (2)..(9): wherein q is selected from the group consisting of 14, 15, 16, 17, 18, 19, and 20.
  VARIANT (3)..(3): Xaa at position 3 is S or K, wherein K is chemically modified by conjugation of the epsilon-amino group of the K side chain with (2-[2-(2-amino-ethoxy)-ethoxy]-acetyl)2-(gamma-Glu)-CO-(CH2)q-CO2 H
  VARIANT (4)..(4): Xaa at position 4 is G, C or K, wherein K is chemically modified by conjugation of the epsilon-amino group of the K side chain with (2-[2-(2-amino-ethoxy)-ethoxy]-acetyl)2 -(gamma-Glu)-CO-(CH2)q-CO2H
  VARIANT (5)..(5): Xaa at position 5 is A or K, wherein K is chemically modified by conjugation of the epsilon-amino group of the K side chain with (2-[2-(2-amino-ethoxy)-ethoxy]-acetyl)2-(gamma-Glu)-CO-(CH2)q-CO2 H
  VARIANT (6)..(6): Xaa at position 6 is P or K, wherein K is chemically modified by conjugation of the epsilon-amino group of the K side chain with (2-[2-(2-amino-ethoxy)-ethoxy]-acetyl)2-(gamma-Glu)-CO-(CH2)q-CO2 H
  VARIANT (7)..(7): Xaa at position 7 is P or K, wherein K is chemically modified by conjugation of the epsilon-amino group of the K side chain with (2-[2-(2-amino-ethoxy)-ethoxy]-acetyl)2-(gamma-Glu)-CO-(CH2)q-CO2 H
  VARIANT (8)..(8): Xaa at position 8 is P or K, wherein K is chemically modified by conjugation of the epsilon-amino group of the K side chain with (2-[2-(2-amino-ethoxy)-ethoxy]-acetyl)2-(gamma-Glu)-CO-(CH2)q-CO2 H
  VARIANT (9)..(9): Xaa at position 9 is C, S or K, wherein K is chemically modified by conjugation of the epsilon-amino group of the K side chain with (2-[2-(2-amino-ethoxy)-ethoxy]-acetyl)2 -(gamma-Glu)-CO-(CH2)q-CO2H
  MOD_RES (9)..(9): The C-terminal group of Xaa at position 9 is modified with R2, wherein the modification is NH2 to from a C-terminal amide or absent
PXXXXXXXX

SEQ ID NO: 6 - protein, 10 aa, Artificial Sequence
  Synthetic Construct; SEQ ID NO:6 is PX32X33X34X35X36X37X38X39X40
  VARIANT (2)..(2): Xaa at position 2 is S or K, wherein K is chemically modified by conjugation of the epsilon-amino group of the K side chain with (2-[2-(2-amino-ethoxy)-ethoxy]-acetyl)2-(gamma-Glu)-CO-(CH2)q-CO2 H
  MISC_FEATURE (2)..(10): wherein q is selected from the group consisting of 14, 15, 16, 17, 18, 19, and 20.
  VARIANT (3)..(3): Xaa at position 3 is S or K, wherein K is chemically modified by conjugation of the epsilon-amino group of the K side chain with (2-[2-(2-amino-ethoxy)-ethoxy]-acetyl)2-(gamma-Glu)-CO-(CH2)q-CO2 H
  VARIANT (4)..(4): Xaa at position 4 is G, C or K, wherein K is chemically modified by conjugation of the epsilon-amino group of the K side chain with (2-[2-(2-amino-ethoxy)-ethoxy]-acetyl)2 -(gamma-Glu)-CO-(CH2)q-CO2H
  VARIANT (5)..(5): Xaa at position 5 is A or K, wherein K is chemically modified by conjugation of the epsilon-amino group of the K side chain with (2-[2-(2-amino-ethoxy)-ethoxy]-acetyl)2-(gamma-Glu)-CO-(CH2)q-CO2 H
  VARIANT (6)..(6): Xaa at position 6 is P or K, wherein K is chemically modified by conjugation of the epsilon-amino group of the K side chain with (2-[2-(2-amino-ethoxy)-ethoxy]-acetyl)2-(gamma-Glu)-CO-(CH2)q-CO2 H
  VARIANT (7)..(7): Xaa at position 7 is P or K, wherein K is chemically modified by conjugation of the epsilon-amino group of the K side chain with K(2-[2-(2-amino-ethoxy)-ethoxy]-acetyl)2-(gamma-Glu)-CO-(CH2)q-CO 2H
  VARIANT (8)..(8): Xaa at position 8 is P or K, wherein K is chemically modified by conjugation of the epsilon-amino group of the K side chain with K(2-[2-(2-amino-ethoxy)-ethoxy]-acetyl)2-(gamma-Glu)-CO-(CH2)q-CO 2H
  VARIANT (9)..(9): Xaa at position 9 is C, S or K, wherein K is chemically modified by conjugation of the epsilon-amino group of the K side chain with (2-[2-(2-amino-ethoxy)-ethoxy]-acetyl)2 -(gamma-Glu)-CO-(CH2)q-CO2H
  VARIANT (10)..(10): Xaa at position 10 is C or K, wherein K is chemically modified by conjugation of the epsilon-amino group of the K side chain with (2-[2-(2-amino-ethoxy)-ethoxy]-acetyl)2-(gamma-Glu)-CO-(CH2)q-CO2 H
  MOD_RES (10)..(10): The C-terminal group of Xaa at position 10 is modified with R2, wherein the modification is NH2 to form a C-terminal amide or absent
PXXXXXXXXX

SEQ ID NO: 7 - protein, 4 aa, Artificial Sequence
  Synthetic Construct; SEQ ID NO:7 is K[(2-[2-(2-amino-ethoxy)-ethoxy]-acetyl)2-(gamma-Glu)-CO-(CH2)q-C O2 H]X32X33X34
  MOD_RES (1)..(1): K is chemically modified by conjugation of the epsilon-amino group of the K side chain with (2-[2-(2-amino-ethoxy)-ethoxy]-acetyl)2-(gamma-Glu)-CO-(CH2)q-CO2 H
  MISC_FEATURE (1)..(1): wherein q is selected from the group consisting of 14, 15, 16, 17, 18, 19, and 20
  VARIANT (2)..(2): Xaa at position 2 is S or K, wherein K is chemically modified by conjugation of the epsilon-amino group of the K side chain with (2-[2-(2-amino-ethoxy)-ethoxy]-acetyl)2-(gamma-Glu)-CO-(CH2)q-CO2 H
  VARIANT (3)..(3): Xaa at position 3 is S or K, wherein K is chemically modified by conjugation of the epsilon-amino group of the K side chain with (2-[2-(2-amino-ethoxy)-ethoxy]-acetyl)2-(gamma-Glu)-CO-(CH2)q-CO2 H
  VARIANT (4)..(4): Xaa at position 4 is G, C or K, wherein K is chemically modified by conjugation of the epsilon-amino group of the K side chain with (2-[2-(2-amino-ethoxy)-ethoxy]-acetyl)2 -(gamma-Glu)-CO-(CH2)q-CO2H
  MOD_RES (4)..(4): The C-terminal group of Xaa at position 4 is modified with R2, wherein the modification is NH2 to form a C-terminal amide or absent
KXXX

SEQ ID NO: 8 - protein, 9 aa, Artificial Sequence
  Synthetic Construct; SEQ ID NO:8 is K[(2-[2-(2-amino-ethoxy)-ethoxy]-acetyl)2-(gamma-Glu)-CO-(CH2)q-C O2H]X32X33X34X35X36X37X38X39
  MOD_RES (1)..(1): K is chemically modified by conjugation of the epsilon-amino group of the K side chain with (2-[2-(2-amino-ethoxy)-ethoxy]-acetyl)2-(gamma-Glu)-CO-(CH2)q-CO2 H
  MISC_FEATURE (1)..(1): wherein q is selected from the group consisting of 14, 15, 16, 17, 18, 19, and 20
  VARIANT (2)..(2): Xaa at position 2 is S or K, wherein K is chemically modified by conjugation of the epsilon-amino group of the K side chain with (2-[2-(2-amino-ethoxy)-ethoxy]-acetyl)2-(gamma-Glu)-CO-(CH2)q-CO2 H
  VARIANT (3)..(3): Xaa at position 3 is S or K, wherein K is chemically modified by conjugation of the epsilon-amino group of the K side chain with (2-[2-(2-amino-ethoxy)-ethoxy]-acetyl)2-(gamma-Glu)-CO-(CH2)q-CO2 H
  VARIANT (4)..(4): Xaa at position 4 is G, C or K, wherein K is chemically modified by conjugation of the epsilon-amino group of the K side chain with (2-[2-(2-amino-ethoxy)-ethoxy]-acetyl)2 -(gamma-Glu)-CO-(CH2)q-CO2H
  VARIANT (5)..(5): Xaa at position 5 is A or K, wherein K is chemically modified by conjugation of the epsilon-amino group of the K side chain with (2-[2-(2-amino-ethoxy)-ethoxy]-acetyl)2-(gamma-Glu)-CO-(CH2)q-CO2 H
  VARIANT (6)..(6): Xaa at position 6 is P or K, wherein K is chemically modified by conjugation of the epsilon-amino group of the K side chain with (2-[2-(2-amino-ethoxy)-ethoxy]-acetyl)2-(gamma-Glu)-CO-(CH2)q-CO2 H
  VARIANT (7)..(7): Xaa at position 7 is P or K, wherein K is chemically modified by conjugation of the epsilon-amino group of the K side chain with (2-[2-(2-amino-ethoxy)-ethoxy]-acetyl)2-(gamma-Glu)-CO-(CH2)q-CO2 H
  VARIANT (8)..(8): Xaa at position 8 is P or K, wherein K is chemically modified by conjugation of the epsilon-amino group of the K side chain with (2-[2-(2-amino-ethoxy)-ethoxy]-acetyl)2-(gamma-Glu)-CO-(CH2)q-CO2 H
  VARIANT (9)..(9): Xaa at position 9 is C, S or K, wherein K is chemically modified by conjugation of the epsilon-amino group of the K side chain with (2-[2-(2-amino-ethoxy)-ethoxy]-acetyl)2-(gamma-Glu)-CO-(CH2)q-CO2
  MOD_RES (9)..(9): The C-terminal group of Xaa at position 9 is modified with R2, wherein the modification is NH2 to form a C-terminal amide or absent
KXXXXXXXX

SEQ ID NO: 9 - protein, 10 aa, Artificial Sequence
  Synthetic Construct; SEQ ID NO:9 is K[(2-[2-(2-amino-ethoxy)-ethoxy]-acetyl)2-(gamma-Glu)-CO-(CH2)q-C O2H]X32X33X34X35X36X37X38X39X40
  MOD_RES (1)..(1): K is chemically modified by conjugation of the epsilon-amino group of the K side chain with (2-[2-(2-amino-ethoxy)-ethoxy]-acetyl)2-(gamma-Glu)-CO-(CH2)q-CO2 H
  MISC_FEATURE (1)..(1): wherein q is selected from the group consisting of 14, 15, 16, 17, 18, 19, and 20
  VARIANT (2)..(2): Xaa at position 2 is S or K, wherein K is chemically modified by conjugation of the epsilon-amino group of the K side chain with (2-[2-(2-amino-ethoxy)-ethoxy]-acetyl)2-(gamma-Glu)-CO-(CH2)q-CO2 H
  VARIANT (3)..(3): Xaa at position 3 is S or K, wherein K is chemically modified by conjugation of the epsilon-amino group of the K side chain with (2-[2-(2-amino-ethoxy)-ethoxy]-acetyl)2-(gamma-Glu)-CO-(CH2)q-CO2 H
  VARIANT (4)..(4): Xaa at position 4 is G, C or K, wherein K is chemically modified by conjugation of the epsilon-amino group of the K side chain with (2-[2-(2-amino-ethoxy)-ethoxy]-acetyl)2 -(gamma-Glu)-CO-(CH2)q-CO2H
  VARIANT (5)..(5): Xaa at position 5 is A or K, wherein K is chemically modified by conjugation of the epsilon-amino group of the K side chain with (2-[2-(2-amino-ethoxy)-ethoxy]-acetyl)2-(gamma-Glu)-CO-(CH2)q-CO2 H
  VARIANT (6)..(6): Xaa at position 6 is P or K, wherein K is chemically modified by conjugation of the epsilon-amino group of the K side chain with (2-[2-(2-amino-ethoxy)-ethoxy]-acetyl)2-(gamma-Glu)-CO-(CH2)q-CO2 H
  VARIANT (7)..(7): Xaa at position 7 is P or K, wherein K is chemically modified by conjugation of the epsilon-amino group of the K side chain with (2-[2-(2-amino-ethoxy)-ethoxy]-acetyl)2-(gamma-Glu)-CO-(CH2)q-CO2 H
  VARIANT (8)..(8): Xaa at position 8 is P or K, wherein K is chemically modified by conjugation of the epsilon-amino group of the K side chain with (2-[2-(2-amino-ethoxy)-ethoxy]-acetyl)2-(gamma-Glu)-CO-(CH2)q-CO2 H
  VARIANT (9)..(9): Xaa at position 9 is C, S or K, wherein K is chemically modified by conjugation of the epsilon-amino group of the K side chain with (2-[2-(2-amino-ethoxy)-ethoxy]-acetyl)2 -(gamma-Glu)-CO-(CH2)q-CO2H
  VARIANT (10)..(10): Xaa at position 10 is C or K, wherein K is chemically modified by conjugation of the epsilon-amino group of the K side chain with (2-[2-(2-amino-ethoxy)-ethoxy]-acetyl)2 -(gamma-Glu)-CO-(CH2)q-CO2H
  MOD_RES (10)..(10): The C-terminal group of Xaa at position 10 is modified with R2, wherein the modification is NH2 to form a C-terminal amide or absent
KXXXXXXXXX

SEQ ID NO: 10 - protein, 39 aa, Artificial Sequence
  Synthetic Construct
  MISC_FEATURE (2)..(2): Xaa at position 2 is Aib
  MISC_FEATURE (6)..(6): Xaa at position 6 is alpha-MeF(2F)
  MISC_FEATURE (13)..(13): Xaa at position 13 is alpha-MeL
  MOD_RES (17)..(17): K at position 17 is chemically modified by conjugation of the epsilon-amino group of the K side chain with (2-[2-(2-amino-ethoxy)-ethoxy]-acetyl)2-(gamma-Glu)-CO-(CH2)18-CO 2H
  MISC_FEATURE (20)..(20): Xaa at position 20 is Aib
  MISC_FEATURE (24)..(24): Xaa at position 24 is D-Glu
  MOD_RES (39)..(39): The Serine at position 39 is amidated
YXEGTXTSDYSIXLDEKAQXEFIXYLIEGGPSSGAPPPS

SEQ ID NO: 11 - protein, 39 aa, Artificial Sequence
  Synthetic Construct
  MISC_FEATURE (2)..(2): Xaa at position 2 is Aib
  MISC_FEATURE (6)..(6): Xaa at position 6 is alpha-MeF(2F)
  MISC_FEATURE (13)..(13): Xaa at position 13 is alpha-MeL
  MISC_FEATURE (16)..(16): Xaa at position 16 is Orn
  MOD_RES (17)..(17): K at position 17 is chemically modified by conjugation of the epsilon-amino group of the K side chain with (2-[2-(2-amino-ethoxy)-ethoxy]-acetyl)2-(gamma-Glu)-CO-(CH2)16-CO 2H
  MISC_FEATURE (20)..(20): Xaa at position 20 is Aib
  MISC_FEATURE (24)..(24): Xaa at position 24 is D-Glu
  MOD_RES (39)..(39): The Serine at position 39 is amidated
YXEGTXTSDYSIXLDXKAQXEFIXYLIEGGPSSGAPPPS

SEQ ID NO: 12 - protein, 39 aa, Artificial Sequence; identical to SEQ ID NO: 11
  Synthetic Construct
  MISC_FEATURE (2)..(2): Xaa at position 2 is Aib
  MISC_FEATURE (6)..(6): Xaa at position 6 is alpha-MeF(2F)
  MISC_FEATURE (13)..(13): Xaa at position 13 is alpha-MeL
  MISC_FEATURE (16)..(16): Xaa at position 16 is Orn
  MOD_RES (17)..(17): K at position 17 is chemically modified by conjugation of the epsilon-amino group of the K side chain with (2-[2-(2-amino-ethoxy)-ethoxy]-acetyl)2-(gamma-Glu)-CO-(CH2)18-CO 2H
  MISC_FEATURE (20)..(20): Xaa at position 20 is Aib
  MISC_FEATURE (24)..(24): Xaa at position 24 is D-Glu
  MISC_FEATURE (39)..(39): The Serine at position 39 is amidated

SEQ ID NO: 13 - protein, 39 aa, Artificial Sequence
  Synthetic Construct
  MISC_FEATURE (2)..(2): Xaa at position 2 is Aib
  MISC_FEATURE (6)..(6): Xaa at position 6 is alpha-MeF(2F)
  MISC_FEATURE (10)..(10): Xaa at position 10 is 4Pal
  MISC_FEATURE (13)..(13): Xaa at position 13 is alpha-MeL
  MISC_FEATURE (16)..(16): Xaa at position 16 is Orn
  MOD_RES (17)..(17): K at position 17 is chemically modified by conjugation of the epsilon-amino group of the K side chain with (2-[2-(2-amino-ethoxy)-ethoxy]-acetyl)2-(gamma-Glu)-CO-(CH2)16-CO 2H
  MISC_FEATURE (20)..(20): Xaa at position 20 is Aib
  MISC_FEATURE (24)..(24): Xaa at position 24 is D-Glu
  MISC_FEATURE (25)..(25): Xaa at position 25 is alpha-MeY
  MOD_RES (39)..(39): The Serine at position 39 is amidated
YXEGTXTSDXSIXLDXKAQXEFIXXLIEGGPSSGAPPPS

SEQ ID NO: 14 - protein, 39 aa, Artificial Sequence
  Synthetic Construct
  MISC_FEATURE (2)..(2): Xaa at position 2 is Aib
  MISC_FEATURE (6)..(6): Xaa at position 6 is alpha-MeF(2F)
  MISC_FEATURE (13)..(13): Xaa at position 13 is alpha-MeL
  MISC_FEATURE (16)..(16): Xaa at position 16 is Orn
  MOD_RES (17)..(17): K at position 17 is chemically modified by conjugation of the epsilon-amino group of the K side chain with (2-[2-(2-amino-ethoxy)-ethoxy]-acetyl)2-(gamma-Glu)-CO-(CH2)16-CO 2H
  MISC_FEATURE (20)..(20): Xaa at position 20 is Aib
  MISC_FEATURE (24)..(24): Xaa at position 24 is D-Glu
  MISC_FEATURE (25)..(25): Xaa at position 25 is alpha-MeY
  MOD_RES (39)..(39): The Serine at position 39 is amidated
YXEGTXTSDVSIXLDXKAQXEFIXXLIEGGPSSGAPPPS

SEQ ID NO: 15 - protein, 39 aa, Artificial Sequence
  Synthetic Construct
  MISC_FEATURE (2)..(2): Xaa at position 2 is Aib
  MOD_RES (17)..(17): Lys at position 17 is chemically modified by conjugation of the epsilon-amino group of the Lys side chain with (2-[2-(2-amino-ethoxy)-ethoxy]-acetyl)2-(gamma-Glu)-CO-(CH2)18-CO 2H
  MISC_FEATURE (20)..(20): Xaa at position 20 is Aib
  MOD_RES (39)..(39): Ser at position 39 is amidated
YXEGTFTSDYSILLDKKAQXAFIEYLLEGGPSSGAPPPS

SEQ ID NO: 16 - protein, 39 aa, Artificial Sequence
  Synthetic Construct
  MISC_FEATURE (2)..(2): Xaa at position 2 is Aib
  MOD_RES (17)..(17): Lys at position 17 is chemically modified by conjugation of the epsilon-amino group of the Lys side chain with (2-[2-(2-amino-ethoxy)-ethoxy]-acetyl)2-(gamma-Glu)-CO-(CH2)18-CO 2H
  MISC_FEATURE (20)..(20): Xaa at position 20 is Aib
  MOD_RES (39)..(39): Ser at position 39 is amidated
YXEGTFTSDYSILLDSKAQXAFIEYLLEGGPSSGAPPPS

SEQ ID NO: 17 - protein, 39 aa, Artificial Sequence
  Synthetic Construct
  MISC_FEATURE (2)..(2): Xaa at position 2 is Aib
  MOD_RES (17)..(17): Lys at position 17 is chemically modified by conjugation of the epsilon-amino group of the Lys side chain with (2-[2-(2-amino-ethoxy)-ethoxy]-acetyl)2-(gamma-Glu)-CO-(CH2)18-CO 2H
  MISC_FEATURE (20)..(20): Xaa at position 20 is Aib
  MOD_RES (39)..(39): Ser at position 39 is amidated
YXEGTFTSDYSILLDKKAQXAFIEYLIEGGPSSGAPPPS

SEQ ID NO: 18 - protein, 39 aa, Artificial Sequence
  Synthetic Construct
  MISC_FEATURE (2)..(2): Xaa at position 2 is Aib
  MOD_RES (17)..(17): Lys at position 17 is chemically modified by conjugation of the epsilon-amino group of the Lys side chain with (2-[2-(2-amino-ethoxy)-ethoxy]-acetyl)2-(gamma-Glu)-CO-(CH2)18-CO 2H
  MISC_FEATURE (20)..(20): Xaa at position 20 is Aib
  MOD_RES (39)..(39): Ser at position 39 is amidated
YXEGTFTSDYSILLDSKAQXAFIEYLIEGGPSSGAPPPS

SEQ ID NO: 19 - protein, 39 aa, Artificial Sequence
  Synthetic Construct
  MISC_FEATURE (2)..(2): Xaa at position 2 is Aib
  MISC_FEATURE (20)..(20): Xaa at position 20 is Aib
  MOD_RES (24)..(24): Lys at position 24 is chemically modified by conjugation of the epsilon-amino group of the Lys side chain with (2-[2-(2-amino-ethoxy)-ethoxy]-acetyl)2-(gamma-Glu)-CO-(CH2)18-CO 2H
  MISC_FEATURE (29)..(29): Xaa at position 29 is Aib
  MOD_RES (39)..(39): Ser at position 39 is amidated
YXEGTFTSDYSILLDSIAQXAFIKYLLAXGPSSGAPPPS

SEQ ID NO: 20 - protein, 39 aa, Artificial Sequence
  Synthetic Construct
  MISC_FEATURE (2)..(2): Xaa at position 2 is Aib
  MISC_FEATURE (20)..(20): Xaa at position 20 is Aib
  MOD_RES (28)..(28): Lys at position 28 is chemically modified by conjugation of the epsilon-amino group of the Lys side chain with (2-[2-(2-amino-ethoxy)-ethoxy]-acetyl)2-(gamma-Glu)-CO-(CH2)18-CO 2H
  MISC_FEATURE (29)..(29): Xaa at position 29 is Aib
  MOD_RES (39)..(39): Ser at position 39 is amidated
YXEGTFTSDYSILLDSIAQXAFIEYLLKXGPSSGAPPPS

SEQ ID NO: 21 - protein, 39 aa, Artificial Sequence
  Synthetic Construct
  MISC_FEATURE (2)..(2): Xaa at position 2 is Aib
  MOD_RES (20)..(20): Lys at position 20 is chemically modified by conjugation of the epsilon-amino group of the Lys side chain with (2-[2-(2-amino-ethoxy)-ethoxy]-acetyl)2-(gamma-Glu)-CO-(CH2)18-CO 2H
  MOD_RES (39)..(39): Ser at position 39 is amidated
YXEGTFTSDYSILLDKIAQKAFIEYLIEGGPSSGAPPPS

SEQ ID NO: 22 - protein, 39 aa, Artificial Sequence
  Synthetic Construct
  MISC_FEATURE (2)..(2): Xaa at position 2 is Aib
  MISC_FEATURE (16)..(16): Xaa at position 16 is Aib
  MOD_RES (20)..(20): Lys at position 20 is chemically modified by conjugation of the epsilon-amino group of the Lys side chain with (2-[2-(2-amino-ethoxy)-ethoxy]-acetyl)2-(gamma-Glu)-CO-(CH2)18-CO 2H
  MOD_RES (39)..(39): Ser at position 39 is amidated
YXEGTFTSDYSILLDXIAQKAFIEYLIEGGPSSGAPPPS

SEQ ID NO: 23 - protein, 39 aa, Artificial Sequence
  Synthetic Construct
  MISC_FEATURE (2)..(2): Xaa at position 2 is Aib
  MOD_RES (20)..(20): Lys at position 20 is chemically modified by conjugation of the epsilon-amino group of the Lys side chain with (2-[2-(2-amino-ethoxy)-ethoxy]-acetyl)2-(gamma-Glu)-CO-(CH2)18-CO 2H
  MISC_FEATURE (29)..(29): Xaa at position 29 is Aib
  MOD_RES (39)..(39): Ser at position 39 is amidated
YXEGTFTSDYSILLDKIAQKEFIQYLLEXGPSSGAPPPS

SEQ ID NO: 24 - protein, 39 aa, Artificial Sequence
  Synthetic Construct
  MISC_FEATURE (2)..(2): Xaa at position 2 is Aib
  MOD_RES (17)..(17): Lys at position 17 is chemically modified by conjugation of the epsilon-amino group of the Lys side chain with (2-[2-(2-amino-ethoxy)-ethoxy]-acetyl)2-(gamma-Glu)-CO-(CH2)18-CO 2H
  MISC_FEATURE (20)..(20): Xaa at position 20 is Aib
  MISC_FEATURE (29)..(29): Xaa at position 29 is Aib
  MOD_RES (39)..(39): Ser at position 39 is amidated
HXEGTFTSDYSILLDKKAQXAFIEYLLEXGPSSGAPPPS

SEQ ID NO: 25 - protein, 39 aa, Artificial Sequence
  Synthetic Construct
  MISC_FEATURE (2)..(2): Xaa at position 2 is Aib
  MOD_RES (17)..(17): Lys at position 17 is chemically modified by conjugation of the epsilon-amino group of the Lys side chain with (2-[2-(2-amino-ethoxy)-ethoxy]-acetyl)2-(gamma-Glu)-CO-(CH2)18-CO 2H
  MISC_FEATURE (20)..(20): Xaa at position 20 is Aib
  MISC_FEATURE (29)..(29): Xaa at position 29 is Aib
  MOD_RES (39)..(39): Ser at position 39 is amidated
HXEGTFTSDYSILLDKKAQXAFIEYLIEXGPSSGAPPPS

SEQ ID NO: 26 - protein, 34 aa, Artificial Sequence
  Synthetic Construct
  MISC_FEATURE (2)..(2): Xaa at position 2 is Aib
  MOD_RES (20)..(20): Lys at position 20 is chemically modified by conjugation of the epsilon-amino group of the Lys side chain with (2-[2-(2-amino-ethoxy)-ethoxy]-acetyl)2-(gamma-Glu)-CO-(CH2)18-CO 2H
  MISC_FEATURE (29)..(29): Xaa at position 29 is Aib
  MOD_RES (34)..(34): Ser at position 34 is amidated
HXEGTFTSDYSILLDKIAQKAFIEYLLEXGPSSG

SEQ ID NO: 27 - protein, 39 aa, Artificial Sequence
  Synthetic Construct
  MISC_FEATURE (2)..(2): Xaa at position 2 is Aib
  MISC_FEATURE (13)..(13): Xaa at position 13 is alpha-methyl-L
  MOD_RES (17)..(17): Lys at position 17 is chemically modified by conjugation of the epsilon-amino group of the Lys side chain with Dab-(2-[2-(2-Amino-ethoxy)-ethoxy]-acetyl)-Dab-(2-[2-(2-Amino-eth oxy)-ethoxy]-acetyl)-CO-(CH2)18-CO2H
  MISC_FEATURE (20)..(20): Xaa at position 20 is alpha-methyl-Lys
  MISC_FEATURE (29)..(29): Xaa at position 29 is Aib
  MOD_RES (39)..(39): Ser at position 39 is amidated
HXEGTFTSDYSIXLDKKAQXAFIQYLLAXGPSSGAPKPS

SEQ ID NO: 28 - protein, 39 aa, Artificial Sequence
  Synthetic Construct
  MISC_FEATURE (2)..(2): Xaa at position 2 is Aib
  MISC_FEATURE (13)..(13): Xaa at position 13 is alpha-methyl-Leu
  MOD_RES (17)..(17): Lys at position 17 is chemically modified by conjugation of the epsilon-amino group of the Lys side chain with Dab-(2-[2-(2-Amino-ethoxy)-ethoxy]-acetyl)-Dab-(2-[2-(2-Amino-eth oxy)-ethoxy]-acetyl)-CO-(CH2)18-CO2H
  MISC_FEATURE (20)..(20): Xaa at position 20 is alpha-methyl-Lys
  MISC_FEATURE (29)..(29): Xaa at position 29 is Aib
  MOD_RES (39)..(39): Ser at position 39 is amidated
HXEGTFTSDYSIXLDKKAQXAFIQYLLAXGPSSGAPPPS

SEQ ID NO: 29 - protein, 39 aa, Artificial Sequence
  Synthetic Construct
  MISC_FEATURE (2)..(2): Xaa at position 2 is Aib
  MISC_FEATURE (13)..(13): Xaa at position 13 is alpha-methyl-Leu
  MOD_RES (17)..(17): Lys at position 17 is chemically modified by conjugation of the epsilon-amino group of the Lys side chain with (2-[2-(2-amino-ethoxy)-ethoxy]-acetyl)2-(gamma-Glu)-CO-(CH2)18-CO 2H
  MISC_FEATURE (20)..(20): Xaa at position 20 is Aib
  MOD_RES (39)..(39): Ser at position 39 is amidated
YXEGTFTSDYSIXLDKKAQXAFIEYLIEGGPSSGAPPPS

SEQ ID NO: 30 - protein, 39 aa, Artificial Sequence
  Synthetic Construct
  MISC_FEATURE (2)..(2): Xaa at position 2 is Aib
  MISC_FEATURE (13)..(13): Xaa at position 13 is alpha-methyl-Leu
  MOD_RES (17)..(17): Lys at position 17 is chemically modified by conjugation of the epsilon-amino group of the Lys side chain with (2-[2-(2-amino-ethoxy)-ethoxy]-acetyl)2-(gamma-Glu)-CO-(CH2)18-CO 2H
  MISC_FEATURE (20)..(20): Xaa at position 20 is alpha-methyl-Lys
  MOD_RES (39)..(39): Ser at position 39 is amidated
YXEGTFTSDYSIXLDEKAQXAFIEYLLEGGPSSGAPPPS

SEQ ID NO: 31 - protein, 39 aa, Artificial Sequence
  Synthetic Construct
  MISC_FEATURE (2)..(2): Xaa at position 2 is Aib
  MISC_FEATURE (13)..(13): Xaa at position 13 is alpha-methyl-Leu
  MOD_RES (17)..(17): Lys at position 17 is chemically modified by conjugation of the epsilon-amino group of the Lys side chain with (2-[2-(2-amino-ethoxy)-ethoxy]-acetyl)2-(gamma-Glu)-CO-(CH2)18-CO 2H
  MISC_FEATURE (20)..(20): Xaa at position 20 is alpha-methyl-Lys
  MISC_FEATURE (29)..(29): Xaa at position 29 is Aib
  MOD_RES (39)..(39): Ser at position 39 is amidated
YXEGTFTSDYSIXLDEKAQXAFIEYLLEXGPSSGAPPPS

SEQ ID NO: 32 - protein, 39 aa, Artificial Sequence
  Synthetic Construct
  MISC_FEATURE (2)..(2): Xaa at position 2 is Aib
  MOD_RES (10)..(10): Lys at position 10 is chemically modified by conjugation of the epsilon-amino group of the Lys side chain with (2-[2-(2-amino-ethoxy)-ethoxy]-acetyl)2-(gamma-Glu)-CO-(CH2)18-CO 2H
  MISC_FEATURE (20)..(20): Xaa at position 20 is Aib
  MOD_RES (39)..(39): Ser at position 39 is amidated
YXEGTFTSDKSILLDKIAQXAFIEYLIEGGPSSGAPPPS

SEQ ID NO: 33 - protein, 39 aa, Artificial Sequence
  Synthetic Construct
  MISC_FEATURE (2)..(2): Xaa at position 2 is Aib
  MOD_RES (11)..(11): Lys at position 11 is chemically modified by conjugation of the epsilon-amino group of the Lys side chain with (2-[2-(2-amino-ethoxy)-ethoxy]-acetyl)2-(gamma-Glu)-CO-(CH2)18-CO 2H
  MISC_FEATURE (20)..(20): Xaa at position 20 is Aib
  MOD_RES (39)..(39): Ser at position 39 is amidated
YXEGTFTSDYKILLDKIAQXAFIEYLIEGGPSSGAPPPS

SEQ ID NO: 34 - protein, 39 aa, Artificial Sequence
  Synthetic Construct
  MISC_FEATURE (2)..(2): Xaa at position 2 is Aib
  MOD_RES (12)..(12): Lys at position 12 is chemically modified by conjugation of the epsilon-amino group of the Lys side chain with (2-[2-(2-amino-ethoxy)-ethoxy]-acetyl)2-(gamma-Glu)-CO-(CH2)18-CO 2H
  MISC_FEATURE (20)..(20): Xaa at position 20 is Aib
  MOD_RES (39)..(39): Ser at position 39 is amidated
YXEGTFTSDYSKLLDKIAQXAFIEYLIEGGPSSGAPPPS

SEQ ID NO: 35 - protein, 39 aa, Artificial Sequence
  Synthetic Construct
  MISC_FEATURE (2)..(2): Xaa at position 2 is Aib
  MOD_RES (13)..(13): Lys at position 13 is chemically modified by conjugation of the epsilon-amino group of the Lys side chain with (2-[2-(2-amino-ethoxy)-ethoxy]-acetyl)2-(gamma-Glu)-CO-(CH2)18-CO 2H
  MISC_FEATURE (20)..(20): Xaa at position 20 is Aib
  MOD_RES (39)..(39): Ser at position 39 is amidated
YXEGTFTSDYSIKLDKIAQXAFIEYLIEGGPSSGAPPPS

SEQ ID NO: 36 - protein, 39 aa, Artificial Sequence
  Synthetic Construct
  MISC_FEATURE (2)..(2): Xaa at position 2 is Aib
  MOD_RES (14)..(14): Lys at position 14 is chemically modified by conjugation of the epsilon-amino group of the Lys side chain with (2-[2-(2-amino-ethoxy)-ethoxy]-acetyl)2-(gamma-Glu)-CO-(CH2)18-CO 2H
  MISC_FEATURE (20)..(20): Xaa at position 20 is Aib
  MOD_RES (39)..(39): Ser at position 39 is amidated
YXEGTFTSDYSILKDKIAQXAFIEYLIEGGPSSGAPPPS

SEQ ID NO: 37 - protein, 39 aa, Artificial Sequence
  Synthetic Construct
  MISC_FEATURE (2)..(2): Xaa at position 2 is Aib
  MOD_RES (15)..(15): Lys at position 15 is chemically modified by conjugation of the epsilon-amino group of the Lys side chain with (2-[2-(2-amino-ethoxy)-ethoxy]-acetyl)2-(gamma-Glu)-CO-(CH2)18-CO 2H
  MISC_FEATURE (20)..(20): Xaa at position 20 is Aib
  MOD_RES (39)..(39): Ser at position 39 is amidated
YXEGTFTSDYSILLKKIAQXAFIEYLIEGGPSSGAPPPS

SEQ ID NO: 38 - protein, 39 aa, Artificial Sequence
  Synthetic Construct
  MISC_FEATURE (2)..(2): Xaa at position 2 is Aib
  MOD_RES (16)..(16): Lys at position 16 is chemically modified by conjugation of the epsilon-amino group of the Lys side chain with (2-[2-(2-amino-ethoxy)-ethoxy]-acetyl)2-(gamma-Glu)-CO-(CH2)18-CO 2H
  MISC_FEATURE (20)..(20): Xaa at position 20 is Aib
  MOD_RES (39)..(39): Ser at position 39 is amidated
YXEGTFTSDYSILLDKIAQXAFIEYLIEGGPSSGAPPPS

SEQ ID NO: 39 - protein, 39 aa, Artificial Sequence
  Synthetic Construct
  MISC_FEATURE (2)..(2): Xaa at position 2 is Aib
  MOD_RES (18)..(18): Lys at position 18 is chemically modified by conjugation of the epsilon-amino group of the Lys side chain with (2-[2-(2-amino-ethoxy)-ethoxy]-acetyl)2-(gamma-Glu)-CO-(CH2)18-CO 2H
  MISC_FEATURE (20)..(20): Xaa at position 20 is Aib
  MOD_RES (39)..(39): Ser at position 39 is amidated
YXEGTFTSDYSILLDKIKQXAFIEYLIEGGPSSGAPPPS

SEQ ID NO: 40 - protein, 39 aa, Artificial Sequence
  Synthetic Construct
  MISC_FEATURE (2)..(2): Xaa at position 2 is Aib
  MOD_RES (19)..(19): Lys at position 19 is chemically modified by conjugation of the epsilon-amino group of the Lys side chain with (2-[2-(2-amino-ethoxy)-ethoxy]-acetyl)2-(gamma-Glu)-CO-(CH2)18-CO 2H
  MISC_FEATURE (20)..(20): Xaa at position 20 is Aib
  MOD_RES (39)..(39): Ser at position 39 is amidated
YXEGTFTSDYSILLDKIAKXAFIEYLIEGGPSSGAPPPS

SEQ ID NO: 41 - protein, 39 aa, Artificial Sequence
  Synthetic Construct
  MISC_FEATURE (2)..(2): Xaa at position 2 is Aib
  MISC_FEATURE (20)..(20): Xaa at position 20 is Aib
  MOD_RES (21)..(21): Lys at position 17 is chemically modified by conjugation of the epsilon-amino group of the Lys side chain with (2-[2-(2-amino-ethoxy)-ethoxy]-acetyl)2-(gamma-Glu)-CO-(CH2)18-CO 2H
  MOD_RES (39)..(39): Ser at position 39 is amidated
YXEGTFTSDYSILLDKIAQXKFIEYLIEGGPSSGAPPPS

SEQ ID NO: 42 - protein, 39 aa, Artificial Sequence
  Synthetic Construct
  MISC_FEATURE (2)..(2): Xaa at position 2 is Aib
  MISC_FEATURE (20)..(20): Xaa at position 20 is Aib
  MOD_RES (23)..(23): Lys at position 23 is chemically modified by conjugation of the epsilon-amino group of the Lys side chain with (2-[2-(2-amino-ethoxy)-ethoxy]-acetyl)2-(gamma-Glu)-CO-(CH2)18-CO 2H
  MOD_RES (39)..(39): Ser at position 39 is amidated
YXEGTFTSDYSILLDKIAQXAFKEYLIEGGPSSGAPPPS

SEQ ID NO: 43 - protein, 39 aa, Artificial Sequence
  Synthetic Construct
  MISC_FEATURE (2)..(2): Xaa at position 2 is Aib
  MISC_FEATURE (20)..(20): Xaa at position 20 is Aib
  MOD_RES (24)..(24): Lys at position 24 is chemically modified by conjugation of the epsilon-amino group of the Lys side chain with (2-[2-(2-amino-ethoxy)-ethoxy]-acetyl)2-(gamma-Glu)-CO-(CH2)18-CO 2H
  MOD_RES (39)..(39): Ser at position 39 is amidated
YXEGTFTSDYSILLDKIAQXAFIKYLIEGGPSSGAPPPS

SEQ ID NO: 44 - protein, 39 aa, Artificial Sequence
  Synthetic Construct
  MISC_FEATURE (2)..(2): Xaa at position 2 is Aib
  MISC_FEATURE (20)..(20): Xaa at position 20 is Aib
  MOD_RES (26)..(26): Lys at position 26 is chemically modified by conjugation of the epsilon-amino group of the Lys side chain with (2-[2-(2-amino-ethoxy)-ethoxy]-acetyl)2-(gamma-Glu)-CO-(CH2)18-CO 2H
  MOD_RES (39)..(39): Ser at position 39 is amidated
YXEGTFTSDYSILLDKIAQXAFIEYKIEGGPSSGAPPPS

SEQ ID NO: 45 - protein, 39 aa, Artificial Sequence
  Synthetic Construct
  MISC_FEATURE (2)..(2): Xaa at position 2 is Aib
  MISC_FEATURE (20)..(20): Xaa at position 20 is Aib
  MOD_RES (27)..(27): Lys at position 27 is chemically modified by conjugation of the epsilon-amino group of the Lys side chain with (2-[2-(2-amino-ethoxy)-ethoxy]-acetyl)2-(gamma-Glu)-CO-(CH2)18-CO 2H
  MOD_RES (39)..(39): Ser at position 39 is amidated
YXEGTFTSDYSILLDKIAQXAFIEYLKEGGPSSGAPPPS

SEQ ID NO: 46 - protein, 39 aa, Artificial Sequence
  Synthetic Construct
  MISC_FEATURE (2)..(2): Xaa at position 2 is Aib
  MISC_FEATURE (20)..(20): Xaa at position 20 is Aib
  MOD_RES (28)..(28): Lys at position 28 is chemically modified by conjugation of the epsilon-amino group of the Lys side chain with (2-[2-(2-amino-ethoxy)-ethoxy]-acetyl)2-(gamma-Glu)-CO-(CH2)18-CO 2H
  MOD_RES (39)..(39): Ser at position 39 is amidated
YXEGTFTSDYSILLDKIAQXAFIEYLIKGGPSSGAPPPS

SEQ ID NO: 47 - protein, 39 aa, Artificial Sequence
  Synthetic Construct
  MISC_FEATURE (2)..(2): Xaa at position 2 is Aib
  MISC_FEATURE (20)..(20): Xaa at position 20 is Aib
  MOD_RES (29)..(29): Lys at position 29 is chemically modified by conjugation of the epsilon-amino group of the Lys side chain with (2-[2-(2-amino-ethoxy)-ethoxy]-acetyl)2-(gamma-Glu)-CO-(CH2)18-CO 2H
  MOD_RES (39)..(39): Ser at position 39 is amidated
YXEGTFTSDYSILLDKIAQXAFIEYLIEKGPSSGAPPPS

SEQ ID NO: 48 - protein, 39 aa, Artificial Sequence
  Synthetic Construct
  MISC_FEATURE (2)..(2): Xaa at position 2 is Aib
  MISC_FEATURE (20)..(20): Xaa at position 20 is Aib
  MOD_RES (30)..(30): Lys at position 30 is chemically modified by conjugation of the epsilon-amino group of the Lys side chain with (2-[2-(2-amino-ethoxy)-ethoxy]-acetyl)2-(gamma-Glu)-CO-(CH2)18-CO 2H
  MOD_RES (39)..(39): Ser at position 39 is amidated
YXEGTFTSDYSILLDKIAQXAFIEYLIEGKPSSGAPPPS

SEQ ID NO: 49 - protein, 39 aa, Artificial Sequence
  Synthetic Construct
  MISC_FEATURE (2)..(2): Xaa at position 2 is Aib
  MISC_FEATURE (20)..(20): Xaa at position 20 is Aib
  MOD_RES (31)..(31): Lys at position 31 is chemically modified by conjugation of the epsilon-amino group of the Lys side chain with (2-[2-(2-amino-ethoxy)-ethoxy]-acetyl)2-(gamma-Glu)-CO-(CH2)18-CO 2H
  MOD_RES (39)..(39): Ser at position 39 is amidated
YXEGTFTSDYSILLDKIAQXAFIEYLIEGGKSSGAPPPS

SEQ ID NO: 50 - protein, 39 aa, Artificial Sequence
  Synthetic Construct
  MISC_FEATURE (2)..(2): Xaa at position 2 is Aib
  MISC_FEATURE (20)..(20): Xaa at position 20 is Aib
  MOD_RES (32)..(32): Lys at position 32 is chemically modified by conjugation of the epsilon-amino group of the Lys side chain with (2-[2-(2-amino-ethoxy)-ethoxy]-acetyl)2-(gamma-Glu)-CO-(CH2)18-CO 2H
  MOD_RES (39)..(39): Ser at position 39 is amidated
YXEGTFTSDYSILLDKIAQXAFIEYLIEGGPKSGAPPPS

SEQ ID NO: 51 - protein, 39 aa, Artificial Sequence
  Synthetic Construct
  MISC_FEATURE (2)..(2): Xaa at position 2 is Aib
  MISC_FEATURE (20)..(20): Xaa at position 20 is Aib
  MOD_RES (33)..(33): Lys at position 33 is chemically modified by conjugation of the epsilon-amino group of the Lys side chain with (2-[2-(2-amino-ethoxy)-ethoxy]-acetyl)2-(gamma-Glu)-CO-(CH2)18-CO 2H
  MOD_RES (39)..(39): Ser at position 39 is amidated
YXEGTFTSDYSILLDKIAQXAFIEYLIEGGPSKGAPPPS

SEQ ID NO: 52 - protein, 39 aa, Artificial Sequence
  Synthetic Construct
  MISC_FEATURE (2)..(2): Xaa at position 2 is Aib
  MISC_FEATURE (20)..(20): Xaa at position 20 is Aib
  MOD_RES (34)..(34): Lys at position 34 is chemically modified by conjugation of the epsilon-amino group of the Lys side chain with (2-[2-(2-amino-ethoxy)-ethoxy]-acetyl)2-(gamma-Glu)-CO-(CH2)18-CO 2H
  MOD_RES (39)..(39): Ser at position 39 is amidated
YXEGTFTSDYSILLDKIAQXAFIEYLIEGGPSSKAPPPS

SEQ ID NO: 53 - protein, 39 aa, Artificial Sequence
  Synthetic Construct
  MISC_FEATURE (2)..(2): Xaa at position 2 is Aib
  MISC_FEATURE (20)..(20): Xaa at position 20 is Aib
  MOD_RES (35)..(35): Lys at position 35 is chemically modified by conjugation of the epsilon-amino group of the Lys side chain with (2-[2-(2-amino-ethoxy)-ethoxy]-acetyl)2-(gamma-Glu)-CO-(CH2)18-CO 2H
  MOD_RES (39)..(39): Ser at position 39 is amidated
YXEGTFTSDYSILLDKIAQXAFIEYLIEGGPSSGKPPPS

SEQ ID NO: 54 - protein, 39 aa, Artificial Sequence
  Synthetic Construct
  MISC_FEATURE (2)..(2): Xaa at position 2 is Aib
  MISC_FEATURE (20)..(20): Xaa at position 20 is Aib
  MOD_RES (36)..(36): Lys at position 36 is chemically modified by conjugation of the epsilon-amino group of the Lys side chain with (2-[2-(2-amino-ethoxy)-ethoxy]-acetyl)2-(gamma-Glu)-CO-(CH2)18-CO 2H
  MOD_RES (39)..(39): Ser at position 39 is amidated
YXEGTFTSDYSILLDKIAQXAFIEYLIEGGPSSGAKPPS

SEQ ID NO: 55 - protein, 39 aa, Artificial Sequence
  Synthetic Construct
  MISC_FEATURE (2)..(2): Xaa at position 2 is Aib
  MISC_FEATURE (20)..(20): Xaa at position 20 is Aib
  MOD_RES (37)..(37): Lys at position 37 is chemically modified by conjugation of the epsilon-amino group of the Lys side chain with (2-[2-(2-amino-ethoxy)-ethoxy]-acetyl)2-(gamma-Glu)-CO-(CH2)18-CO 2H
  MOD_RES (39)..(39): Ser at position 39 is amidated
YXEGTFTSDYSILLDKIAQXAFIEYLIEGGPSSGAPKPS

SEQ ID NO: 56 - protein, 39 aa, Artificial Sequence
  Synthetic Construct
  MISC_FEATURE (2)..(2): Xaa at position 2 is Aib
  MISC_FEATURE (20)..(20): Xaa at position 20 is Aib
  MOD_RES (38)..(38): Lys at position 38 is chemically modified by conjugation of the epsilon-amino group of the Lys side chain with (2-[2-(2-amino-ethoxy)-ethoxy]-acetyl)2-(gamma-Glu)-CO-(CH2)18-CO 2H
  MOD_RES (39)..(39): Ser at position 39 is amidated
YXEGTFTSDYSILLDKIAQXAFIEYLIEGGPSSGAPPKS

SEQ ID NO: 57 - protein, 39 aa, Artificial Sequence
  Synthetic Construct
  MISC_FEATURE (2)..(2): Xaa at position 2 is Aib
  MISC_FEATURE (20)..(20): Xaa at position 20 is Aib
  MOD_RES (39)..(39): Lys at position 39 is chemically modified by conjugation of the epsilon-amino group of the Lys side chain with (2-[2-(2-amino-ethoxy)-ethoxy]-acetyl)2-(gamma-Glu)-CO-(CH2)18-CO 2H
  MOD_RES (39)..(39): Lys at position 39 is amidated
YXEGTFTSDYSILLDKIAQXAFIEYLIEGGPSSGAPPPK

SEQ ID NO: 58 - protein, 40 aa, Artificial Sequence
  Synthetic Construct
  MISC_FEATURE (2)..(2): Xaa at position 2 is Aib
  MISC_FEATURE (20)..(20): Xaa at position 20 is Aib
  MOD_RES (40)..(40): Lys at position 40 is chemically modified by conjugation of the epsilon-amino group of the Lys side chain with (2-[2-(2-amino-ethoxy)-ethoxy]-acetyl)2-(gamma-Glu)-CO-(CH2)18-CO 2H
  MOD_RES (40)..(40): Lys at position 40 is amidated
YXEGTFTSDYSILLDKIAQXAFIEYLIEGGPSSGAPPPSK

SEQ ID NO: 59 - protein, 34 aa, Artificial Sequence
  Synthetic Construct
  MISC_FEATURE (2)..(2): Xaa at position 2 is Aib
  MOD_RES (17)..(17): Lys at position 17 is chemically modified by conjugation of the epsilon-amino group of the Lys side chain with (2-[2-(2-amino-ethoxy)-ethoxy]-acetyl)2-(gamma-Glu)-CO-(CH2)18-CO 2H
  MISC_FEATURE (20)..(20): Xaa at position 20 is Aib
  MOD_RES (34)..(34): Gly at position 34 is amidated
YXEGTFTSDYSILLDKKAQXAFIEYLIEGGPSSG

SEQ ID NO: 60 - protein, 30 aa, Artificial Sequence
  Synthetic Construct
  MISC_FEATURE (2)..(2): Xaa at position 2 is Aib
  MOD_RES (17)..(17): Lys at position 17 is chemically modified by conjugation of the epsilon-amino group of the Lys side chain with (2-[2-(2-amino-ethoxy)-ethoxy]-acetyl)2-(gamma-Glu)-CO-(CH2)18-CO 2H
  MISC_FEATURE (20)..(20): Xaa at position 20 is Aib
  MOD_RES (30)..(30): Gly at position 30 is amidated
YXEGTFTSDYSILLDKKAQXAFIEYLIEGG

SEQ ID NO: 61 - protein, 39 aa, Artificial Sequence
  Synthetic Construct
  MISC_FEATURE (2)..(2): Xaa at position 2 is Aib
  MISC_FEATURE (13)..(13): Xaa at position 13 is alpha-methyl-Leu
  MOD_RES (17)..(17): Lys at position 17 is chemically modified by conjugation of the epsilon-amino group of the Lys side chain with (2-[2-(2-amino-ethoxy)-ethoxy]-acetyl)2-(gamma-Glu)-CO-(CH2)18-CO 2H
  MISC_FEATURE (20)..(20): Xaa at position 20 is Aib
  MOD_RES (39)..(39): Ser at position 39 is amidated
YXEGTFTSDYSIXLDSKAQXAFIEYLIEGGPSSGAPPPS

SEQ ID NO: 62 - protein, 39 aa, Artificial Sequence
  Synthetic Construct
  MISC_FEATURE (2)..(2): Xaa at position 2 is Aib
  MISC_FEATURE (13)..(13): Xaa at position 13 is alpha-methyl-Leu
  MOD_RES (17)..(17): Lys at position 17 is chemically modified by conjugation of the epsilon-amino group of the Lys side chain with (2-[2-(2-amino-ethoxy)-ethoxy]-acetyl)2-(gamma-Glu)-CO-(CH2)18-CO 2H
  MISC_FEATURE (20)..(20): Xaa at position 20 is Aib
  MOD_RES (39)..(39): Ser at position 39 is amidated
HXEGTFTSDYSIXLDKKAQXAFIEYLIEGGPSSGAPPPS

SEQ ID NO: 63 - protein, 39 aa, Artificial Sequence
  Synthetic Construct
  MISC_FEATURE (2)..(2): Xaa at position 2 is Aib
  MISC_FEATURE (13)..(13): Xaa at position 13 is alpha-methyl-Leu
  MOD_RES (17)..(17): Lys at position 17 is chemically modified by conjugation of the epsilon-amino group of the Lys side chain with (2-[2-(2-amino-ethoxy)-ethoxy]-acetyl)2-(gamma-Glu)-CO-(CH2)18-CO 2H
  MOD_RES (39)..(39): Ser at position 39 is amidated
HXEGTFTSDYSIXLDKKAQHAFIEYLIEGGPSSGAPPPS

SEQ ID NO: 64 - protein, 39 aa, Artificial Sequence
  Synthetic Construct
  MISC_FEATURE (2)..(2): Xaa at position 2 is Aib
  MISC_FEATURE (13)..(13): Xaa at position 13 is alpha-methyl-Leu
  MOD_RES (17)..(17): Lys at position 17 is chemically modified by conjugation of the epsilon-amino group of the Lys side chain with (2-[2-(2-amino-ethoxy)-ethoxy]-acetyl)2-(gamma-Glu)-CO-(CH2)18-CO 2H
  MOD_RES (39)..(39): Ser at position 39 is amidated
HXEGTFTSDYSIXLDEKAQHAFIEYLIEGGPSSGAPPPS

SEQ ID NO: 65 - protein, 39 aa, Artificial Sequence
  Synthetic Construct
  MISC_FEATURE (2)..(2): Xaa at position 2 is Aib
  MISC_FEATURE (13)..(13): Xaa at position 13 is alpha-methyl-Leu
  MOD_RES (17)..(17): Lys at position 17 is chemically modified by conjugation of the epsilon-amino group of the Lys side chain with (2-[2-(2-amino-ethoxy)-ethoxy]-acetyl)2-(gamma-Glu)-CO-(CH2)18-CO 2H
  MOD_RES (39)..(39): Ser at position 39 is amidated
YXEGTFTSDYSIXLDEKAQHAFIEYLIEGGPSSGAPPPS

SEQ ID NO: 66 - protein, 39 aa, Artificial Sequence
  Synthetic Construct
  MISC_FEATURE (2)..(2): Xaa at position 2 is Aib
  MISC_FEATURE (6)..(6): Xaa at position 6 is alpha-methyl-Phe
  MOD_RES (17)..(17): Lys at position 17 is chemically modified by conjugation of the epsilon-amino group of the Lys side chain with (2-[2-(2-amino-ethoxy)-ethoxy]-acetyl)2-(gamma-Glu)-CO-(CH2)18-CO 2H
  MISC_FEATURE (20)..(20): Xaa at position 20 is Aib
  MOD_RES (39)..(39): Ser at position 39 is amidated
YXEGTXTSDYSILLDKKAQXAFIEYLIEGGPSSGAPPPS

SEQ ID NO: 67 - protein, 39 aa, Artificial Sequence
  Synthetic Construct
  MISC_FEATURE (2)..(2): Xaa at position 2 is Aib
  MOD_RES (17)..(17): Lys at position 17 is chemically modified by conjugation of the epsilon-amino group of the Lys side chain with (2-[2-(2-amino-ethoxy)-ethoxy]-acetyl)2-(gamma-Glu)-CO-(CH2)18-CO 2H
  MISC_FEATURE (20)..(20): Xaa at position 20 is Aib
  MOD_RES (39)..(39): Ser at position 39 is amidated
YXEGTFTSDYSSLLDKKAQXAFIEYLIEGGPSSGAPPPS

SEQ ID NO: 68 - protein, 39 aa, Artificial Sequence
  Synthetic Construct
  MISC_FEATURE (2)..(2): Xaa at position 2 is Aib
  MISC_FEATURE (13)..(13): Xaa at position 13 is alpha-methyl-Leu
  MOD_RES (17)..(17): Lys at position 17 is chemically modified by conjugation of the epsilon-amino group of the Lys side chain with (2-[2-(2-amino-ethoxy)-ethoxy]-acetyl)2-(gamma-Glu)-CO-(CH2)18-CO 2H
  MISC_FEATURE (20)..(20): Xaa at position 20 is Aib
  MOD_RES (39)..(39): Ser at position 39 is amidated
YXEGTFTSDYSIXLDEKAQXAFIEYLIEGGPSSGAPPPS

SEQ ID NO: 69 - protein, 39 aa, Artificial Sequence
  Synthetic Construct
  MISC_FEATURE (2)..(2): Xaa at position 2 is Aib
  MISC_FEATURE (13)..(13): Xaa at position 13 is alpha-methyl-Leu
  MISC_FEATURE (16)..(16): Xaa at position 16 is Aib
  MOD_RES (17)..(17): Lys at position 17 is chemically modified by conjugation of the epsilon-amino group of the Lys side chain with (2-[2-(2-amino-ethoxy)-ethoxy]-acetyl)2-(gamma-Glu)-CO-(CH2)18-CO 2H
  MISC_FEATURE (20)..(20): Xaa at position 20 is Aib
  MOD_RES (39)..(39): Ser at position 39 is amidated
YXEGTFTSDYSIXLDXKAQXAFIEYLIEGGPSSGAPPPS

SEQ ID NO: 70 - protein, 39 aa, Artificial Sequence
  Synthetic Construct
  MISC_FEATURE (2)..(2): Xaa at position 2 is Aib
  MISC_FEATURE (13)..(13): Xaa at position 13 is alpha-methyl-Leu
  MOD_RES (17)..(17): Lys at position 17 is chemically modified by conjugation of the epsilon-amino group of the Lys side chain with (2-[2-(2-amino-ethoxy)-ethoxy]-acetyl)2-(gamma-Glu)-CO-(CH2)18-CO 2H
  MISC_FEATURE (20)..(20): Xaa at position 20 is Aib
  MOD_RES (39)..(39): Ser at position 39 is amidated
YXEGTFTSDYSIXLDSKAQXAFIEYLLEGGPSSGAPPPS

SEQ ID NO: 71 - protein, 30 aa, Artificial Sequence
  Synthetic Construct
  MISC_FEATURE (2)..(2): Xaa at position 2 is Aib
  MISC_FEATURE (13)..(13): Xaa at position 13 is alpha-methyl-Leu
  MOD_RES (17)..(17): Lys at position 17 is chemically modified by conjugation of the epsilon-amino group of the Lys side chain with (2-[2-(2-amino-ethoxy)-ethoxy]-acetyl)2-(gamma-Glu)-CO-(CH2)18-CO 2H
  MISC_FEATURE (20)..(20): Xaa at position 20 is Aib
  MOD_RES (30)..(30): Gly at position 30 is amidated
YXEGTFTSDYSIXLDKKAQXAFIEYLIEGG

SEQ ID NO: 72 - protein, 30 aa, Artificial Sequence
  Synthetic Construct
  MISC_FEATURE (2)..(2): Xaa at position 2 is Aib
  MISC_FEATURE (13)..(13): Xaa at position 13 is alpha-methyl-Leu
  MOD_RES (17)..(17): Lys at position 17 is chemically modified by conjugation of the epsilon-amino group of the Lys side chain with (2-[2-(2-amino-ethoxy)-ethoxy]-acetyl)2-(gamma-Glu)-CO-(CH2)18-CO 2H
  MISC_FEATURE (20)..(20): Xaa at position 20 is Aib
  MOD_RES (30)..(30): Gly at position 30 is amidated
YXEGTFTSDYSIXLDEKAQXAFIEYLIEGG

SEQ ID NO: 73 - protein, 30 aa, Artificial Sequence
  Synthetic Construct
  MISC_FEATURE (2)..(2): Xaa at position 2 is Aib
  MISC_FEATURE (13)..(13): Xaa at position 13 is alpha-methyl-Leu
  MOD_RES (17)..(17): Lys at position 17 is chemically modified by conjugation of the epsilon-amino group of the Lys side chain with (2-[2-(2-amino-ethoxy)-ethoxy]-acetyl)2-(gamma-Glu)-CO-(CH2)18-CO 2H
  MISC_FEATURE (20)..(20): Xaa at position 20 is Aib
  MOD_RES (30)..(30): Gly at position 30 is amidated
YXEGTFTSDYSIXLDSKAQXAFIEYLIEGG

SEQ ID NO: 74 - protein, 30 aa, Artificial Sequence
  Synthetic Construct
  MISC_FEATURE (2)..(2): Xaa at position 2 is Aib
  MISC_FEATURE (13)..(13): Xaa at position 13 is alpha-methyl-Leu
  MOD_RES (17)..(17): Lys at position 17 is chemically modified by conjugation of the epsilon-amino group of the Lys side chain with (2-[2-(2-amino-ethoxy)-ethoxy]-acetyl)2-(gamma-Glu)-CO-(CH2)18-CO 2H
  MISC_FEATURE (20)..(20): Xaa at position 20 is Aib
  MOD_RES (30)..(30): Gly at position 30 is amidated
YXEGTFTSDYSIXLDTKAQXAFIEYLIEGG

SEQ ID NO: 75 - protein, 39 aa, Artificial Sequence; identical to SEQ ID NO: 30
  Synthetic Construct
  MISC_FEATURE (2)..(2): Xaa at position 2 is Aib
  MISC_FEATURE (13)..(13): Xaa at position 13 is alpha-methyl-Leu
  MOD_RES (17)..(17): Lys at position 17 is chemically modified by conjugation of the epsilon-amino group of the Lys side chain with (2-[2-(2-amino-ethoxy)-ethoxy]-acetyl)2-(gamma-Glu)-CO-(CH2)18-CO 2H
  MISC_FEATURE (20)..(20): Xaa at position 20 is Aib
  MOD_RES (39)..(39): Ser at position 39 is amidated

SEQ ID NO: 76 - protein, 39 aa, Artificial Sequence
  Synthetic Construct
  MISC_FEATURE (2)..(2): Xaa at position 2 is Aib
  MOD_RES (17)..(17): Lys at position 17 is chemically modified by conjugation of the epsilon-amino group of the Lys side chain with (2-[2-(2-amino-ethoxy)-ethoxy]-acetyl)2-(gamma-Glu)-CO-(CH2)18-CO 2H
  MISC_FEATURE (20)..(20): Xaa at position 20 is Aib
  MISC_FEATURE (22)..(22): Xaa at position 22 is alpha-methyl-Phe
  MOD_RES (39)..(39): Ser at position 39 is amidated
YXEGTFTSDYSILLDKKAQXAXIEYLIEGGPSSGAPPPS

SEQ ID NO: 77 - protein, 39 aa, Artificial Sequence
  Synthetic Construct
  MISC_FEATURE (2)..(2): Xaa at position 2 is Aib
  MISC_FEATURE (11)..(11): Xaa at position 11 is alpha-methyl-Ser
  MOD_RES (17)..(17): Lys at position 17 is chemically modified by conjugation of the epsilon-amino group of the Lys side chain with (2-[2-(2-amino-ethoxy)-ethoxy]-acetyl)2-(gamma-Glu)-CO-(CH2)18-CO 2H
  MISC_FEATURE (20)..(20): Xaa at position 20 is Aib
  MOD_RES (39)..(39): Ser at position 39 is amidated
YXEGTFTSDYXILLDKKAQXAFIEYLIEGGPSSGAPPPS

SEQ ID NO: 78 - protein, 39 aa, Artificial Sequence
  Synthetic Construct
  MISC_FEATURE (2)..(2): Xaa at position 2 is Aib
  MISC_FEATURE (6)..(6): Xaa at position 6 is alpha-methyl-Phe
  MISC_FEATURE (13)..(13): Xaa at position 13 is alpha-methyl-Leu
  MOD_RES (17)..(17): Lys at position 17 is chemically modified by conjugation of the epsilon-amino group of the Lys side chain with (2-[2-(2-amino-ethoxy)-ethoxy]-acetyl)2-(gamma-Glu)-CO-(CH2)18-CO 2H
  MISC_FEATURE (20)..(20): Xaa at position 20 is Aib
  MOD_RES (39)..(39): Ser at position 39 is amidated
YXEGTXTSDYSIXLDKKAQXAFIEYLIEGGPSSGAPPPS

SEQ ID NO: 79 - protein, 30 aa, Artificial Sequence
  Synthetic Construct
  MISC_FEATURE (2)..(2): Xaa at position 2 is Aib
  MOD_RES (10)..(10): Lys at position 10 is chemically modified by conjugation of the epsilon-amino group of the Lys side chain with (2-[2-(2-amino-ethoxy)-ethoxy]-acetyl)2-(gamma-Glu)-CO-(CH2)18-CO 2H
  MISC_FEATURE (20)..(20): Xaa at position 20 is Aib
  MOD_RES (30)..(30): Gly at position 30 is amidated
YXEGTFTSDKSILLDKIAQXAFIEYLIEGG

SEQ ID NO: 80 - protein, 30 aa, Artificial Sequence
  Synthetic Construct
  MISC_FEATURE (2)..(2): Xaa at position 2 is Aib
  MOD_RES (14)..(14): Lys at position 14 is chemically modified by conjugation of the epsilon-amino group of the Lys side chain with (2-[2-(2-amino-ethoxy)-ethoxy]-acetyl)2-(gamma-Glu)-CO-(CH2)18-CO 2H
  MISC_FEATURE (20)..(20): Xaa at position 20 is Aib
  MOD_RES (30)..(30): Gly at position 30 is amidated
YXEGTFTSDYSILKDKIAQXAFIEYLIEGG

SEQ ID NO: 81 - protein, 30 aa, Artificial Sequence
  Synthetic Construct
  MISC_FEATURE (2)..(2): Xaa at position 2 is Aib
  MISC_FEATURE (20)..(20): Xaa at position 20 is Aib
  MOD_RES (21)..(21): Lys at position 21 is chemically modified by conjugation of the epsilon-amino group of the Lys side chain with (2-[2-(2-amino-ethoxy)-ethoxy]-acetyl)2-(gamma-Glu)-CO-(CH2)18-CO 2H
  MOD_RES (30)..(30): Gly at position 30 is amidated
YXEGTFTSDYSILLDKIAQXKFIEYLIEGG

SEQ ID NO: 82 - protein, 30 aa, Artificial Sequence
  Synthetic Construct
  MISC_FEATURE (2)..(2): Xaa at position 2 is Aib
  MISC_FEATURE (20)..(20): Xaa at position 20 is Aib
  MOD_RES (28)..(28): Lys at position 28 is chemically modified by conjugation of the epsilon-amino group of the Lys side chain with (2-[2-(2-amino-ethoxy)-ethoxy]-acetyl)2-(gamma-Glu)-CO-(CH2)18-CO 2H
  MOD_RES (30)..(30): Gly at position 30 is amidated
YXEGTFTSDYSILLDKIAQXAFIEYLIKGG

SEQ ID NO: 83 - protein, 39 aa, Artificial Sequence
  Synthetic Construct
  MISC_FEATURE (2)..(2): Xaa at position 2 is Aib
  MISC_FEATURE (13)..(13): Xaa at position 13 is alpha-methyl-Leu
  MOD_RES (17)..(17): Lys at position 17 is chemically modified by conjugation of the epsilon-amino group of the Lys side chain with (2-[2-(2-amino-ethoxy)-ethoxy]-acetyl)2-(gamma-Glu)-CO-(CH2)18-CO 2H
  MISC_FEATURE (20)..(20): Xaa at position 20 is Aib
  MISC_FEATURE (22)..(22): Xaa at position 22 is alpha-methyl-Phe
  MOD_RES (39)..(39): Ser at position 39 is amidated
YXEGTFTSDYSIXLDKKAQXAXIEYLIEGGPSSGAPPPS

SEQ ID NO: 84 - protein, 39 aa, Artificial Sequence
  Synthetic Construct
  MISC_FEATURE (2)..(2): Xaa at position 2 is Aib
  MISC_FEATURE (13)..(13): Xaa at position 13 is alpha-methyl-Leu
  MOD_RES (17)..(17): Lys at position 17 is chemically modified by conjugation of the epsilon-amino group of the Lys side chain with (2-[2-(2-amino-ethoxy)-ethoxy]-acetyl)2-(gamma-Glu)-CO-(CH2)18-CO 2H
  MISC_FEATURE (20)..(20): Xaa at position 20 is Aib
  MISC_FEATURE (26)..(26): Xaa at position 26 is alpha-methyl-Leu
  MOD_RES (39)..(39): Ser at position 39 is amidated
YXEGTFTSDYSIXLDKKAQXAFIEYXIEGGPSSGAPPPS

SEQ ID NO: 85 - protein, 39 aa, Artificial Sequence
  Synthetic Construct
  MISC_FEATURE (2)..(2): Xaa at position 2 is Aib
  MISC_FEATURE (6)..(6): Xaa at position 6 is alpha-methyl-Phe
  MISC_FEATURE (13)..(13): Xaa at position 13 is alpha-methyl-Leu
  MOD_RES (17)..(17): Lys at position 17 is chemically modified by conjugation of the epsilon-amino group of the Lys side chain with (2-[2-(2-amino-ethoxy)-ethoxy]-acetyl)2-(gamma-Glu)-CO-(CH2)18-CO 2H
  MISC_FEATURE (20)..(20): Xaa at position 20 is Aib
  MISC_FEATURE (22)..(22): Xaa at position 22 is alpha-methyl-Phe
  MOD_RES (39)..(39): Ser at position 39 is amidated
YXEGTXTSDYSIXLDKKAQXAXIEYLIEGGPSSGAPPPS

SEQ ID NO: 86 - protein, 38 aa, Artificial Sequence
  Synthetic Construct
  MISC_FEATURE (2)..(2): Xaa at position 2 is Aib
  MISC_FEATURE (19)..(19): Xaa at position 19 is Aib
  MOD_RES (37)..(37): Lys at position 37 is chemically modified by conjugation of the epsilon-amino group of the Lys side chain with (2-[2-(2-amino-ethoxy)-ethoxy]-acetyl)2-(gamma-Glu)-CO-(CH2)18-CO 2H
  MOD_RES (38)..(38): Ser at position 38 is amidated
YXEGTFTSDYSILLKIAQXAFIEYLIEGGPSSGAPPKS

SEQ ID NO: 87 - protein, 39 aa, Artificial Sequence
  Synthetic Construct
  MISC_FEATURE (1)..(1): Xaa at position 1 is D-Tyr
  MISC_FEATURE (2)..(2): Xaa at position 2 is Aib
  MOD_RES (17)..(17): Lys at position 17 is chemically modified by conjugation of the epsilon-amino group of the Lys side chain with (2-[2-(2-amino-ethoxy)-ethoxy]-acetyl)2-(gamma-Glu)-CO-(CH2)18-CO 2H
  MISC_FEATURE (20)..(20): Xaa at position 20 is Aib
  MOD_RES (39)..(39): Ser at position 39 is amidated
XXEGTFTSDYSILLDKKAQXAFIEYLIEGGPSSGAPPPS

SEQ ID NO: 88 - protein, 39 aa, Artificial Sequence
  Synthetic Construct
  MISC_FEATURE (1)..(1): Xaa at position 1 is D-Tyr
  MOD_RES (1)..(1): The N-terminal amino is acetylated
  MOD_RES (17)..(17): Lys at position 17 is chemically modified by conjugation of the epsilon-amino group of the Lys side chain with (2-[2-(2-amino-ethoxy)-ethoxy]-acetyl)2-(gamma-Glu)-CO-(CH2)18-CO 2H
  MISC_FEATURE (20)..(20): Xaa at position 20 is Aib
  MOD_RES (39)..(39): Ser at position 39 is amidated
XAEGTFTSDYSILLDKKAQXAFIEYLIEGGPSSGAPPPS

SEQ ID NO: 89 - protein, 39 aa, Artificial Sequence; identical to SEQ ID NO: 17
  Synthetic Construct
  MISC_FEATURE (2)..(2): Xaa at position 2 is D-Ala
  MOD_RES (17)..(17): Lys at position 17 is chemically modified by conjugation of the epsilon-amino group of the Lys side chain with (2-[2-(2-amino-ethoxy)-ethoxy]-acetyl)2-(gamma-Glu)-CO-(CH2)18-CO 2H
  MISC_FEATURE (20)..(20): Xaa at position 20 is Aib
  MOD_RES (39)..(39): Ser at position 39 is amidated

SEQ ID NO: 90 - protein, 39 aa, Artificial Sequence; identical to SEQ ID NO: 77
  Synthetic Construct
  MISC_FEATURE (2)..(2): Xaa at position 2 is Aib
  MISC_FEATURE (11)..(11): Xaa at position 11 is D-Ser
  MOD_RES (17)..(17): Lys at position 17 is chemically modified by conjugation of the epsilon-amino group of the Lys side chain with (2-[2-(2-amino-ethoxy)-ethoxy]-acetyl)2-(gamma-Glu)-CO-(CH2)18-CO 2H
  MISC_FEATURE (20)..(20): Xaa at position 20 is Aib
  MOD_RES (39)..(39): Ser at position 39 is amidated

SEQ ID NO: 91 - protein, 39 aa, Artificial Sequence
  Synthetic Construct
  MISC_FEATURE (2)..(2): Xaa at position 2 is Aib
  MISC_FEATURE (12)..(12): Xaa at position 12 is D-Ile
  MOD_RES (17)..(17): Lys at position 17 is chemically modified by conjugation of the epsilon-amino group of the Lys side chain with (2-[2-(2-amino-ethoxy)-ethoxy]-acetyl)2-(gamma-Glu)-CO-(CH2)18-CO 2H
  MISC_FEATURE (20)..(20): Xaa at position 20 is Aib
  MOD_RES (39)..(39): Ser at position 39 is amidated
YXEGTFTSDYSXLLDKKAQXAFIEYLIEGGPSSGAPPPS

SEQ ID NO: 92 - protein, 39 aa, Artificial Sequence
  Synthetic Construct
  MISC_FEATURE (2)..(2): Xaa at position 2 is Aib
  MOD_RES (17)..(17): Lys at position 17 is chemically modified by conjugation of the epsilon-amino group of the Lys side chain with (2-[2-(2-amino-ethoxy)-ethoxy]-acetyl)2-(gamma-Glu)-CO-(CH2)18-CO 2H
  MISC_FEATURE (20)..(20): Xaa at position 20 is Aib
  MISC_FEATURE (28)..(28): Xaa at position 28 is D-Glu
  MOD_RES (39)..(39): Ser at position 39 is amidated
YXEGTFTSDYSILLDKKAQXAFIEYLIXGGPSSGAPPPS

SEQ ID NO: 93 - protein, 39 aa, Artificial Sequence
  Synthetic Construct
  MISC_FEATURE (2)..(2): Xaa at position 2 is Aib
  MOD_RES (17)..(17): Lys at position 17 is chemically modified by conjugation of the epsilon-amino group of the Lys side chain with (2-[2-(2-amino-ethoxy)-ethoxy]-acetyl)2-(gamma-Glu)-CO-(CH2)18-CO 2H
  MISC_FEATURE (20)..(20): Xaa at position 20 is Aib
  MISC_FEATURE (24)..(24): Xaa at position 24 is D-Glu
  MOD_RES (39)..(39): Ser at position 39 is amidated
YXEGTFTSDYSILLDKKAQXAFIXYLIEGGPSSGAPPPS

SEQ ID NO: 94 - protein, 39 aa, Artificial Sequence
  Synthetic Construct
  MISC_FEATURE (2)..(2): Xaa at position 2 is Aib
  MOD_RES (17)..(17): Lys at position 17 is chemically modified by conjugation of the epsilon-amino group of the Lys side chain with (2-[2-(2-amino-ethoxy)-ethoxy]-acetyl)2-(gamma-Glu)-CO-(CH2)18-CO 2H
  MISC_FEATURE (20)..(20): Xaa at position 20 is Aib
  MOD_RES (39)..(39): Ser at position 39 is amidated
YXEGTFTSDASILLDKKAQXAFIEYLIEGGPSSGAPPPS

SEQ ID NO: 95 - protein, 39 aa, Artificial Sequence
  Synthetic Construct
  MISC_FEATURE (2)..(2): Xaa at position 2 is Aib
  MOD_RES (17)..(17): Lys at position 17 is chemically modified by conjugation of the epsilon-amino group of the Lys side chain with (2-[2-(2-amino-ethoxy)-ethoxy]-acetyl)2-(gamma-Glu)-CO-(CH2)18-CO 2H
  MISC_FEATURE (20)..(20): Xaa at position 20 is Aib
  MOD_RES (39)..(39): Ser at position 39 is amidated
YXEGTFTSDYSILLDKKAQXAFIEYLIEAGPSSGAPPPS

SEQ ID NO: 96 - protein, 39 aa, Artificial Sequence; identical to SEQ ID NO: 17
  Synthetic Construct
  MISC_FEATURE (2)..(2): Xaa at position 2 is alpha-methyl-Pro
  MOD_RES (17)..(17): Lys at position 17 is chemically modified by conjugation of the epsilon-amino group of the Lys side chain with (2-[2-(2-amino-ethoxy)-ethoxy]-acetyl)2-(gamma-Glu)-CO-(CH2)18-CO 2H
  MISC_FEATURE (20)..(20): Xaa at position 20 is Aib
  MOD_RES (39)..(39): Ser at position 39 is amidated

SEQ ID NO: 97 - protein, 39 aa, Artificial Sequence
  Synthetic Construct
  MOD_RES (17)..(17): Lys at position 17 is chemically modified by conjugation of the epsilon-amino group of the Lys side chain with (2-[2-(2-amino-ethoxy)-ethoxy]-acetyl)2-(gamma-Glu)-CO-(CH2)18-CO 2H
  MISC_FEATURE (20)..(20): Xaa at position 20 is Aib
  MOD_RES (39)..(39): Ser at position 39 is amidated
YPEGTFTSDYSILLDKKAQXAFIEYLIEGGPSSGAPPPS

SEQ ID NO: 98 - protein, 39 aa, Artificial Sequence
  Synthetic Construct
  MISC_FEATURE (2)..(2): Xaa at position 2 is Aib
  MISC_FEATURE (3)..(3): Xaa at position 3 is Aad
  MOD_RES (17)..(17): Lys at position 17 is chemically modified by conjugation of the epsilon-amino group of the Lys side chain with (2-[2-(2-amino-ethoxy)-ethoxy]-acetyl)2-(gamma-Glu)-CO-(CH2)18-CO 2H
  MISC_FEATURE (20)..(20): Xaa at position 20 is Aib
  MOD_RES (39)..(39): Ser at position 39 is amidated
YXXGTFTSDYSILLDKKAQXAFIEYLIEGGPSSGAPPPS

SEQ ID NO: 99 - protein, 39 aa, Artificial Sequence
  Synthetic Construct
  MISC_FEATURE (2)..(2): Xaa at position 2 is Aib
  MOD_RES (17)..(17): Lys at position 17 is chemically modified by conjugation of the epsilon-amino group of the Lys side chain with (2-[2-(2-amino-ethoxy)-ethoxy]-acetyl)2-(gamma-Glu)-CO-(CH2)18-CO 2H
  MISC_FEATURE (20)..(20): Xaa at position 20 is Aib
  MOD_RES (39)..(39): Ser at position 39 is amidated
YXNGTFTSDYSILLDKKAQXAFIEYLIEGGPSSGAPPPS

SEQ ID NO: 100 - protein, 39 aa, Artificial Sequence; identical to SEQ ID NO: 98
  Synthetic Construct
  MISC_FEATURE (2)..(2): Xaa at position 2 is Aib
  MISC_FEATURE (3)..(3): Xaa at position 3 is gamma-Glu
  MOD_RES (17)..(17): Lys at position 17 is chemically modified by conjugation of the epsilon-amino group of the Lys side chain with (2-[2-(2-amino-ethoxy)-ethoxy]-acetyl)2-(gamma-Glu)-CO-(CH2)18-CO 2H
  MISC_FEATURE (20)..(20): Xaa at position 20 is Aib
  MOD_RES (39)..(39): Ser at position 39 is amidated

SEQ ID NO: 101 - protein, 30 aa, Artificial Sequence
  Synthetic Construct
  MISC_FEATURE (2)..(2): Xaa at position 2 is Aib
  MISC_FEATURE (6)..(6): Xaa at position 6 is alpha-methyl-Phe
  MOD_RES (10)..(10): Lys at position 10 is chemically modified by conjugation of the epsilon-amino group of the Lys side chain with (2-[2-(2-amino-ethoxy)-ethoxy]-acetyl)2-(gamma-Glu)-CO-(CH2)18-CO 2H
  MISC_FEATURE (20)..(20): Xaa at position 20 is Aib
  MOD_RES (30)..(30): Gly at position 30 is amidated
YXEGTXTSDKSILLDKIAQXAFIEYLIEGG

SEQ ID NO: 102 - protein, 30 aa, Artificial Sequence
  Synthetic Construct
  MISC_FEATURE (2)..(2): Xaa at position 2 is Aib
  MISC_FEATURE (6)..(6): Xaa at position 6 is alpha-methyl-Phe
  MOD_RES (14)..(14): Lys at position 14 is chemically modified by conjugation of the epsilon-amino group of the Lys side chain with (2-[2-(2-amino-ethoxy)-ethoxy]-acetyl)2-(gamma-Glu)-CO-(CH2)18-CO 2H
  MISC_FEATURE (20)..(20): Xaa at position 20 is Aib
  MISC_FEATURE (30)..(30): Gly at position 30 is amidated
YXEGTXTSDYSILKDKIAQXAFIEYLIEGG

SEQ ID NO: 103 - protein, 30 aa, Artificial Sequence
  Synthetic Construct
  MISC_FEATURE (2)..(2): Xaa at position 2 is Aib
  MISC_FEATURE (6)..(6): Xaa at position 6 is alpha-methyl-Phe
  MISC_FEATURE (20)..(20): Xaa at position 20 is Aib
  MOD_RES (21)..(21): Lys at position 21 is chemically modified by conjugation of the epsilon-amino group of the Lys side chain with (2-[2-(2-amino-ethoxy)-ethoxy]-acetyl)2-(gamma-Glu)-CO-(CH2)18-CO 2H
  MISC_FEATURE (30)..(30): Gly at position 30 is amidated
YXEGTXTSDYSILLDKIAQXKFIEYLIEGG

SEQ ID NO: 104 - protein, 30 aa, Artificial Sequence
  Synthetic Construct
  MISC_FEATURE (2)..(2): Xaa at position 2 is Aib
  MISC_FEATURE (6)..(6): Xaa at position 6 is alpha-methyl-Phe
  MISC_FEATURE (20)..(20): Xaa at position 20 is Aib
  MOD_RES (28)..(28): Lys at position 28 is chemically modified by conjugation of the epsilon-amino group of the Lys side chain with (2-[2-(2-amino-ethoxy)-ethoxy]-acetyl)2-(gamma-Glu)-CO-(CH2)18-CO 2H
  MOD_RES (30)..(30): Gly at position 30 is amidated
YXEGTXTSDYSILLDKIAQXAFIEYLIKGG

SEQ ID NO: 105 - protein, 30 aa, Artificial Sequence
  Synthetic Construct
  MISC_FEATURE (2)..(2): Xaa at position 2 is Aib
  MOD_RES (10)..(10): Lys at position 10 is chemically modified by conjugation of the epsilon-amino group of the Lys side chain with (2-[2-(2-amino-ethoxy)-ethoxy]-acetyl)2-(gamma-Glu)-CO-(CH2)18-CO 2H
  MISC_FEATURE (13)..(13): Xaa at position 13 is alpha-methyl-Leu
  MISC_FEATURE (20)..(20): Xaa at position 20 is Aib
  MOD_RES (30)..(30): Gly at position 30 is amidated
YXEGTFTSDKSIXLDKIAQXAFIEYLIEGG

SEQ ID NO: 106 - protein, 30 aa, Artificial Sequence
  Synthetic Construct
  MISC_FEATURE (2)..(2): Xaa at position 2 is Aib
  MISC_FEATURE (13)..(13): Xaa at position 13 is alpha-methyl-Leu
  MISC_FEATURE (20)..(20): Xaa at position 20 is Aib
  MOD_RES (28)..(28): Lys at position 28 is chemically modified by conjugation of the epsilon-amino group of the Lys side chain with (2-[2-(2-amino-ethoxy)-ethoxy]-acetyl)2-(gamma-Glu)-CO-(CH2)18-CO 2H
  MOD_RES (30)..(30): Gly at position 30 is amidated
YXEGTFTSDYSIXLDKIAQXAFIEYLIKGG

SEQ ID NO: 107 - protein, 30 aa, Artificial Sequence
  Synthetic Construct
  MISC_FEATURE (2)..(2): Xaa at position 2 is Aib
  MISC_FEATURE (6)..(6): Xaa at position 13 is alpha-methyl-Phe
  MOD_RES (17)..(17): Lys at position 17 is chemically modified by conjugation of the epsilon-amino group of the Lys side chain with (2-[2-(2-amino-ethoxy)-ethoxy]-acetyl)2-(gamma-Glu)-CO-(CH2)18-CO 2H
  MISC_FEATURE (20)..(20): Xaa at position 20 is Aib
  MOD_RES (30)..(30): Gly at position 30 is amidated
YXEGTXTSDYSILLDKKAQXAFIEYLIEGG

SEQ ID NO: 108 - protein, 30 aa, Artificial Sequence
  Synthetic Construct
  MISC_FEATURE (2)..(2): Xaa at position 2 is Aib
  MISC_FEATURE (6)..(6): Xaa at position 6 is alpha-methyl-Phe
  MISC_FEATURE (13)..(13): Xaa at position 13 is alpha-methyl-Leu
  MOD_RES (17)..(17): Lys at position 17 is chemically modified by conjugation of the epsilon-amino group of the Lys side chain with (2-[2-(2-amino-ethoxy)-ethoxy]-acetyl)2-(gamma-Glu)-CO-(CH2)18-CO 2H
  MISC_FEATURE (20)..(20): Xaa at position 20 is Aib
  MOD_RES (30)..(30): Gly at position 30 is amidated
YXEGTXTSDYSIXLDKKAQXAFIEYLIEGG

SEQ ID NO: 109 - protein, 30 aa, Artificial Sequence
  Synthetic Construct
  MISC_FEATURE (2)..(2): Xaa at position 2 is Aib
  MISC_FEATURE (6)..(6): Xaa at position 6 is alpha-methyl-Phe
  MISC_FEATURE (13)..(13): Xaa at position 13 is alpha-methyl-Leu
  MOD_RES (17)..(17): Lys at position 17 is chemically modified by conjugation of the epsilon-amino group of the Lys side chain with (2-[2-(2-amino-ethoxy)-ethoxy]-acetyl)2-(gamma-Glu)-CO-(CH2)18-CO 2H
  MISC_FEATURE (20)..(20): Xaa at position 20 is Aib
  MOD_RES (30)..(30): Gly at position 30 is amidated
YXEGTXTSDYSIXLDEKAQXAFIEYLIEGG

SEQ ID NO: 110 - protein, 30 aa, Artificial Sequence; identical to SEQ ID NO: 109
  Synthetic Construct
  MISC_FEATURE (2)..(2): Xaa at position 2 is Aib
  MISC_FEATURE (6)..(6): Xaa at position 6 is alpha-methyl-Phe(2F)
  MISC_FEATURE (13)..(13): Xaa at position 13 is Aib
  MOD_RES (17)..(17): Lys at position 17 is chemically modified by conjugation of the epsilon-amino group of the Lys side chain with (2-[2-(2-amino-ethoxy)-ethoxy]-acetyl)2-(gamma-Glu)-CO-(CH2)18-CO 2H
  MISC_FEATURE (20)..(20): Xaa at position 20 is Aib
  MOD_RES (30)..(30): Gly at position 30 is amidated

SEQ ID NO: 111 - protein, 30 aa, Artificial Sequence; identical to SEQ ID NO: 109
  Synthetic Construct
  MISC_FEATURE (2)..(2): Xaa at position 2 is Aib
  MISC_FEATURE (6)..(6): Xaa at position 6 is alpha-methyl-Phe
  MISC_FEATURE (13)..(13): Xaa at position 13 is Aib
  MOD_RES (17)..(17): Lys at position 17 is chemically modified by conjugation of the epsilon-amino group of the Lys side chain with (2-[2-(2-amino-ethoxy)-ethoxy]-acetyl)2-(gamma-Glu)-CO-(CH2)18-CO 2H
  MISC_FEATURE (20)..(20): Xaa at position 20 is Aib
  MOD_RES (30)..(30): Gly at position 30 is amidated

SEQ ID NO: 112 - protein, 30 aa, Artificial Sequence
  Synthetic Construct
  MISC_FEATURE (2)..(2): Xaa at position 2 is Aib
  MISC_FEATURE (6)..(6): Xaa at position 6 is alpha-methyl-Phe(2F)
  MISC_FEATURE (13)..(13): Xaa at position 13 is alpha-methyl-Leu
  MOD_RES (17)..(17): Lys at position 17 is chemically modified by conjugation of the epsilon-amino group of the Lys side chain with (2-[2-(2-amino-ethoxy)-ethoxy]-acetyl)2-(gamma-Glu)-CO-(CH2)18-CO 2H
  MISC_FEATURE (20)..(20): Xaa at position 20 is Aib
  MOD_RES (30)..(30): Gly at position 30 is amidated
YXEGTXTSDYSIXLDEKAQXEFIEYLIEGG

SEQ ID NO: 113 - protein, 30 aa, Artificial Sequence; identical to SEQ ID NO: 112
  Synthetic Construct
  MISC_FEATURE (2)..(2): Xaa at position 2 is Aib
  MISC_FEATURE (6)..(6): Xaa at position 6 is alpha-methyl-Phe(2F)
  MISC_FEATURE (13)..(13): Xaa at position 13 is alpha-methyl-Leu
  MOD_RES (17)..(17): Lys at position 17 is chemically modified by conjugation of the epsilon-amino group of the Lys side chain with (2-[2-(2-amino-ethoxy)-ethoxy]-acetyl)2-(gamma-Glu)-CO-(CH2)16-CO 2H
  MISC_FEATURE (20)..(20): Xaa at position 20 is Aib
  MOD_RES (30)..(30): Gly at position 30 is amidated

SEQ ID NO: 114 - protein, 39 aa, Artificial Sequence; identical to SEQ ID NO: 87
  Synthetic Construct
  MISC_FEATURE (1)..(2): Xaa at position 1 combines with Xaa at position 2 to form desHis-psi[NHCO]-Aib
  MOD_RES (17)..(17): Lys at position 17 is chemically modified by conjugation of the epsilon-amino group of the Lys side chain with (2-[2-(2-amino-ethoxy)-ethoxy]-acetyl)2-(gamma-Glu)-CO-(CH2)18-CO 2H
  MISC_FEATURE (20)..(20): Xaa at position 20 is Aib
  MOD_RES (39)..(39): Ser at position 39 is amidated

SEQ ID NO: 115 - protein, 39 aa, Artificial Sequence; identical to SEQ ID NO: 87
  Synthetic Construct
  MISC_FEATURE (1)..(2): Xaa at position 1 combines with Xaa at position 2 to form desHis-Aib
  MOD_RES (17)..(17): Lys at position 17 is chemically modified by conjugation of the epsilon-amino group of the Lys side chain with (2-[2-(2-amino-ethoxy)-ethoxy]-acetyl)2-(gamma-Glu)-CO-(CH2)18-CO 2H
  MISC_FEATURE (20)..(20): Xaa at position 20 is Aib
  MOD_RES (39)..(39): Ser at position 39 is amidated

SEQ ID NO: 116 - protein, 39 aa, Artificial Sequence; identical to SEQ ID NO: 87
  Synthetic Construct
  MISC_FEATURE (1)..(1): Xaa at position 1 is Des-Tyr
  MISC_FEATURE (2)..(2): Xaa at position 2 is Aib
  MOD_RES (17)..(17): Lys at position 17 is chemically modified by conjugation of the epsilon-amino group of the Lys side chain with (2-[2-(2-amino-ethoxy)-ethoxy]-acetyl)2-(gamma-Glu)-CO-(CH2)18-CO 2H
  MISC_FEATURE (20)..(20): Xaa at position 20 is Aib
  MOD_RES (39)..(39): Ser at position 39 is amidated

SEQ ID NO: 117 - protein, 39 aa, Artificial Sequence; identical to SEQ ID NO: 17
  Synthetic Construct
  MISC_FEATURE (2)..(2): Xaa at position 2 is Aib
  MOD_RES (17)..(17): Lys at position 17 is chemically modified by conjugation of the epsilon-amino group of the Lys side chain with (2-[2-(2-amino-ethoxy)-ethoxy]-acetyl)-AOC-(gamma-Glu)-CO-(CH2)18 -CO2H
  MISC_FEATURE (20)..(20): Xaa at position 20 is Aib
  MOD_RES (39)..(39): Ser at position 39 is amidated

SEQ ID NO: 118 - protein, 39 aa, Artificial Sequence; identical to SEQ ID NO: 17
  Synthetic Construct
  MISC_FEATURE (2)..(2): Xaa at position 2 is Aib
  MOD_RES (17)..(17): Lys at position 17 is chemically modified by conjugation of the epsilon-amino group of the Lys side chain with AOC-(2-[2-(2-amino-ethoxy)-ethoxy]-acetyl)-(gamma-Glu)-CO-(CH2)18 -CO2H
  MISC_FEATURE (20)..(20): Xaa at position 20 is Aib
  MOD_RES (39)..(39): Ser at position 39 is amidated

SEQ ID NO: 119 - protein, 39 aa, Artificial Sequence; identical to SEQ ID NO: 17
  Synthetic Construct
  MISC_FEATURE (2)..(2): Xaa at position 2 is Aib
  MOD_RES (17)..(17): Lys at position 17 is chemically modified by conjugation of the epsilon-amino group of the Lys side chain with (2-[2-(2-amino-ethoxy)-ethoxy]-acetyl)-(gamma-Glu)-(Trx)-CO-(CH2) 18-CO2H
  MISC_FEATURE (20)..(20): Xaa at position 20 is Aib
  MOD_RES (39)..(39): Ser at position 39 is amidated

SEQ ID NO: 120 - protein, 39 aa, Artificial Sequence; identical to SEQ ID NO: 17
  Synthetic Construct
  MISC_FEATURE (2)..(2): Xaa at position 2 is Aib
  MOD_RES (17)..(17): Lys at position 17 is chemically modified by conjugation of the epsilon-amino group of the Lys side chain with (2-[2-(2-amino-ethoxy)-ethoxy]-acetyl)-(Trx)-(gamma-Glu)-CO-(CH2) 18-CO2H
  MISC_FEATURE (20)..(20): Xaa at position 20 is Aib
  MOD_RES (39)..(39): Ser at position 39 is amidated

SEQ ID NO: 121 - protein, 39 aa, Artificial Sequence; identical to SEQ ID NO: 17
  Synthetic Construct
  MISC_FEATURE (2)..(2): Xaa at position 2 is Aib
  MOD_RES (17)..(17): Lys at position 17 is chemically modified by conjugation of the epsilon-amino group of the Lys side chain with (2-[2-(2-amino-ethoxy)-ethoxy]-acetyl)-(epsilon-Lys)-(gamma-Glu)- CO-(CH2)18-CO2H
  MISC_FEATURE (20)..(20): Xaa at position 20 is Aib
  MOD_RES (39)..(39): Ser at position 39 is amidated

SEQ ID NO: 122 - protein, 39 aa, Artificial Sequence; identical to SEQ ID NO: 17
  Synthetic Construct
  MISC_FEATURE (2)..(2): Xaa at position 2 is Aib
  MOD_RES (17)..(17): Lys at position 17 is chemically modified by conjugation of the epsilon-amino group of the Lys side chain with (2-[2-(2-amino-ethoxy)-ethoxy]-acetyl)2-(epsilon-Lys)-CO-(CH2)18- CO2H
  MISC_FEATURE (20)..(20): Xaa at position 20 is Aib
  MOD_RES (39)..(39): Ser at position 39 is amidated

SEQ ID NO: 123 - protein, 39 aa, Artificial Sequence; identical to SEQ ID NO: 17
  Synthetic Construct
  MISC_FEATURE (2)..(2): Xaa at position 2 is Aib
  MOD_RES (17)..(17): Lys at position 17 is chemically modified by conjugation of the epsilon-amino group of the Lys side chain with (2-[2-(2-amino-ethoxy)-ethoxy]-acetyl)-(epsilon-Lys)-(epsilon-Lys )-CO-(CH2)18-CO2H
  MISC_FEATURE (20)..(20): Xaa at position 2 is Aib
  MOD_RES (39)..(39): Ser at position 39 is amidated

SEQ ID NO: 124 - protein, 39 aa, Artificial Sequence
  Synthetic Construct
  MISC_FEATURE (2)..(2): Xaa at position 2 is Aib
  MISC_FEATURE (6)..(6): Xaa at position 6 is alpha-methyl-Phe
  MISC_FEATURE (13)..(13): Xaa at position 13 is alpha-methyl-Leu
  MOD_RES (17)..(17): Lys at position 17 is chemically modified by conjugation of the epsilon-amino group of the Lys side chain with (2-[2-(2-amino-ethoxy)-ethoxy]-acetyl)2-(gamma-Glu)-CO-(CH2)18-CO 2H
  MISC_FEATURE (20)..(20): Xaa at position 20 is Aib
  MOD_RES (39)..(39): Ser at position 39 is amidated
YXEGTXTSDYSIXLDEKAQXAFIEYLIEGGPSSGAPPPS

SEQ ID NO: 125 - protein, 39 aa, Artificial Sequence
  Synthetic Construct
  MISC_FEATURE (2)..(2): Xaa at position 2 is Aib
  MISC_FEATURE (6)..(6): Xaa at position 6 is alpha-methyl-Phe
  MISC_FEATURE (13)..(13): Xaa at position 13 is alpha-methyl-Leu
  MOD_RES (17)..(17): Lys at position 17 is chemically modified by conjugation of the epsilon-amino group of the Lys side chain with (2-[2-(2-amino-ethoxy)-ethoxy]-acetyl)2-(gamma-Glu)-CO-(CH2)18-CO 2H
  MISC_FEATURE (20)..(20): Xaa at position 20 is Aib
  MOD_RES (39)..(39): Ser at position 39 is amidated
YXEGTXTSDYSIXLDEKAQXEFIEYLIEGGPSSGAPPPS

SEQ ID NO: 126 - protein, 39 aa, Artificial Sequence; identical to SEQ ID NO: 124
  Synthetic Construct
  MISC_FEATURE (2)..(2): Xaa at position 2 is Aib
  MISC_FEATURE (6)..(6): Xaa at position 6 is alpha-methyl-Phe
  MISC_FEATURE (13)..(13): Xaa at position 13 is Aib
  MOD_RES (17)..(17): Lys at position 17 is chemically modified by conjugation of the epsilon-amino group of the Lys side chain with (2-[2-(2-amino-ethoxy)-ethoxy]-acetyl)2-(gamma-Glu)-CO-(CH2)18-CO 2H
  MISC_FEATURE (20)..(20): Xaa at position 20 is Aib
  MOD_RES (39)..(39): Ser at position 39 is amidated

SEQ ID NO: 127 - protein, 39 aa, Artificial Sequence; identical to SEQ ID NO: 125
  Synthetic Construct
  MISC_FEATURE (2)..(2): Xaa at position 2 is Aib
  MISC_FEATURE (6)..(6): Xaa at position 6 is alpha-methyl-Phe(2F)
  MISC_FEATURE (13)..(13): Xaa at position 13 is alpha-methyl-Leu
  MOD_RES (17)..(17): Lys at position 17 is chemically modified by conjugation of the epsilon-amino group of the Lys side chain with (2-[2-(2-amino-ethoxy)-ethoxy]-acetyl)2-(gamma-Glu)-CO-(CH2)18-CO 2H
  MISC_FEATURE (20)..(20): Xaa at position 20 is Aib
  MOD_RES (39)..(39): Ser at position 39 is amidated

SEQ ID NO: 128 - protein, 39 aa, Artificial Sequence
  Synthetic Construct
  MISC_FEATURE (2)..(2): Xaa at position 2 is Aib
  MISC_FEATURE (6)..(6): Xaa at position 6 is alpha-methyl-Phe
  MISC_FEATURE (13)..(13): Xaa at position 13 is alpha-methyl-Leu
  MOD_RES (17)..(17): Lys at position 17 is chemically modified by conjugation of the epsilon-amino group of the Lys side chain with (2-[2-(2-amino-ethoxy)-ethoxy]-acetyl)2-(gamma-Glu)-CO-(CH2)18-CO 2H
  MISC_FEATURE (20)..(20): Xaa at position 20 is Aib
  MOD_RES (39)..(39): Ser at position 39 is amidated
FXEGTXTSDYSIXLDEKAQXAFIEYLIEGGPSSGAPPPS

SEQ ID NO: 129 - protein, 39 aa, Artificial Sequence
  Synthetic Construct
  MISC_FEATURE (2)..(2): Xaa at position 2 is Aib
  MISC_FEATURE (3)..(3): Xaa at position 3 is cTA
  MISC_FEATURE (6)..(6): Xaa at position 6 is alpha-methyl-Phe
  MISC_FEATURE (13)..(13): Xaa at position 13 is alpha-methyl-Leu
  MOD_RES (17)..(17): Lys at position 17 is chemically modified by conjugation of the epsilon-amino group of the Lys side chain with (2-[2-(2-amino-ethoxy)-ethoxy]-acetyl)2-(gamma-Glu)-CO-(CH2)18-CO 2H
  MISC_FEATURE (20)..(20): Xaa at position 20 is Aib
  MOD_RES (39)..(39): Ser at position 39 is amidated
YXXGTXTSDYSIXLDEKAQXAFIEYLIEGGPSSGAPPPS

SEQ ID NO: 130 - protein, 39 aa, Artificial Sequence
  Synthetic Construct
  MISC_FEATURE (2)..(2): Xaa at position 2 is Aib
  MISC_FEATURE (6)..(6): Xaa at position 6 is alpha-methyl-Phe
  MISC_FEATURE (13)..(13): Xaa at position 13 is alpha-methyl-Leu
  MOD_RES (17)..(17): Lys at position 17 is chemically modified by conjugation of the epsilon-amino group of the Lys side chain with (2-[2-(2-amino-ethoxy)-ethoxy]-acetyl)2-(gamma-Glu)-CO-(CH2)18-CO 2H
  MOD_RES (39)..(39): Ser at position 39 is amidated
YXEGTXTSDYSIXLDEKAQQAFIEYLIEGGPSSGAPPPS

SEQ ID NO: 131 - protein, 39 aa, Artificial Sequence
  Synthetic Construct
  MISC_FEATURE (2)..(2): Xaa at position 2 is Aib
  MISC_FEATURE (6)..(6): Xaa at position 6 is alpha-methyl-Phe
  MISC_FEATURE (13)..(13): Xaa at position 13 is alpha-methyl-Leu
  MOD_RES (17)..(17): Lys at position 17 is chemically modified by conjugation of the epsilon-amino group of the Lys side chain with (2-[2-(2-amino-ethoxy)-ethoxy]-acetyl)2-(gamma-Glu)-CO-(CH2)18-CO 2H
  MISC_FEATURE (29)..(29): Xaa at position 29 is Aib
  MOD_RES (39)..(39): Ser at position 39 is amidated
YXEGTXTSDYSIXLDEKAQQAFIEYLIEXGPSSGAPPPS

SEQ ID NO: 132 - protein, 34 aa, Artificial Sequence
  Synthetic Construct
  MISC_FEATURE (2)..(2): Xaa at position 2 is Aib
  MISC_FEATURE (6)..(6): Xaa at position 6 is alpha-methyl-Phe
  MISC_FEATURE (13)..(13): Xaa at position 13 is alpha-methyl-Leu
  MOD_RES (17)..(17): Lys at position 17 is chemically modified by conjugation of the epsilon-amino group of the Lys side chain with (2-[2-(2-amino-ethoxy)-ethoxy]-acetyl)2-(gamma-Glu)-CO-(CH2)18-CO 2H
  MISC_FEATURE (20)..(20): Xaa at position 20 is Aib
  MOD_RES (34)..(34): Gly at position 34 is amidated
YXEGTXTSDYSIXLDKKAQXEFIEYLIEGGPSSG

SEQ ID NO: 133 - protein, 34 aa, Artificial Sequence
  Synthetic Construct
  MISC_FEATURE (2)..(2): Xaa at position 2 is Aib
  MISC_FEATURE (6)..(6): Xaa at position 6 is alpha-methyl-Phe
  MISC_FEATURE (13)..(13): Xaa at position 13 is alpha-methyl-Leu
  MOD_RES (17)..(17): Lys at position 17 is chemically modified by conjugation of the epsilon-amino group of the Lys side chain with (2-[2-(2-amino-ethoxy)-ethoxy]-acetyl)2-(gamma-Glu)-CO-(CH2)18-CO 2H
  MISC_FEATURE (20)..(20): Xaa at position 20 is Aib
  MOD_RES (34)..(34): Gly at position 34 is amidated
YXEGTXTSDYSIXLDEKAQXEFIEYLIEGGPSSG

SEQ ID NO: 134 - protein, 39 aa, Artificial Sequence; identical to SEQ ID NO: 78
  Synthetic Construct
  MISC_FEATURE (2)..(2): Xaa at position 2 is Aib
  MISC_FEATURE (6)..(6): Xaa at position 6 is alpha-methyl-Phe
  MISC_FEATURE (13)..(13): Xaa at position 13 is alpha-methyl-Leu
  MOD_RES (17)..(17): Lys at position 17 is chemically modified by conjugation of the epsilon-amino group of the Lys side chain with (2-[2-(2-amino-ethoxy)-ethoxy]-acetyl)2-(gamma-Glu)2-CO-(CH2)18-C O2H
  MISC_FEATURE (20)..(20): Xaa at position 20 is Aib
  MOD_RES (39)..(39): Ser at position 39 is amidated

SEQ ID NO: 135 - protein, 39 aa, Artificial Sequence
  Synthetic Construct
  MISC_FEATURE (2)..(2): Xaa at position 2 is Aib
  MISC_FEATURE (6)..(6): Xaa at position 6 is alpha-methyl-Phe
  MISC_FEATURE (13)..(13): Xaa at position 13 is alpha-methyl-Leu
  MOD_RES (17)..(17): Lys at position 17 is chemically modified by conjugation of the epsilon-amino group of the Lys side chain with (2-[2-(2-amino-ethoxy)-ethoxy]-acetyl)2-(gamma-Glu)-CO-(CH2)18-CO 2H
  MISC_FEATURE (20)..(20): Xaa at position 20 is Aib
  MOD_RES (39)..(39): Ser at position 39 is amidated
YXEGTXTSDYSIXLDKKAQXAFIEYLIEAGPSSGAPPPS

SEQ ID NO: 136 - protein, 39 aa, Artificial Sequence
  Synthetic Construct
  MISC_FEATURE (2)..(2): Xaa at position 2 is Aib
  MISC_FEATURE (6)..(6): Xaa at position 6 is alpha-methyl-Phe
  MOD_RES (17)..(17): Lys at position 17 is chemically modified by conjugation of the epsilon-amino group of the Lys side chain with (2-[2-(2-amino-ethoxy)-ethoxy]-acetyl)2-(gamma-Glu)-CO-(CH2)18-CO 2H
  MISC_FEATURE (20)..(20): Xaa at position 20 is Aib
  MOD_RES (39)..(39): Ser at position 39 is amidated
YXEGTXTSDISILLDKKAQXAFIEYLIEGGPSSGAPPPS

SEQ ID NO: 137 - protein, 39 aa, Artificial Sequence
  Synthetic Construct
  MISC_FEATURE (2)..(2): Xaa at position 2 is Aib
  MISC_FEATURE (6)..(6): Xaa at position 6 is alpha-methyl-Phe
  MOD_RES (17)..(17): Lys at position 17 is chemically modified by conjugation of the epsilon-amino group of the Lys side chain with (2-[2-(2-amino-ethoxy)-ethoxy]-acetyl)2-(gamma-Glu)-CO-(CH2)18-CO 2H
  MISC_FEATURE (20)..(20): Xaa at position 20 is Aib
  MOD_RES (39)..(39): Ser at position 39 is amidated
YXEGTXTSDHSILLDKKAQXAFIEYLIEGGPSSGAPPPS

SEQ ID NO: 138 - protein, 39 aa, Artificial Sequence
  Synthetic Construct
  MISC_FEATURE (2)..(2): Xaa at position 2 is Aib
  MISC_FEATURE (6)..(6): Xaa at position 6 is alpha-methyl-Phe
  MOD_RES (17)..(17): Lys at position 17 is chemically modified by conjugation of the epsilon-amino group of the Lys side chain with (2-[2-(2-amino-ethoxy)-ethoxy]-acetyl)2-(gamma-Glu)-CO-(CH2)18-CO 2H
  MISC_FEATURE (20)..(20): Xaa at position 20 is Aib
  MOD_RES (39)..(39): Ser at position 39 is amidated
YXEGTXTSDLSILLDKKAQXAFIEYLIEGGPSSGAPPPS

SEQ ID NO: 139 - protein, 39 aa, Artificial Sequence
  Synthetic Construct
  MISC_FEATURE (2)..(2): Xaa at position 2 is Aib
  MISC_FEATURE (6)..(6): Xaa at position 6 is alpha-methyl-Phe
  MOD_RES (17)..(17): Lys at position 17 is chemically modified by conjugation of the epsilon-amino group of the Lys side chain with (2-[2-(2-amino-ethoxy)-ethoxy]-acetyl)2-(gamma-Glu)-CO-(CH2)18-CO 2H
  MISC_FEATURE (20)..(20): Xaa at position 20 is Aib
  MOD_RES (39)..(39): Ser at position 39 is amidated
YXEGTXTSDESILLDKKAQXAFIEYLIEGGPSSGAPPPS

SEQ ID NO: 140 - protein, 39 aa, Artificial Sequence
  Synthetic Construct
  MISC_FEATURE (2)..(2): Xaa at position 2 is Aib
  MISC_FEATURE (6)..(6): Xaa at position 6 is alpha-methyl-Phe
  MISC_FEATURE (10)..(10): Xaa at position 10 is alpha-methyl-Phe
  MOD_RES (17)..(17): Lys at position 17 is chemically modified by conjugation of the epsilon-amino group of the Lys side chain with (2-[2-(2-amino-ethoxy)-ethoxy]-acetyl)2-(gamma-Glu)-CO-(CH2)18-CO 2H
  MISC_FEATURE (20)..(20): Xaa at position 20 is Aib
  MOD_RES (39)..(39): Ser at position 39 is amidated
YXEGTXTSDXSILLDKKAQXAFIEYLIEGGPSSGAPPPS

SEQ ID NO: 141 - protein, 39 aa, Artificial Sequence; identical to SEQ ID NO: 140
  Synthetic Construct
  MISC_FEATURE (2)..(2): Xaa at position 2 is Aib
  MISC_FEATURE (6)..(6): Xaa at position 6 is alpha-methyl-Phe
  MISC_FEATURE (10)..(10): Xaa at position 10 is 3Pal
  MOD_RES (17)..(17): Lys at position 17 is chemically modified by conjugation of the epsilon-amino group of the Lys side chain with (2-[2-(2-amino-ethoxy)-ethoxy]-acetyl)2-(gamma-Glu)-CO-(CH2)18-CO 2H
  MISC_FEATURE (20)..(20): Xaa at position 20 is Aib
  MOD_RES (39)..(39): Ser at position 39 is amidated

SEQ ID NO: 142 - protein, 39 aa, Artificial Sequence
  Synthetic Construct
  MISC_FEATURE (1)..(1): Xaa at position 1 is DesTyr
  MISC_FEATURE (2)..(2): Xaa at position 2 is Aib
  MISC_FEATURE (6)..(6): Xaa at position 6 is alpha-methyl-Phe
  MISC_FEATURE (13)..(13): Xaa at position 13 is Aib
  MOD_RES (17)..(17): Lys at position 17 is chemically modified by conjugation of the epsilon-amino group of the Lys side chain with (2-[2-(2-amino-ethoxy)-ethoxy]-acetyl)2-(gamma-Glu)-CO-(CH2)18-CO 2H
  MISC_FEATURE (20)..(20): Xaa at position 20 is Aib
  MOD_RES (39)..(39): Ser at position 39 is amidated
XXEGTXTSDYSIXLDEKAQXAFIEYLIEGGPSSGAPPPS

SEQ ID NO: 143 - protein, 39 aa, Artificial Sequence
  Synthetic Construct
  MISC_FEATURE (1)..(1): Xaa at position 1 is DesTyr
  MISC_FEATURE (2)..(2): Xaa at position 2 is Aib
  MISC_FEATURE (6)..(6): Xaa at position 6 is alpha-methyl-Phe(2F)
  MISC_FEATURE (13)..(13): Xaa at position 13 is alpha-methyl-Leu
  MOD_RES (17)..(17): Lys at position 17 is chemically modified by conjugation of the epsilon-amino group of the Lys side chain with (2-[2-(2-amino-ethoxy)-ethoxy]-acetyl)2-(gamma-Glu)-CO-(CH2)18-CO 2H
  MISC_FEATURE (20)..(20): Xaa at position 20 is Aib
  MOD_RES (39)..(39): Ser at position 39 is amidated
XXEGTXTSDYSIXLDEKAQXEFIEYLIEGGPSSGAPPPS

SEQ ID NO: 144 - protein, 39 aa, Artificial Sequence
  Synthetic Construct
  MISC_FEATURE (2)..(2): Xaa at position 2 is Aib
  MOD_RES (17)..(17): Lys at position 17 is chemically modified by conjugation of the epsilon-amino group of the Lys side chain with (2-[2-(2-amino-ethoxy)-ethoxy]-acetyl)2-(gamma-Glu)-CO-(CH2)18-CO 2H
  MISC_FEATURE (20)..(20): Xaa at position 20 is Aib
  MOD_RES (39)..(39): Ser at position 39 is amidated
HXNGTFTSDYSILLDKKAQXAFIEYLIEGGPSSGAPPPS

SEQ ID NO: 145 - protein, 39 aa, Artificial Sequence
  Synthetic Construct
  MISC_FEATURE (2)..(2): Xaa at position 2 is Aib
  MOD_RES (17)..(17): Lys at position 17 is chemically modified by conjugation of the epsilon-amino group of the Lys side chain with (2-[2-(2-amino-ethoxy)-ethoxy]-acetyl)2-(gamma-Glu)-CO-(CH2)18-CO 2H
  MISC_FEATURE (20)..(20): Xaa at position 20 is Aib
  MOD_RES (39)..(39): Ser at position 39 is amidated
YXEGTFTSDASILLDKKAQXAFIEYLIEAGPSSGAPPPS

SEQ ID NO: 146 - protein, 39 aa, Artificial Sequence
  Synthetic Construct
  MISC_FEATURE (2)..(2): Xaa at position 2 is Aib
  MISC_FEATURE (6)..(6): Xaa at position 6 is alpha-methyl-Phe
  MISC_FEATURE (13)..(13): Xaa at position 13 is alpha-methyl-Leu
  MOD_RES (17)..(17): Lys at position 17 is chemically modified by conjugation of the epsilon-amino group of the Lys side chain with (2-[2-(2-amino-ethoxy)-ethoxy]-acetyl)2-(gamma-Glu)-CO-(CH2)18-CO 2H
  MISC_FEATURE (20)..(20): Xaa at position 20 is Aib
  MISC_FEATURE (21)..(21): Xaa at position 21 is Aad
  MOD_RES (39)..(39): Ser at position 39 is amidated
YXEGTXTSDYSIXLDKKAQXXFIEYLIEGGPSSGAPPPS

SEQ ID NO: 147 - protein, 39 aa, Artificial Sequence
  Synthetic Construct
  MISC_FEATURE (2)..(2): Xaa at position 2 is Aib
  MISC_FEATURE (6)..(6): Xaa at position 6 is alpha-methyl-Phe
  MISC_FEATURE (13)..(13): Xaa at position 13 is alpha-methyl-Leu
  MOD_RES (17)..(17): Lys at position 17 is chemically modified by conjugation of the epsilon-amino group of the Lys side chain with (2-[2-(2-amino-ethoxy)-ethoxy]-acetyl)2-(gamma-Glu)-CO-(CH2)18-CO 2H
  MISC_FEATURE (20)..(20): Xaa at position 20 is Aib
  MOD_RES (39)..(39): Ser at position 39 is amidated
YXEGTXTSDYSIXLDKKAQXSFIEYLIEGGPSSGAPPPS

SEQ ID NO: 148 - protein, 39 aa, Artificial Sequence
  Synthetic Construct
  MISC_FEATURE (2)..(2): Xaa at position 2 is Aib
  MISC_FEATURE (6)..(6): Xaa at position 6 is alpha-methyl-Phe
  MISC_FEATURE (13)..(13): Xaa at position 13 is alpha-methyl-Leu
  MOD_RES (17)..(17): Lys at position 17 is chemically modified by conjugation of the epsilon-amino group of the Lys side chain with (2-[2-(2-amino-ethoxy)-ethoxy]-acetyl)2-(gamma-Glu)-CO-(CH2)18-CO 2H
  MISC_FEATURE (20)..(20): Xaa at position 20 is Aib
  MOD_RES (39)..(39): Ser at position 39 is amidated
YXEGTXTSDYSIXLDKKAQXTFIEYLIEGGPSSGAPPPS

SEQ ID NO: 149 - protein, 39 aa, Artificial Sequence
  Synthetic Construct
  MISC_FEATURE (2)..(2): Xaa at position 2 is Aib
  MISC_FEATURE (6)..(6): Xaa at position 6 is alpha-methyl-Phe
  MISC_FEATURE (13)..(13): Xaa at position 13 is alpha-methyl-Leu
  MOD_RES (17)..(17): Lys at position 17 is chemically modified by conjugation of the epsilon-amino group of the Lys side chain with (2-[2-(2-amino-ethoxy)-ethoxy]-acetyl)2-(gamma-Glu)-CO-(CH2)18-CO 2H
  MISC_FEATURE (20)..(20): Xaa at position 20 is Aib
  MOD_RES (39)..(39): Ser at position 39 is amidated
YXEGTXTSDYSIXLDKKAQXDFIEYLIEGGPSSGAPPPS

SEQ ID NO: 150 - protein, 39 aa, Artificial Sequence
  Synthetic Construct
  MISC_FEATURE (2)..(2): Xaa at position 2 is Aib
  MISC_FEATURE (6)..(6): Xaa at position 6 is alpha-methyl-Phe
  MISC_FEATURE (13)..(13): Xaa at position 13 is alpha-methyl-Leu
  MOD_RES (17)..(17): Lys at position 17 is chemically modified by conjugation of the epsilon-amino group of the Lys side chain with (2-[2-(2-amino-ethoxy)-ethoxy]-acetyl)2-(gamma-Glu)-CO-(CH2)18-CO 2H
  MISC_FEATURE (20)..(20): Xaa at position 20 is Aib
  MOD_RES (39)..(39): Ser at position 39 is amidated
YXEGTXTSDYSIXLDKKAQXIFIEYLIEGGPSSGAPPPS

SEQ ID NO: 151 - protein, 39 aa, Artificial Sequence
  Synthetic Construct
  MISC_FEATURE (2)..(2): Xaa at position 2 is Aib
  MISC_FEATURE (6)..(6): Xaa at position 6 is alpha-methyl-Phe
  MISC_FEATURE (13)..(13): Xaa at position 13 is alpha-methyl-Leu
  MOD_RES (17)..(17): Lys at position 17 is chemically modified by conjugation of the epsilon-amino group of the Lys side chain with (2-[2-(2-amino-ethoxy)-ethoxy]-acetyl)2-(gamma-Glu)-CO-(CH2)18-CO 2H
  MISC_FEATURE (20)..(20): Xaa at position 2 is Aib
  MOD_RES (39)..(39): Ser at position 39 is amidated
YXEGTXTSDYSIXLDKKAQXHFIEYLIEGGPSSGAPPPS

SEQ ID NO: 152 - protein, 39 aa, Artificial Sequence; identical to SEQ ID NO: 146
  Synthetic Construct
  MISC_FEATURE (2)..(2): Xaa at position 2 is Aib
  MISC_FEATURE (6)..(6): Xaa at position 6 is alpha-methyl-Phe
  MISC_FEATURE (13)..(13): Xaa at position 13 is alpha-methyl-Leu
  MOD_RES (17)..(17): Lys at position 17 is chemically modified by conjugation of the epsilon-amino group of the Lys side chain with (2-[2-(2-amino-ethoxy)-ethoxy]-acetyl)2-(gamma-Glu)-CO-(CH2)18-CO 2H
  MISC_FEATURE (20)..(20): Xaa at position 20 is Aib
  MISC_FEATURE (21)..(21): Xaa at position 21 is Aib
  MOD_RES (39)..(39): Ser at position 39 is amidated

SEQ ID NO: 153 - protein, 39 aa, Artificial Sequence
  Synthetic Construct
  MISC_FEATURE (2)..(2): Xaa at position 2 is Aib
  MISC_FEATURE (6)..(6): Xaa at position 6 is alpha-methyl-Phe
  MISC_FEATURE (13)..(13): Xaa at position 13 is alpha-methyl-Leu
  MOD_RES (17)..(17): Lys at position 17 is chemically modified by conjugation of the epsilon-amino group of the Lys side chain with (2-[2-(2-amino-ethoxy)-ethoxy]-acetyl)2-(gamma-Glu)-CO-(CH2)18-CO 2H
  MISC_FEATURE (21)..(21): Xaa at position 21 is Aib
  MOD_RES (39)..(39): Ser at position 39 is amidated
YXEGTXTSDYSIXLDKKAQHXFIEYLIEGGPSSGAPPPS

SEQ ID NO: 154 - protein, 39 aa, Artificial Sequence
  Synthetic Construct
  MISC_FEATURE (2)..(2): Xaa at position 2 is Aib
  MISC_FEATURE (6)..(6): Xaa at position 6 is alpha-methyl-Phe
  MISC_FEATURE (13)..(13): Xaa at position 13 is alpha-methyl-Leu
  MOD_RES (17)..(17): Lys at position 17 is chemically modified by conjugation of the epsilon-amino group of the Lys side chain with (2-[2-(2-amino-ethoxy)-ethoxy]-acetyl)2-(gamma-Glu)-CO-(CH2)18-CO 2H
  MISC_FEATURE (20)..(20): Xaa at position 20 is Aib
  MOD_RES (39)..(39): Ser at position 39 is amidated
YXEGTXTSDASIXLDKKAQXAFIEYLIEGGPSSGAPPPS

SEQ ID NO: 155 - protein, 39 aa, Artificial Sequence
  Synthetic Construct
  MISC_FEATURE (2)..(2): Xaa at position 2 is Aib
  MISC_FEATURE (6)..(6): Xaa at position 6 is alpha-methyl-Phe(2F)
  MISC_FEATURE (13)..(13): Xaa at position 13 is alpha-methyl-Leu
  MOD_RES (17)..(17): Lys at position 17 is chemically modified by conjugation of the epsilon-amino group of the Lys side chain with (2-[2-(2-amino-ethoxy)-ethoxy]-acetyl)2-(gamma-Glu)-CO-(CH2)18-CO 2H
  MISC_FEATURE (20)..(20): Xaa at position 20 is Aib
  MOD_RES (39)..(39): Ser at position 39 is amidated
YXEGTXTSDYSIXLDEKAQXEFIQYLIEGGPSSGAPPPS

SEQ ID NO: 156 - protein, 39 aa, Artificial Sequence; identical to SEQ ID NO: 10
  Synthetic Construct
  MISC_FEATURE (2)..(2): Xaa at position 2 is Aib
  MISC_FEATURE (6)..(6): Xaa at position 6 is alpha-methyl-Phe(2F)
  MISC_FEATURE (13)..(13): Xaa at position 13 is alpha-methyl-Leu
  MOD_RES (17)..(17): Lys at position 17 is chemically modified by conjugation of the epsilon-amino group of the Lys side chain with (2-[2-(2-amino-ethoxy)-ethoxy]-acetyl)2-(gamma-Glu)-CO-(CH2)18-CO 2H
  MISC_FEATURE (20)..(20): Xaa at position 20 is Aib
  MISC_FEATURE (24)..(24): Xaa at position 24 is Aad
  MOD_RES (39)..(39): Ser at position 39 is amidated

SEQ ID NO: 157 - protein, 39 aa, Artificial Sequence
  Synthetic Construct
  MISC_FEATURE (2)..(2): Xaa at position 2 is Aib
  MISC_FEATURE (6)..(6): Xaa at position 6 is alpha-methyl-Phe(2F)
  MISC_FEATURE (13)..(13): Xaa at position 13 is alpha-methyl-Leu
  MOD_RES (17)..(17): Lys at position 17 is chemically modified by conjugation of the epsilon-amino group of the Lys side chain with (2-[2-(2-amino-ethoxy)-ethoxy]-acetyl)2-(gamma-Glu)-CO-(CH2)18-CO 2H
  MISC_FEATURE (20)..(20): Xaa at position 20 is Aib
  MOD_RES (39)..(39): Ser at position 39 is amidated
YXEGTXTSDYSIXLDEKAQXEFIAYLIEGGPSSGAPPPS

SEQ ID NO: 158 - protein, 39 aa, Artificial Sequence
  Synthetic Construct
  MISC_FEATURE (2)..(2): Xaa at position 2 is Aib
  MISC_FEATURE (6)..(6): Xaa at position 6 is alpha-methyl-Phe(2F)
  MISC_FEATURE (13)..(13): Xaa at position 13 is alpha-methyl-Leu
  MOD_RES (17)..(17): Lys at position 17 is chemically modified by conjugation of the epsilon-amino group of the Lys side chain with (2-[2-(2-amino-ethoxy)-ethoxy]-acetyl)2-(gamma-Glu)-CO-(CH2)18-CO 2H
  MISC_FEATURE (20)..(20): Xaa at position 20 is Aib
  MOD_RES (39)..(39): Ser at position 39 is amidated
YXEGTXTSDYSIXLDEKAQXEFIVYLIEGGPSSGAPPPS

SEQ ID NO: 159 - protein, 39 aa, Artificial Sequence
  Synthetic Construct
  MISC_FEATURE (2)..(2): Xaa at position 2 is Aib
  MISC_FEATURE (6)..(6): Xaa at position 6 is alpha-methyl-Phe(2F)
  MISC_FEATURE (13)..(13): Xaa at position 13 is alpha-methyl-Leu
  MOD_RES (17)..(17): Lys at position 17 is chemically modified by conjugation of the epsilon-amino group of the Lys side chain with (2-[2-(2-amino-ethoxy)-ethoxy]-acetyl)2-(gamma-Glu)-CO-(CH2)18-CO 2H
  MISC_FEATURE (20)..(20): Xaa at position 20 is Aib
  MOD_RES (39)..(39): Ser at position 39 is amidated
YXEGTXTSDYSIXLDEKAQXEFISYLIEGGPSSGAPPPS

SEQ ID NO: 160 - protein, 39 aa, Artificial Sequence
  Synthetic Construct
  MISC_FEATURE (2)..(2): Xaa at position 2 is Aib
  MISC_FEATURE (6)..(6): Xaa at position 6 is alpha-methyl-Phe(2F)
  MISC_FEATURE (13)..(13): Xaa at position 13 is alpha-methyl-Leu
  MOD_RES (17)..(17): Lys at position 17 is chemically modified by conjugation of the epsilon-amino group of the Lys side chain with (2-[2-(2-amino-ethoxy)-ethoxy]-acetyl)2-(gamma-Glu)-CO-(CH2)18-CO 2H
  MISC_FEATURE (20)..(20): Xaa at position 20 is Aib
  MOD_RES (39)..(39): Ser at position 39 is amidated
YXEGTXTSDYSIXLDEKAQXEFIPYLIEGGPSSGAPPPS

SEQ ID NO: 161 - protein, 39 aa, Artificial Sequence; identical to SEQ ID NO: 10
  Synthetic Construct
  MISC_FEATURE (2)..(2): Xaa at position 2 is Aib
  MISC_FEATURE (6)..(6): Xaa at position 6 is alpha-methyl-Phe(2F)
  MISC_FEATURE (13)..(13): Xaa at position 13 is alpha-methyl-Leu
  MOD_RES (17)..(17): Lys at position 17 is chemically modified by conjugation of the epsilon-amino group of the Lys side chain with (2-[2-(2-amino-ethoxy)-ethoxy]-acetyl)2-(gamma-Glu)-CO-(CH2)18-CO 2H
  MISC_FEATURE (20)..(20): Xaa at position 20 is Aib
  MISC_FEATURE (24)..(24): Xaa at position 24 is Aib
  MOD_RES (39)..(39): Ser at position 39 is amidated

SEQ ID NO: 162 - protein, 39 aa, Artificial Sequence
  Synthetic Construct
  MISC_FEATURE (2)..(2): Xaa at position 2 is Aib
  MISC_FEATURE (6)..(6): Xaa at position 6 is alpha-methyl-Phe(2F)
  MISC_FEATURE (13)..(13): Xaa at position 13 is alpha-methyl-Leu
  MOD_RES (17)..(17): Lys at position 17 is chemically modified by conjugation of the epsilon-amino group of the Lys side chain with (2-[2-(2-amino-ethoxy)-ethoxy]-acetyl)2-(gamma-Glu)-CO-(CH2)18-CO 2H
  MISC_FEATURE (20)..(20): Xaa at position 20 is Aib
  MOD_RES (39)..(39): Ser at position 39 is amidated
YXEGTXTSDYSIXLDEKAQXEFIHYLIEGGPSSGAPPPS

SEQ ID NO: 163 - protein, 39 aa, Artificial Sequence
  Synthetic Construct
  MISC_FEATURE (2)..(2): Xaa at position 2 is Aib
  MISC_FEATURE (6)..(6): Xaa at position 6 is alpha-methyl-Phe(2F)
  MISC_FEATURE (13)..(13): Xaa at position 13 is alpha-methyl-Leu
  MOD_RES (17)..(17): Lys at position 17 is chemically modified by conjugation of the epsilon-amino group of the Lys side chain with (2-[2-(2-amino-ethoxy)-ethoxy]-acetyl)2-(gamma-Glu)-CO-(CH2)18-CO 2H
  MISC_FEATURE (20)..(20): Xaa at position 20 is Aib
  MOD_RES (39)..(39): Ser at position 39 is amidated
YXEGTXTSDHSIXLDEKAQXEFIEYLIEGGPSSGAPPPS

SEQ ID NO: 164 - protein, 39 aa, Artificial Sequence
  Synthetic Construct
  MISC_FEATURE (2)..(2): Xaa at position 2 is Aib
  MISC_FEATURE (6)..(6): Xaa at position 6 is alpha-methyl-Phe(2F)
  MISC_FEATURE (10)..(10): Xaa at position 10 is cTA
  MISC_FEATURE (13)..(13): Xaa at position 13 is alpha-methyl-Leu
  MOD_RES (17)..(17): Lys at position 17 is chemically modified by conjugation of the epsilon-amino group of the Lys side chain with (2-[2-(2-amino-ethoxy)-ethoxy]-acetyl)2-(gamma-Glu)-CO-(CH2)18-CO 2H
  MISC_FEATURE (20)..(20): Xaa at position 20 is Aib
  MOD_RES (39)..(39): Ser at position 39 is amidated
YXEGTXTSDXSIXLDEKAQXEFIEYLIEGGPSSGAPPPS

SEQ ID NO: 165 - protein, 39 aa, Artificial Sequence; identical to SEQ ID NO: 164
  Synthetic Construct
  MISC_FEATURE (2)..(2): Xaa at position 2 is Aib
  MISC_FEATURE (6)..(6): Xaa at position 6 is alpha-methyl-Phe(2F)
  MISC_FEATURE (10)..(10): Xaa at position 10 is 2Pal
  MISC_FEATURE (13)..(13): Xaa at position 13 is alpha-methyl-Leu
  MOD_RES (17)..(17): Lys at position 17 is chemically modified by conjugation of the epsilon-amino group of the Lys side chain with (2-[2-(2-amino-ethoxy)-ethoxy]-acetyl)2-(gamma-Glu)-CO-(CH2)18-CO 2H
  MISC_FEATURE (20)..(20): Xaa at position 20 is Aib
  MOD_RES (39)..(39): Ser at position 39 is amidated

SEQ ID NO: 166 - protein, 39 aa, Artificial Sequence; identical to SEQ ID NO: 164
  Synthetic Construct
  MISC_FEATURE (2)..(2): Xaa at position 2 is Aib
  MISC_FEATURE (6)..(6): Xaa at position 6 is alpha-methyl-Phe(2F)
  MISC_FEATURE (10)..(10): Xaa at position 10 is 3Pal
  MISC_FEATURE (13)..(13): Xaa at position 13 is alpha-methyl-Leu
  MOD_RES (17)..(17): Lys at position 17 is chemically modified by conjugation of the epsilon-amino group of the Lys side chain with (2-[2-(2-amino-ethoxy)-ethoxy]-acetyl)2-(gamma-Glu)-CO-(CH2)18-CO 2H
  MISC_FEATURE (20)..(20): Xaa at position 20 is Aib
  MOD_RES (39)..(39): Ser at position 39 is amidated

SEQ ID NO: 167 - protein, 39 aa, Artificial Sequence; identical to SEQ ID NO: 164
  Synthetic Construct
  MISC_FEATURE (2)..(2): Xaa at position 2 is Aib
  MISC_FEATURE (6)..(6): Xaa at position 6 is alpha-methyl-Phe(2F)
  MISC_FEATURE (10)..(10): Xaa at position 10 is 4Pal
  MISC_FEATURE (13)..(13): Xaa at position 13 is alpha-methyl-Leu
  MOD_RES (17)..(17): Lys at position 17 is chemically modified by conjugation of the epsilon-amino group of the Lys side chain with (2-[2-(2-amino-ethoxy)-ethoxy]-acetyl)2-(gamma-Glu)-CO-(CH2)18-CO 2H
  MISC_FEATURE (20)..(20): Xaa at position 20 is Aib
  MOD_RES (39)..(39): Ser at position 39 is amidated

SEQ ID NO: 168 - protein, 39 aa, Artificial Sequence; identical to SEQ ID NO: 164
  Synthetic Construct
  MISC_FEATURE (2)..(2): Xaa at position 2 is Aib
  MISC_FEATURE (6)..(6): Xaa at position 6 is alpha-methyl-Phe(2F)
  MISC_FEATURE (10)..(10): Xaa at position 10 is alpha-methyl-Phe
  MISC_FEATURE (13)..(13): Xaa at position 13 is alpha-methyl-Leu
  MOD_RES (17)..(17): Lys at position 17 is chemically modified by conjugation of the epsilon-amino group of the Lys side chain with (2-[2-(2-amino-ethoxy)-ethoxy]-acetyl)2-(gamma-Glu)-CO-(CH2)18-CO 2H
  MISC_FEATURE (20)..(20): Xaa at position 20 is Aib
  MOD_RES (39)..(39): Ser at position 39 is amidated

SEQ ID NO: 169 - protein, 39 aa, Artificial Sequence
  Synthetic Construct
  MISC_FEATURE (2)..(2): Xaa at position 2 is Aib
  MISC_FEATURE (6)..(6): Xaa at position 6 is alpha-methyl-Phe(2F)
  MISC_FEATURE (10)..(10): Xaa at position 10 is Aib
  MISC_FEATURE (13)..(13): Xaa at position 13 is alpha-methyl-Leu
  MOD_RES (17)..(17): Lys at position 17 is chemically modified by conjugation of the epsilon-amino group of the Lys side chain with (2-[2-(2-amino-ethoxy)-ethoxy]-acetyl)2-(gamma-Glu)-CO-(CH2)18-CO 2H
  MISC_FEATURE (20)..(20): Xaa at position 20 is Aib
  MISC_FEATURE (24)..(24): Xaa at position 24 is D-Glu
  MOD_RES (39)..(39): Ser at position 39 is amidated
YXEGTXTSDXSIXLDEKAQXTFIXYLIEGGPSSGAPPPS

SEQ ID NO: 170 - protein, 34 aa, Artificial Sequence
  Synthetic Construct
  MISC_FEATURE (2)..(2): Xaa at position 2 is Aib
  MISC_FEATURE (6)..(6): Xaa at position 6 is alpha-methyl-Phe(2F)
  MISC_FEATURE (13)..(13): Xaa at position 13 is alpha-methyl-Leu
  MOD_RES (17)..(17): Lys at position 17 is chemically modified by conjugation of the epsilon-amino group of the Lys side chain with (2-[2-(2-amino-ethoxy)-ethoxy]-acetyl)2-(gamma-Glu)2-CO-(CH2)18-C O2H
  MISC_FEATURE (20)..(20): Xaa at position 20 is Aib
  MISC_FEATURE (24)..(24): Xaa at position 24 is D-Glu
  MOD_RES (34)..(34): Gly at position 34 is amidated
YXEGTXTSDHSIXLDEKAQXTFIXYLIEGGPSSG

SEQ ID NO: 171 - protein, 34 aa, Artificial Sequence
  Synthetic Construct
  MISC_FEATURE (2)..(2): Xaa at position 2 is Aib
  MISC_FEATURE (6)..(6): Xaa at position 6 is alpha-methyl-Phe(2F)
  MISC_FEATURE (13)..(13): Xaa at position 13 is alpha-methyl-Leu
  MOD_RES (17)..(17): Lys at position 17 is chemically modified by conjugation of the epsilon-amino group of the Lys side chain with (2-[2-(2-amino-ethoxy)-ethoxy]-acetyl)2-(gamma-Glu)2-CO-(CH2)18-C O2H
  MISC_FEATURE (20)..(20): Xaa at position 20 is Aib
  MISC_FEATURE (24)..(24): Xaa at position 24 is D-Glu
  MOD_RES (34)..(34): Gly at position 34 is amidated
YXEGTXTSDHSIXLDEKAQXTFIXHLIEGGPSSG

SEQ ID NO: 172 - protein, 39 aa, Artificial Sequence
  Synthetic Construct
  MISC_FEATURE (2)..(2): Xaa at position 2 is Aib
  MISC_FEATURE (6)..(6): Xaa at position 6 is alpha-methyl-Phe(2F)
  MISC_FEATURE (13)..(13): Xaa at position 13 is alpha-methyl-Leu
  MOD_RES (17)..(17): Lys at position 17 is chemically modified by conjugation of the epsilon-amino group of the Lys side chain with (2-[2-(2-amino-ethoxy)-ethoxy]-acetyl)2-(gamma-Glu)-CO-(CH2)18-CO 2H
  MISC_FEATURE (20)..(20): Xaa at position 20 is Aib
  MOD_RES (39)..(39): Ser at position 39 is amidated
HXEGTXTSDYSIXLDEKAQXEFIEYLIEGGPSSGAPPPS

SEQ ID NO: 173 - protein, 39 aa, Artificial Sequence
  Synthetic Construct
  MISC_FEATURE (2)..(2): Xaa at position 2 is Aib
  MISC_FEATURE (6)..(6): Xaa at position 6 is alpha-methyl-Phe(2F)
  MISC_FEATURE (13)..(13): Xaa at position 13 is alpha-methyl-Leu
  MOD_RES (17)..(17): Lys at position 17 is chemically modified by conjugation of the epsilon-amino group of the Lys side chain with (2-[2-(2-amino-ethoxy)-ethoxy]-acetyl)2-(gamma-Glu)-CO-(CH2)18-CO 2H
  MISC_FEATURE (20)..(20): Xaa at position 20 is Aib
  MISC_FEATURE (24)..(24): Xaa at position 24 is D-Glu
  MISC_FEATURE (28)..(28): Xaa at position 28 is D-Glu
  MOD_RES (39)..(39): Ser at position 39 is amidated
YXEGTXTSDHSIXLDEKAQXTFIXYLIXGGPSSGAPPPS

SEQ ID NO: 174 - protein, 39 aa, Artificial Sequence
  Synthetic Construct
  MISC_FEATURE (2)..(2): Xaa at position 2 is Aib
  MISC_FEATURE (6)..(6): Xaa at position 6 is alpha-methyl-Phe(2F)
  MISC_FEATURE (13)..(13): Xaa at position 13 is alpha-methyl-Leu
  MOD_RES (17)..(17): Lys at position 17 is chemically modified by conjugation of the epsilon-amino group of the Lys side chain with (2-[2-(2-amino-ethoxy)-ethoxy]-acetyl)2-(gamma-Glu)-CO-(CH2)18-CO 2H
  MISC_FEATURE (20)..(20): Xaa at position 20 is Aib
  MISC_FEATURE (24)..(24): Xaa at position 24 is D-Glu
  MISC_FEATURE (25)..(25): Xaa at position 25 is alpha-methyl-Phe
  MISC_FEATURE (28)..(28): Xaa at position 28 is D-Glu
  MOD_RES (39)..(39): Ser at position 39 is amidated
YXEGTXTSDHSIXLDEKAQXTFIXXLIXGGPSSGAPPPS

SEQ ID NO: 175 - protein, 30 aa, Artificial Sequence
  Synthetic Construct
  MISC_FEATURE (2)..(2): Xaa at position 2 is Aib
  MISC_FEATURE (6)..(6): Xaa at position 6 is alpha-methyl-Phe(2F)
  MISC_FEATURE (13)..(13): Xaa at position 13 is alpha-methyl-Leu
  MOD_RES (17)..(17): Lys at position 17 is chemically modified by conjugation of the epsilon-amino group of the Lys side chain with (2-[2-(2-amino-ethoxy)-ethoxy]-acetyl)2-(gamma-Glu)-CO-(CH2)18-CO 2H
  MISC_FEATURE (20)..(20): Xaa at position 20 is Aib
  MISC_FEATURE (24)..(24): Xaa at position 24 is D-Glu
  MOD_RES (30)..(30)
YXEGTXTSDHSIXLDEKAQXTFIXYLIEGG

SEQ ID NO: 176 - protein, 34 aa, Artificial Sequence; identical to SEQ ID NO: 170
  Synthetic Construct
  MISC_FEATURE (2)..(2): Xaa at position 2 is Aib
  MISC_FEATURE (6)..(6): Xaa at position 6 is alpha-methyl-Phe(2F)
  MISC_FEATURE (13)..(13): Xaa at position 13 is alpha-methyl-Leu
  MOD_RES (17)..(17): Lys at position 17 is chemically modified by conjugation of the epsilon-amino group of the Lys side chain with (2-[2-(2-amino-ethoxy)-ethoxy]-acetyl)2-(gamma-Glu)-CO-(CH2)18-CO 2H
  MISC_FEATURE (20)..(20): Xaa at position 20 is Aib
  MISC_FEATURE (24)..(24): Xaa at position 24 is D-Glu
  MOD_RES (34)..(34): Gly at position 34 is amidated

SEQ ID NO: 177 - protein, 39 aa, Artificial Sequence
  Synthetic Construct
  MISC_FEATURE (2)..(2): Xaa at position 2 is Aib
  MISC_FEATURE (6)..(6): Xaa at position 6 is alpha-methyl-Phe(2F)
  MISC_FEATURE (13)..(13): Xaa at position 13 is alpha-methyl-Leu
  MOD_RES (17)..(17): Lys at position 17 is chemically modified by conjugation of the epsilon-amino group of the Lys side chain with (2-[2-(2-amino-ethoxy)-ethoxy]-acetyl)2-(gamma-Glu)-CO-(CH2)18-CO 2H
  MISC_FEATURE (20)..(20): Xaa at position 20 is Aib
  MISC_FEATURE (24)..(24): Xaa at position 24 is D-Glu
  MOD_RES (39)..(39): Ser at position 39 is amidated
YXEGTXTSDHSIXLDEKAQXTFIXYLIEGGPSSGAPPPS

SEQ ID NO: 178 - protein, 39 aa, Artificial Sequence; identical to SEQ ID NO: 177
  Synthetic Construct
  MISC_FEATURE (2)..(2): Xaa at position 2 is Aib
  MISC_FEATURE (6)..(6): Xaa at position 6 is alpha-methyl-Phe(2F)
  MISC_FEATURE (13)..(13): Xaa at position 13 is alpha-methyl-Leu
  MOD_RES (17)..(17): Lys at position 17 is chemically modified by conjugation of the epsilon-amino group of the Lys side chain with (2-[2-(2-amino-ethoxy)-ethoxy]-acetyl)2-(gamma-Glu)-CO-(CH2)16-CO 2H
  MISC_FEATURE (20)..(20): Xaa at position 20 is Aib
  MISC_FEATURE (24)..(24): Xaa at position 24 is D-Glu
  MOD_RES (39)..(39): Ser at position 39 is amidated

SEQ ID NO: 179 - protein, 39 aa, Artificial Sequence; identical to SEQ ID NO: 177
  Synthetic Construct
  MISC_FEATURE (2)..(2): Xaa at position 2 is Aib
  MISC_FEATURE (6)..(6): Xaa at position 6 is alpha-methyl-Phe(2F)
  MISC_FEATURE (13)..(13): Xaa at position 13 is alpha-methyl-Leu
  MOD_RES (17)..(17): Lys at position 17 is chemically modified by conjugation of the epsilon-amino group of the Lys side chain with (2-[2-(2-amino-ethoxy)-ethoxy]-acetyl)2-(gamma-Glu)-CO-(CH2)14-CO 2H
  MISC_FEATURE (20)..(20): Xaa at position 20 is Aib
  MISC_FEATURE (24)..(24): Xaa at position 24 is D-Glu
  MOD_RES (39)..(39): Ser at position 39 is amidated

SEQ ID NO: 180 - protein, 39 aa, Artificial Sequence
  Synthetic Construct
  MISC_FEATURE (2)..(2): Xaa at position 2 is Aib
  MISC_FEATURE (6)..(6): Xaa at position 6 is alpha-methyl-Phe(2F)
  MISC_FEATURE (13)..(13): Xaa at position 13 is alpha-methyl-Leu
  MISC_FEATURE (16)..(16): Xaa at position 16 is Orn
  MOD_RES (17)..(17): Lys at position 17 is chemically modified by conjugation of the epsilon-amino group of the Lys side chain with (2-[2-(2-amino-ethoxy)-ethoxy]-acetyl)2-(gamma-Glu)-CO-(CH2)18-CO 2H
  MISC_FEATURE (20)..(20): Xaa at position 20 is Aib
  MISC_FEATURE (24)..(24): Xaa at position 24 is D-Glu
  MOD_RES (39)..(39): Ser at position 39 is amidated
YXEGTXTSDHSIXLDXKAQXTFIXYLIEGGPSSGAPPPS

SEQ ID NO: 181 - protein, 39 aa, Artificial Sequence; identical to SEQ ID NO: 180
  Synthetic Construct
  MISC_FEATURE (2)..(2): Xaa at position 2 is Aib
  MISC_FEATURE (6)..(6): Xaa at position 6 is alpha-methyl-Phe(2F)
  MISC_FEATURE (13)..(13): Xaa at position 13 is alpha-methyl-Leu
  MISC_FEATURE (16)..(16): Xaa at position 16 is Dab
  MOD_RES (17)..(17): Lys at position 17 is chemically modified by conjugation of the epsilon-amino group of the Lys side chain with (2-[2-(2-amino-ethoxy)-ethoxy]-acetyl)2-(gamma-Glu)-CO-(CH2)18-CO 2H
  MISC_FEATURE (20)..(20): Xaa at position 20 is a Aib
  MISC_FEATURE (24)..(24): Xaa at position 24 is D-Glu
  MOD_RES (39)..(39): Ser at position 39 is amidated

SEQ ID NO: 182 - protein, 39 aa, Artificial Sequence; identical to SEQ ID NO: 180
  Synthetic Construct
  MISC_FEATURE (2)..(2): Xaa at position 2 is Aib
  MISC_FEATURE (6)..(6): Xaa at position 6 is alpha-methyl-Phe(2F)
  MISC_FEATURE (13)..(13): Xaa at position 13 is alpha-methyl-Leu
  MISC_FEATURE (16)..(16): Xaa at position 16 is Dap
  MOD_RES (17)..(17): Lys at position 17 is chemically modified by conjugation of the epsilon-amino group of the Lys side chain with (2-[2-(2-amino-ethoxy)-ethoxy]-acetyl)2-(gamma-Glu)-CO-(CH2)18-CO 2H
  MISC_FEATURE (20)..(20): Xaa at position 20 is Aib
  MISC_FEATURE (24)..(24): Xaa at position 24 is D-Glu
  MOD_RES (39)..(39): Ser at position 39 is amidated

SEQ ID NO: 183 - protein, 39 aa, Artificial Sequence; identical to SEQ ID NO: 177
  Synthetic Construct
  MISC_FEATURE (2)..(2): Xaa at position 2 is Aib
  MISC_FEATURE (6)..(6): Xaa at position 6 is alpha-methyl-Phe(2F)
  MISC_FEATURE (13)..(13): Xaa at position 13 is alpha-methyl-Leu
  MOD_RES (17)..(17): Lys at position 17 is chemically modified by conjugation of the epsilon-amino group of the Lys side chain with (2-[2-(2-amino-ethoxy)-ethoxy]-acetyl)2-CO-(CH2)18-CO2H
  MISC_FEATURE (20)..(20): Xaa at position 20 is Aib
  MISC_FEATURE (24)..(24): Xaa at position 24 is D-Glu
  MOD_RES (39)..(39): Ser at position 39 is amidated

SEQ ID NO: 184 - protein, 39 aa, Artificial Sequence; identical to SEQ ID NO: 177
  Synthetic Construct
  MISC_FEATURE (2)..(2): Xaa at position 2 is Aib
  MISC_FEATURE (6)..(6): Xaa at position 6 is alpha-methyl-Phe(2F)
  MISC_FEATURE (13)..(13): Xaa at position 13 is alpha-methyl-Leu
  MOD_RES (17)..(17): Lys at position 17 is chemically modified by conjugation of the epsilon-amino group of the Lys side chain with (2-[2-(2-amino-ethoxy)-ethoxy]-acetyl)2-(epsilon-Lys)-CO-(CH2)18- CO2H
  MISC_FEATURE (20)..(20): Xaa at position 20 is Aib
  MISC_FEATURE (24)..(24): Xaa at position 24 is D-Glu
  MOD_RES (39)..(39): Ser at position 39 is amidated

SEQ ID NO: 185 - protein, 39 aa, Artificial Sequence; identical to SEQ ID NO: 177
  Synthetic Construct
  MISC_FEATURE (2)..(2): Xaa at position 2 is Aib
  MISC_FEATURE (6)..(6): Xaa at position 6 is alpha-methyl-Phe(2F)
  MISC_FEATURE (13)..(13): Xaa at position 13 is alpha-methyl-Leu
  MOD_RES (17)..(17): Lys at position 17 is chemically modified by conjugation of the epsilon-amino group of the Lys side chain with (2-[2-(2-amino-ethoxy)-ethoxy]-acetyl)2-(epsilon-Lys)-CO-(CH2)16- CO2H
  MISC_FEATURE (20)..(20): Xaa at position 20 is Aib
  MISC_FEATURE (24)..(24): Xaa at position 24 is D-Glu
  MOD_RES (39)..(39): Ser at position 39 is amidated

SEQ ID NO: 186 - protein, 39 aa, Artificial Sequence
  Synthetic Construct
  MISC_FEATURE (2)..(2): Xaa at position 2 is Aib
  MISC_FEATURE (6)..(6): Xaa at position 6 is alpha-methyl-Phe(2F)
  MISC_FEATURE (13)..(13): Xaa at position 13 is alpha-methyl-Leu
  MOD_RES (17)..(17): Lys at position 17 is chemically modified by conjugation of the epsilon-amino group of the Lys side chain with (2-[2-(2-amino-ethoxy)-ethoxy]-acetyl)2-(gamma-Glu)-CO-(CH2)16-CO 2H
  MISC_FEATURE (20)..(20): Xaa at position 20 is Aib
  MISC_FEATURE (24)..(24): Xaa at position 24 is D-Glu
  MOD_RES (39)..(39): Ser at position 39 is amidated
YXEGTXTSDHSIXLDEKAQXHFIXYLIEGGPSSGAPPPS

SEQ ID NO: 187 - protein, 39 aa, Artificial Sequence; identical to SEQ ID NO: 186
  Synthetic Construct
  MISC_FEATURE (2)..(2): Xaa at position 2 is Aib
  MISC_FEATURE (6)..(6): Xaa at position 6 is alpha-methyl-Phe(2F)
  MISC_FEATURE (13)..(13): Xaa at position 13 is alpha-methyl-Leu
  MOD_RES (17)..(17): Lys at position 17 is chemically modified by conjugation of the epsilon-amino group of the Lys side chain with (2-[2-(2-amino-ethoxy)-ethoxy]-acetyl)2-(gamma-Glu)-CO-(CH2)14-CO 2H
  MISC_FEATURE (20)..(20): Xaa at position 20 is Aib
  MISC_FEATURE (24)..(24): Xaa at position 24 is D-Glu
  MOD_RES (39)..(39): Ser at position 39 is amidated

SEQ ID NO: 188 - protein, 34 aa, Artificial Sequence
  Synthetic Construct
  MISC_FEATURE (2)..(2): Xaa at position 2 is Aib
  MISC_FEATURE (6)..(6): Xaa at position 6 is alpha-methyl-Phe(2F)
  MISC_FEATURE (13)..(13): Xaa at position 13 is alpha-methyl-Leu
  MOD_RES (17)..(17): Lys at position 17 is chemically modified by conjugation of the epsilon-amino group of the Lys side chain with (2-[2-(2-amino-ethoxy)-ethoxy]-acetyl)2-(gamma-Glu)-CO-(CH2)16-CO 2H
  MISC_FEATURE (20)..(20): Xaa at position 20 is Aib
  MISC_FEATURE (24)..(24): Xaa at position 24 is D-Glu
  MOD_RES (34)..(34): Gly at position 34 is amidated
YXEGTXTSDHSIXLDEKAQXHFIXYLIEGGPSSG

SEQ ID NO: 189 - protein, 30 aa, Artificial Sequence
  Synthetic Construct
  MISC_FEATURE (2)..(2): Xaa at position 2 is Aib
  MISC_FEATURE (6)..(6): Xaa at position 6 is alpha-methyl-Phe(2F)
  MISC_FEATURE (13)..(13): Xaa at position 13 is alpha-methyl-Leu
  MOD_RES (17)..(17): Lys at position 17 is chemically modified by conjugation of the epsilon-amino group of the Lys side chain with (2-[2-(2-amino-ethoxy)-ethoxy]-acetyl)2-(gamma-Glu)-CO-(CH2)16-CO 2H
  MISC_FEATURE (20)..(20): Xaa at position 20 is Aib
  MISC_FEATURE (24)..(24): Xaa at position 24 is D-Glu
  MOD_RES (30)..(30): Gly at position 30 is amidated
YXEGTXTSDHSIXLDEKAQXHFIXYLIEGG

SEQ ID NO: 190 - protein, 39 aa, Artificial Sequence
  Synthetic Construct
  MISC_FEATURE (2)..(2): Xaa at position 2 is Aib
  MISC_FEATURE (6)..(6): Xaa at position 6 is alpha-methyl-Phe(2F)
  MISC_FEATURE (10)..(10): Xaa at position 10 is 3Pal
  MISC_FEATURE (13)..(13): Xaa at position 13 is alpha-methyl-Leu
  MOD_RES (17)..(17): Lys at position 17 is chemically modified by conjugation of the epsilon-amino group of the Lys side chain with (2-[2-(2-amino-ethoxy)-ethoxy]-acetyl)2-(gamma-Glu)-CO-(CH2)18-CO 2H
  MISC_FEATURE (20)..(20): Xaa at position 20 is Aib
  MISC_FEATURE (24)..(24): Xaa at position 24 is D-Glu
  MOD_RES (39)..(39): Ser at position 39 is amidated
YXEGTXTSDXSIXLDEKAQXEFIXYLIEGGPSSGAPPPS

SEQ ID NO: 191 - protein, 39 aa, Artificial Sequence; identical to SEQ ID NO: 190
  Synthetic Construct
  MISC_FEATURE (2)..(2): Xaa at position 2 is Aib
  MISC_FEATURE (6)..(6): Xaa at position 6 is alpha-methyl-Phe(2F)
  MISC_FEATURE (10)..(10): Xaa at position 10 is 4Pal
  MISC_FEATURE (13)..(13): Xaa at position 13 is alpha-methyl-Leu
  MOD_RES (17)..(17): Lys at position 17 is chemically modified by conjugation of the epsilon-amino group of the Lys side chain with (2-[2-(2-amino-ethoxy)-ethoxy]-acetyl)2-(gamma-Glu)-CO-(CH2)18-CO 2H
  MISC_FEATURE (20)..(20): Xaa at position 20 is Aib
  MISC_FEATURE (24)..(24): Xaa at position 24 is D-Glu
  MOD_RES (39)..(39): Ser at position 39 is amidated

SEQ ID NO: 192 - protein, 39 aa, Artificial Sequence
  Synthetic Construct
  MISC_FEATURE (2)..(2): Xaa at position 2 is Aib
  MISC_FEATURE (6)..(6): Xaa at position 6 is alpha-methyl-Phe(2F)
  MISC_FEATURE (13)..(13): Xaa at position 13 is alpha-methyl-Leu
  MOD_RES (17)..(17): Lys at position 17 is chemically modified by conjugation of the epsilon-amino group of the Lys side chain with (2-[2-(2-amino-ethoxy)-ethoxy]-acetyl)2-(gamma-Glu)-CO-(CH2)18-CO 2H
  MISC_FEATURE (20)..(20): Xaa at position 20 is Aib
  MISC_FEATURE (24)..(24): Xaa at position 24 is D-Glu
  MOD_RES (39)..(39): Ser at position 39 is amidated
YXEGTXTSDLSIXLDEKAQXEFIXYLIEGGPSSGAPPPS

SEQ ID NO: 193 - protein, 39 aa, Artificial Sequence; identical to SEQ ID NO: 190
  Synthetic Construct
  MISC_FEATURE (2)..(2): Xaa at position 2 is Aib
  MISC_FEATURE (6)..(6): Xaa at position 6 is alpha-methyl-Phe(2F)
  MISC_FEATURE (10)..(10): Xaa at position 10 is D-Tyr
  MISC_FEATURE (13)..(13): Xaa at position 13 is alpha-methyl-Leu
  MOD_RES (17)..(17): Lys at position 17 is chemically modified by conjugation of the epsilon-amino group of the Lys side chain with (2-[2-(2-amino-ethoxy)-ethoxy]-acetyl)2-(gamma-Glu)-CO-(CH2)18-CO 2H
  MISC_FEATURE (20)..(20): Xaa at position 20 is Aib
  MISC_FEATURE (24)..(24): Xaa at position 24 is D-Glu
  MOD_RES (39)..(39): Ser at position 39 is amidated

SEQ ID NO: 194 - protein, 39 aa, Artificial Sequence; identical to SEQ ID NO: 190
  Synthetic Construct
  MISC_FEATURE (2)..(2): Xaa at position 2 is Aib
  MISC_FEATURE (6)..(6): Xaa at position 6 is alpha-methyl-Phe(2F)
  MISC_FEATURE (10)..(10): Xaa at position 10 is D-His
  MISC_FEATURE (13)..(13): Xaa at position 13 is alpha-methyl-Leu
  MOD_RES (17)..(17): Lys at position 17 is chemically modified by conjugation of the epsilon-amino group of the Lys side chain with (2-[2-(2-amino-ethoxy)-ethoxy]-acetyl)2-(gamma-Glu)-CO-(CH2)18-CO 2H
  MISC_FEATURE (20)..(20): Xaa at position 20 is Aib
  MISC_FEATURE (24)..(24): Xaa at position 24 is D-Glu
  MOD_RES (39)..(39): Ser at position 39 is amidated

SEQ ID NO: 195 - protein, 39 aa, Artificial Sequence; identical to SEQ ID NO: 190
  Synthetic Construct
  MISC_FEATURE (2)..(2): Xaa at position 2 is Aib
  MISC_FEATURE (6)..(6): Xaa at position 6 is alpha-methyl-Phe(2F)
  MISC_FEATURE (10)..(10): Xaa at position 10 is alpha-methyl-Tyr
  MISC_FEATURE (13)..(13): Xaa at position 13 is alpha-methyl-Leu
  MOD_RES (17)..(17): Lys at position 17 is chemically modified by conjugation of the epsilon-amino group of the Lys side chain with (2-[2-(2-amino-ethoxy)-ethoxy]-acetyl)2-(gamma-Glu)-CO-(CH2)18-CO 2H
  MISC_FEATURE (20)..(20): Xaa at position 20 is Aib
  MISC_FEATURE (24)..(24): Xaa at position 24 is D-Glu
  MOD_RES (39)..(39): Ser at position 39 is amidated

SEQ ID NO: 196 - protein, 39 aa, Artificial Sequence
  Synthetic Construct
  MISC_FEATURE (2)..(2): Xaa at position 2 is Aib
  MISC_FEATURE (6)..(6): Xaa at position 6 is alpha-methyl-Phe(2F)
  MISC_FEATURE (13)..(13): Xaa at position 13 is alpha-methyl-Leu
  MOD_RES (17)..(17): Lys at position 17 is chemically modified by conjugation of the epsilon-amino group of the Lys side chain with (2-[2-(2-amino-ethoxy)-ethoxy]-acetyl)2-(gamma-Glu)-CO-(CH2)18-CO 2H
  MISC_FEATURE (20)..(20): Xaa at position 20 is Aib
  MISC_FEATURE (24)..(24): Xaa at position 24 is D-Glu
  MOD_RES (39)..(39): Ser at position 39 is amidated
YXEGTXTSDQSIXLDEKAQXEFIXYLIEGGPSSGAPPPS

SEQ ID NO: 197 - protein, 39 aa, Artificial Sequence; identical to SEQ ID NO: 190
  Synthetic Construct
  MISC_FEATURE (2)..(2): Xaa at position 2 is Aib
  MISC_FEATURE (6)..(6): Xaa at position 6 is alpha-methyl-Phe(2F)
  MISC_FEATURE (10)..(10): Xaa at position 10 is 3Pal
  MISC_FEATURE (13)..(13): Xaa at position 13 is alpha-methyl-Leu
  MOD_RES (17)..(17): Lys at position 17 is chemically modified by conjugation of the epsilon-amino group of the Lys side chain with (2-[2-(2-amino-ethoxy)-ethoxy]-acetyl)2-(gamma-Glu)-CO-(CH2)18-CO 2H
  MISC_FEATURE (20)..(20): Xaa at position 20 is Aib
  MISC_FEATURE (24)..(24): Xaa at position 24 is Aib
  MOD_RES (39)..(39): Ser at position 39 is amidated

SEQ ID NO: 198 - protein, 39 aa, Artificial Sequence; identical to SEQ ID NO: 190
  Synthetic Construct
  MISC_FEATURE (2)..(2): Xaa at position 2 is Aib
  MISC_FEATURE (6)..(6): Xaa at position 6 is alpha-methyl-Phe(2F)
  MISC_FEATURE (10)..(10): Xaa at position 10 is 4Pal
  MISC_FEATURE (13)..(13): Xaa at position 13 is alpha-methyl-Leu
  MOD_RES (17)..(17): Lys at position 17 is chemically modified by conjugation of the epsilon-amino group of the Lys side chain with (2-[2-(2-amino-ethoxy)-ethoxy]-acetyl)2-(gamma-Glu)-CO-(CH2)18-CO 2H
  MISC_FEATURE (20)..(20): Xaa at position 20 is Aib
  MISC_FEATURE (24)..(24): Xaa at position 24 is Aib
  MOD_RES (39)..(39): Ser at position 39 is amidated

SEQ ID NO: 199 - protein, 39 aa, Artificial Sequence
  Synthetic Construct
  MISC_FEATURE (2)..(2): Xaa at position 2 is Aib
  MISC_FEATURE (6)..(6): Xaa at position 6 is alpha-methyl-Phe(2F)
  MISC_FEATURE (10)..(10): Xaa at position 10 is 3Pal
  MISC_FEATURE (13)..(13): Xaa at position 13 is alpha-methyl-Leu
  MOD_RES (17)..(17): Lys at position 17 is chemically modified by conjugation of the epsilon-amino group of the Lys side chain with (2-[2-(2-amino-ethoxy)-ethoxy]-acetyl)2-(gamma-Glu)-CO-(CH2)18-CO 2H
  MISC_FEATURE (20)..(20): Xaa at position 20 is Aib
  MISC_FEATURE (24)..(24): Xaa at position 24 is D-Glu
  MOD_RES (39)..(39): Ser at position 39 is amidated
HXEGTXTSDXSIXLDEKAQXEFIXYLIEGGPSSGAPPPS

SEQ ID NO: 200 - protein, 39 aa, Artificial Sequence
  Synthetic Construct
  MISC_FEATURE (2)..(2): Xaa at position 2 is Aib
  MISC_FEATURE (6)..(6): Xaa at position 6 is alpha-methyl-Phe(2F)
  MISC_FEATURE (13)..(13): Xaa at position 13 is alpha-methyl-Leu
  MOD_RES (17)..(17): Lys at position 17 is chemically modified by conjugation of the epsilon-amino group of the Lys side chain with (2-[2-(2-amino-ethoxy)-ethoxy]-acetyl)2-(gamma-Glu)-CO-(CH2)18-CO 2H
  MISC_FEATURE (20)..(20): Xaa at position 20 is Aib
  MISC_FEATURE (24)..(24): Xaa at position 24 is D-Glu
  MOD_RES (39)..(39): Ser at position 39 is amidated
YXEGTXTSDVSIXLDEKAQXEFIXYLIEGGPSSGAPPPS

SEQ ID NO: 201 - protein, 39 aa, Artificial Sequence
  Synthetic Construct
  MISC_FEATURE (2)..(2): Xaa at position 2 is Aib
  MISC_FEATURE (6)..(6): Xaa at position 6 is alpha-methyl-Phe(2F)
  MISC_FEATURE (13)..(13): Xaa at position 13 is alpha-methyl-Leu
  MOD_RES (17)..(17): Lys at position 17 is chemically modified by conjugation of the epsilon-amino group of the Lys side chain with (2-[2-(2-amino-ethoxy)-ethoxy]-acetyl)2-(gamma-Glu)-CO-(CH2)18-CO 2H
  MISC_FEATURE (20)..(20): Xaa at position 20 is Aib
  MISC_FEATURE (24)..(24): Xaa at position 24 is D-Glu
  MOD_RES (39)..(39): Ser at position 39 is amidated
YXEGTXTSDASIXLDEKAQXEFIXYLIEGGPSSGAPPPS

SEQ ID NO: 202 - protein, 39 aa, Artificial Sequence
  Synthetic Construct
  MISC_FEATURE (2)..(2): Xaa at position 2 is alpha-methyl-Pro
  MOD_RES (17)..(17): Lys at position 17 is chemically modified by conjugation of the epsilon-amino group of the Lys side chain with (2-[2-(2-amino-ethoxy)-ethoxy]-acetyl)2-(gamma-Glu)-CO-(CH2)18-CO 2H
  MOD_RES (39)..(39): Ser at position 39 is amidated
YXEGTFTSDYSILLDEKAQQAFIEYLIEGGPSSGAPPPS

SEQ ID NO: 203 - protein, 39 aa, Artificial Sequence
  Synthetic Construct
  MISC_FEATURE (2)..(2): Xaa at position 2 is alpha-methyl-Pro
  MOD_RES (17)..(17): Lys at position 17 is chemically modified by conjugation of the epsilon-amino group of the Lys side chain with (2-[2-(2-amino-ethoxy)-ethoxy]-acetyl)2-(gamma-Glu)-CO-(CH2)18-CO 2H
  MOD_RES (39)..(39): Ser at position 39 is amidated
YXEGTFTSDYSILLDEKAQHAFIEYLIEGGPSSGAPPPS

SEQ ID NO: 204 - protein, 39 aa, Artificial Sequence
  Synthetic Construct
  MISC_FEATURE (2)..(2): Xaa at position 2 is alpha-methyl-Pro
  MOD_RES (17)..(17): Lys at position 17 is chemically modified by conjugation of the epsilon-amino group of the Lys side chain with (2-[2-(2-amino-ethoxy)-ethoxy]-acetyl)2-(gamma-Glu)-CO-(CH2)18-CO 2H
  MOD_RES (39)..(39): Ser at position 39 is amidated
YXEGTFTSDYSILLDRKAQQAFIEYLIEGGPSSGAPPPS

SEQ ID NO: 205 - protein, 39 aa, Artificial Sequence
  Synthetic Construct
  MISC_FEATURE (2)..(2): Xaa at position 2 is alpha-methyl-Pro
  MOD_RES (17)..(17): Lys at position 17 is chemically modified by conjugation of the epsilon-amino group of the Lys side chain with (2-[2-(2-amino-ethoxy)-ethoxy]-acetyl)2-(gamma-Glu)-CO-(CH2)18-CO 2H
  MOD_RES (39)..(39): Ser at position 39 is amidated
YXEGTFTSDYSILLDRKAQHAFIEYLIEGGPSSGAPPPS

SEQ ID NO: 206 - protein, 34 aa, Artificial Sequence
  Synthetic Construct
  MISC_FEATURE (2)..(2): Xaa at position 2 is alpha-methyl-Pro
  MOD_RES (17)..(17): Lys at position 17 is chemically modified by conjugation of the epsilon-amino group of the Lys side chain with (2-[2-(2-amino-ethoxy)-ethoxy]-acetyl)2-(gamma-Glu)-CO-(CH2)16-CO 2H
  MOD_RES (34)..(34): Gly at position 34 is amidated
YXEGTFTSDYSILLDEKAQQAFIEYLIEGGPSSG

SEQ ID NO: 207 - protein, 34 aa, Artificial Sequence
  Synthetic Construct
  MISC_FEATURE (1)..(1): Xaa at position 1 is D-Tyr
  MISC_FEATURE (2)..(2): Xaa at position 2 is alpha-methyl-Pro
  MOD_RES (17)..(17): Lys at position 17 is chemically modified by conjugation of the epsilon-amino group of the Lys side chain with (2-[2-(2-amino-ethoxy)-ethoxy]-acetyl)2-(gamma-Glu)-CO-(CH2)16-CO 2H
  MOD_RES (34)..(34): Gly at position 34 is amidated
XXEGTFTSDYSILLDEKAQQAFIEYLIEGGPSSG

SEQ ID NO: 208 - protein, 39 aa, Artificial Sequence
  Synthetic Construct
  MISC_FEATURE (1)..(1): Xaa at position 1 is DesTyr
  MISC_FEATURE (2)..(2): Xaa at position 2 is Aib
  MOD_RES (17)..(17): Lys at position 17 is chemically modified by conjugation of the epsilon-amino group of the Lys side chain with (2-[2-(2-amino-ethoxy)-ethoxy]-acetyl)2-(gamma-Glu)-CO-(CH2)18-CO 2H
  MOD_RES (39)..(39): Ser at position 39 is amidated
XXEGTFTSDYSILLDEKAQQAFIEYLIEGGPSSGAPPPS

SEQ ID NO: 209 - protein, 39 aa, Artificial Sequence
  Synthetic Construct
  MISC_FEATURE (1)..(1): Xaa at position 1 is DesTyr
  MOD_RES (17)..(17): Lys at position 17 is chemically modified by conjugation of the epsilon-amino group of the Lys side chain with (2-[2-(2-amino-ethoxy)-ethoxy]-acetyl)2-(gamma-Glu)-CO-(CH2)18-CO 2H
  MOD_RES (39)..(39): Ser at position 39 is amidated
XAEGTFTSDYSILLDEKAQQAFIEYLIEGGPSSGAPPPS

SEQ ID NO: 210 - protein, 39 aa, Artificial Sequence; identical to SEQ ID NO: 208
  Synthetic Construct
  MISC_FEATURE (1)..(1): Xaa at position 1 is DesHis
  MISC_FEATURE (2)..(2): Xaa at position 2 is alpha-methyl-Pro
  MOD_RES (17)..(17): Lys at position 17 is chemically modified by conjugation of the epsilon-amino group of the Lys side chain with (2-[2-(2-amino-ethoxy)-ethoxy]-acetyl)2-(gamma-Glu)-CO-(CH2)18-CO 2H
  MOD_RES (39)..(39): Ser at position 39 is amidated

SEQ ID NO: 211 - protein, 39 aa, Artificial Sequence
  Synthetic Construct
  MISC_FEATURE (2)..(2): Xaa at position 2 is Aib
  MISC_FEATURE (6)..(6): Xaa at position 6 is alpha-methyl-Phe(2F)
  MISC_FEATURE (10)..(10): Xaa at position 10 is 4Pal
  MISC_FEATURE (13)..(13): Xaa at position 13 is alpha-methyl-Leu
  MOD_RES (17)..(17): Lys at position 17 is chemically modified by conjugation of the epsilon-amino group of the Lys side chain with (2-[2-(2-Amino-ethoxy)-ethoxy]-acetyl)-(gamma-Glu)-(2-[2-(2-Amino -ethoxy)-ethoxy]-acetyl)-CO-(CH2)18-CO2H
  MISC_FEATURE (20)..(20): Xaa at position 20 is Aib
  MISC_FEATURE (24)..(24): Xaa at position 24 is D-Glu
  MOD_RES (39)..(39): Ser at position 39 is amidated
YXEGTXTSDXSIXLDKKAQXEFIXYLIEGGPSSGAPPPS

SEQ ID NO: 212 - protein, 39 aa, Artificial Sequence; identical to SEQ ID NO: 211
  Synthetic Construct
  MISC_FEATURE (2)..(2): Xaa at position 2 is Aib
  MISC_FEATURE (6)..(6): Xaa at position 6 is alpha-methyl-Phe(2F)
  MISC_FEATURE (10)..(10): Xaa at position 10 is 4Pal
  MISC_FEATURE (13)..(13): Xaa at position 13 is alpha-methyl-Leu
  MOD_RES (17)..(17): Lys at position 17 is chemically modified by conjugation of the epsilon-amino group of the Lys side chain with (2-[2-(2-amino-ethoxy)-ethoxy]-acetyl)2-(gamma-Glu)-CO-(CH2)18-CO 2H
  MISC_FEATURE (20)..(20): Xaa at position 20 is Aib
  MISC_FEATURE (24)..(24): Xaa at position 24 is D-Glu
  MOD_RES (39)..(39): Ser at position 39 is amidated

SEQ ID NO: 213 - protein, 39 aa, Artificial Sequence; identical to SEQ ID NO: 190
  Synthetic Construct
  MISC_FEATURE (2)..(2): Xaa at position 2 is Aib
  MISC_FEATURE (6)..(6): Xaa at position 6 is alpha-methyl-Phe(2F)
  MISC_FEATURE (10)..(10): Xaa at position 10 is 4Pal
  MISC_FEATURE (13)..(13): Xaa at position 13 is alpha-methyl-Leu
  MOD_RES (17)..(17): Lys at position 17 is chemically modified by conjugation of the epsilon-amino group of the Lys side chain with (2-[2-(2-amino-ethoxy)-ethoxy]-acetyl)2-(gamma-Glu)-CO-(CH2)16-CO 2H
  MISC_FEATURE (20)..(20): Xaa at position 20 is Aib
  MISC_FEATURE (24)..(24): Xaa at position 24 is D-Glu
  MOD_RES (39)..(39): Ser at position 39 is amidated

SEQ ID NO: 214 - protein, 39 aa, Artificial Sequence; identical to SEQ ID NO: 190
  Synthetic Construct
  MISC_FEATURE (2)..(2): Xaa at position 2 is Aib
  MISC_FEATURE (6)..(6): Xaa at position 6 is alpha-methyl-Phe(2F)
  MISC_FEATURE (10)..(10): Xaa at position 10 is 4Pal
  MISC_FEATURE (13)..(13): Xaa at position 13 is alpha-methyl-Leu
  MOD_RES (17)..(17): Lys at position 17 is chemically modified by conjugation of the epsilon-amino group of the Lys side chain with (2-[2-(2-amino-ethoxy)-ethoxy]-acetyl)2-CO-(CH2)16-CO2H
  MISC_FEATURE (20)..(20): Xaa at position 20 is Aib
  MISC_FEATURE (24)..(24): Xaa at position 24 is D-Glu
  MOD_RES (39)..(39): Ser at position 39 is amidated

SEQ ID NO: 215 - protein, 39 aa, Artificial Sequence; identical to SEQ ID NO: 190
  Synthetic Construct
  MISC_FEATURE (2)..(2): Xaa at position 2 is Aib
  MISC_FEATURE (6)..(6): Xaa at position 6 is alpha-methyl-Phe(2F)
  MISC_FEATURE (10)..(10): Xaa at position 10 is 4Pal
  MISC_FEATURE (13)..(13): Xaa at position 13 is alpha-methyl-Leu
  MOD_RES (17)..(17): Lys at position 17 is chemically modified by conjugation of the epsilon-amino group of the Lys side chain with (2-[2-(2-amino-ethoxy)-ethoxy]-acetyl)2-CO-(CH2)18-CO2H
  MISC_FEATURE (20)..(20): Xaa at position 20 is Aib
  MISC_FEATURE (24)..(24): Xaa at position 24 is D-Glu
  MOD_RES (39)..(39): Ser at position 39 is amidated

SEQ ID NO: 216 - protein, 39 aa, Artificial Sequence; identical to SEQ ID NO: 190
  Synthetic Construct
  MISC_FEATURE (2)..(2): Xaa at position 2 is Aib
  MISC_FEATURE (6)..(6): Xaa at position 6 is alpha-methyl-Phe(2F)
  MISC_FEATURE (10)..(10): Xaa at position 10 is 4Pal
  MISC_FEATURE (13)..(13): Xaa at position 13 is alpha-methyl-Leu
  MOD_RES (17)..(17): Lys at position 17 is chemically modified by conjugation of the epsilon-amino group of the Lys side chain with (2-[2-(2-Amino-ethoxy)-ethoxy]-acetyl)2-(epsilon-Lys)-CO-(CH2)18- CO2H
  MISC_FEATURE (20)..(20): Xaa at position 20 is Aib
  MISC_FEATURE (24)..(24): Xaa at position 24 is D-Glu
  MOD_RES (39)..(39): Ser at position 39 is amidated

SEQ ID NO: 217 - protein, 39 aa, Artificial Sequence; identical to SEQ ID NO: 10
  Synthetic Construct
  MISC_FEATURE (2)..(2): Xaa at position 2 is Aib
  MISC_FEATURE (6)..(6): Xaa at position 6 is alpha-methyl-Phe(2F)
  MISC_FEATURE (13)..(13): Xaa at position 13 is alpha-methyl-Leu
  MOD_RES (17)..(17): Lys at position 17 is chemically modified by conjugation of the epsilon-amino group of the Lys side chain with (2-[2-(2-amino-ethoxy)-ethoxy]-acetyl)2-(gamma-Glu)-CO-(CH2)14-CO 2H
  MISC_FEATURE (20)..(20): Xaa at position 20 is Aib
  MISC_FEATURE (24)..(24): Xaa at position 24 is D-Glu
  MOD_RES (39)..(39): Ser at position 39 is amidated

SEQ ID NO: 218 - protein, 39 aa, Artificial Sequence; identical to SEQ ID NO: 11
  Synthetic Construct
  MISC_FEATURE (2)..(2): Xaa at position 2 is Aib
  MISC_FEATURE (6)..(6): Xaa at position 6 is alpha-methyl-Phe(2F)
  MISC_FEATURE (13)..(13): Xaa at position 13 is alpha-methyl-Leu
  MISC_FEATURE (16)..(16): Xaa at position 16 is Dab
  MOD_RES (17)..(17): Lys at position 17 is chemically modified by conjugation of the epsilon-amino group of the Lys side chain with (2-[2-(2-amino-ethoxy)-ethoxy]-acetyl)2-(gamma-Glu)-CO-(CH2)16-CO 2H
  MISC_FEATURE (20)..(20): Xaa at position 20 is Aib
  MISC_FEATURE (24)..(24): Xaa at position 24 is D-Glu
  MOD_RES (39)..(39): Ser at position 39 is amidated

SEQ ID NO: 219 - protein, 39 aa, Artificial Sequence; identical to SEQ ID NO: 11
  Synthetic Construct
  MISC_FEATURE (2)..(2): Xaa at position 2 is Aib
  MISC_FEATURE (6)..(6): Xaa at position 6 is alpha-methyl-Phe(2F)
  MISC_FEATURE (13)..(13): Xaa at position 13 is alpha-methyl-Leu
  MISC_FEATURE (16)..(16): Xaa at position 16 is Dap
  MOD_RES (17)..(17): Lys at position 17 is chemically modified by conjugation of the epsilon-amino group of the Lys side chain with (2-[2-(2-amino-ethoxy)-ethoxy]-acetyl)2-(gamma-Glu)-CO-(CH2)16-CO 2H
  MISC_FEATURE (20)..(20): Xaa at position 20 is Aib
  MISC_FEATURE (24)..(24): Xaa at position 24 is D-Glu
  MOD_RES (39)..(39): Ser at position 39 is amidated

SEQ ID NO: 220 - protein, 39 aa, Artificial Sequence
  Synthetic Construct
  MISC_FEATURE (2)..(2): Xaa at position 2 is Aib
  MISC_FEATURE (6)..(6): Xaa at position 6 is alpha-methyl-Phe(2F)
  MISC_FEATURE (13)..(13): Xaa at position 13 is alpha-methyl-Leu
  MOD_RES (17)..(17): Lys at position 17 is chemically modified by conjugation of the epsilon-amino group of the Lys side chain with (2-[2-(2-Amino-ethoxy)-ethoxy]-acetyl)-(gamma-Glu)-(2-[2-(2-Amino -ethoxy)-ethoxy]-acetyl)-CO-(CH2)18-CO2H
  MISC_FEATURE (20)..(20): Xaa at position 20 is Aib
  MISC_FEATURE (24)..(24): Xaa at position 24 is D-Glu
  MOD_RES (39)..(39): Ser at position 39 is amidated
YXEGTXTSDYSIXLDKKAQXEFIXYLIEGGPSSGAPPPS

SEQ ID NO: 221 - protein, 39 aa, Artificial Sequence; identical to SEQ ID NO: 220
  Synthetic Construct
  MISC_FEATURE (2)..(2): Xaa at position 2 is Aib
  MISC_FEATURE (6)..(6): Xaa at position 6 is alpha-methyl-Phe(2F)
  MISC_FEATURE (13)..(13): Xaa at position 13 is alpha-methyl-Leu
  MOD_RES (17)..(17): Lys at position 17 is chemically modified by conjugation of the epsilon-amino group of the Lys side chain with (2-[2-(2-amino-ethoxy)-ethoxy]-acetyl)2-(gamma-Glu)-CO-(CH2)18-CO 2H
  MISC_FEATURE (20)..(20): Xaa at position 20 is Aib
  MISC_FEATURE (24)..(24): Xaa at position 24 is D-Glu
  MOD_RES (39)..(39): Ser at position 39 is amidated

SEQ ID NO: 222 - protein, 39 aa, Artificial Sequence; identical to SEQ ID NO: 10
  Synthetic Construct
  MISC_FEATURE (2)..(2): Xaa at position 2 is Aib
  MISC_FEATURE (6)..(6): Xaa at position 6 is alpha-methyl-Phe
  MISC_FEATURE (13)..(13): Xaa at position 13 is alpha-methyl-Leu
  MOD_RES (17)..(17): Lys at position 17 is chemically modified by conjugation of the epsilon-amino group of the Lys side chain with (2-[2-(2-amino-ethoxy)-ethoxy]-acetyl)2-(gamma-Glu)-CO-(CH2)16-CO 2H
  MISC_FEATURE (20)..(20): Xaa at position 20 is Aib
  MISC_FEATURE (24)..(24): Xaa at position 24 is D-Glu
  MOD_RES (39)..(39): Ser at position 39 is amidated

SEQ ID NO: 223 - protein, 39 aa, Artificial Sequence; identical to SEQ ID NO: 10
  Synthetic Construct
  MISC_FEATURE (2)..(2): Xaa at position 2 is Aib
  MISC_FEATURE (6)..(6): Xaa at position 6 is alpha-methyl-Phe(2F)
  MISC_FEATURE (13)..(13): Xaa at position 13 is alpha-methyl-Leu
  MOD_RES (17)..(17): Lys at position 17 is chemically modified by conjugation of the epsilon-amino group of the Lys side chain with (2-[2-(2-amino-ethoxy)-ethoxy]-acetyl)2-CO-(CH2)16-CO2H
  MISC_FEATURE (20)..(20): Xaa at position 20 is Aib
  MISC_FEATURE (24)..(24): Xaa at position 24 is D-Glu
  MOD_RES (39)..(39): Ser at position 39 is amidated

SEQ ID NO: 224 - protein, 39 aa, Artificial Sequence; identical to SEQ ID NO: 10
  Synthetic Construct
  MISC_FEATURE (2)..(2): Xaa at position 2 is Aib
  MISC_FEATURE (6)..(6): Xaa at position 6 is alpha-methyl-Phe(2F)
  MISC_FEATURE (13)..(13): Xaa at position 13 is alpha-methyl-Leu
  MOD_RES (17)..(17): Lys at position 17 is chemically modified by conjugation of the epsilon-amino group of the Lys side chain with (2-[2-(2-amino-ethoxy)-ethoxy]-acetyl)2-CO-(CH2)18-CO2H
  MISC_FEATURE (20)..(20): Xaa at position 20 is Aib
  MISC_FEATURE (24)..(24): Xaa at position 24 is D-Glu
  MOD_RES (39)..(39): Ser at position 39 is amidated

SEQ ID NO: 225 - protein, 39 aa, Artificial Sequence; identical to SEQ ID NO: 10
  Synthetic Construct
  MISC_FEATURE (2)..(2): Xaa at position 2 is Aib
  MISC_FEATURE (6)..(6): Xaa at position 6 is alpha-methyl-Phe(2F)
  MISC_FEATURE (13)..(13): Xaa at position 13 is alpha-methyl-Leu
  MOD_RES (17)..(17): Lys at position 17 is chemically modified by conjugation of the epsilon-amino group of the Lys side chain with (2-[2-(2-amino-ethoxy)-ethoxy]-acetyl)2-(epsilon-Lys)-CO-(CH2)18- CO2H
  MISC_FEATURE (20)..(20): Xaa at position 20 is Aib
  MISC_FEATURE (24)..(24): Xaa at position 24 is D-Glu
  MOD_RES (39)..(39): Ser at position 39 is amidated

SEQ ID NO: 226 - protein, 39 aa, Artificial Sequence; identical to SEQ ID NO: 11
  Synthetic Construct
  MISC_FEATURE (2)..(2): Xaa at position 2 is Aib
  MISC_FEATURE (6)..(6): Xaa at position 6 is alpha-methyl-Phe(2F)
  MISC_FEATURE (13)..(13): Xaa at position 13 is alpha-methyl-Leu
  MISC_FEATURE (16)..(16): Xaa at position 16 is Dab
  MOD_RES (17)..(17): Lys at position 17 is chemically modified by conjugation of the epsilon-amino group of the Lys side chain with (2-[2-(2-amino-ethoxy)-ethoxy]-acetyl)2-(gamma-Glu)-CO-(CH2)18-CO 2H
  MISC_FEATURE (20)..(20): Xaa at position 20 is Aib
  MISC_FEATURE (24)..(24): Xaa at position 24 is D-Glu
  MOD_RES (39)..(39): Ser at position 39 is amidated

SEQ ID NO: 227 - protein, 39 aa, Artificial Sequence; identical to SEQ ID NO: 11
  Synthetic Construct
  MISC_FEATURE (2)..(2): Xaa at position 2 is Aib
  MISC_FEATURE (6)..(6): Xaa at position 6 is alpha-methyl-Phe(2F)
  MISC_FEATURE (13)..(13): Xaa at position 13 is alpha-methyl-Leu
  MISC_FEATURE (16)..(16): Xaa at position 16 is Dap
  MOD_RES (17)..(17): Lys at position 17 is chemically modified by conjugation of the epsilon-amino group of the Lys side chain with (2-[2-(2-amino-ethoxy)-ethoxy]-acetyl)2-(gamma-Glu)-CO-(CH2)18-CO 2H
  MISC_FEATURE (20)..(20): Xaa at position 20 is Aib
  MISC_FEATURE (24)..(24): Xaa at position 24 is D-Glu
  MOD_RES (39)..(39): Ser at position 39 is amidated

SEQ ID NO: 228 - protein, 34 aa, Artificial Sequence
  Synthetic Construct
  MISC_FEATURE (2)..(2): Xaa at position 2 is Aib
  MISC_FEATURE (6)..(6): Xaa at position 6 is alpha-methyl-Phe(2F)
  MISC_FEATURE (13)..(13): Xaa at position 13 is alpha-methyl-Leu
  MOD_RES (17)..(17): Lys at position 17 is chemically modified by conjugation of the epsilon-amino group of the Lys side chain with (2-[2-(2-amino-ethoxy)-ethoxy]-acetyl)2-(gamma-Glu)-CO-(CH2)16-CO 2H
  MISC_FEATURE (20)..(20): Xaa at position 20 is Aib
  MISC_FEATURE (24)..(24): Xaa at position 24 is D-Glu
  MOD_RES (34)..(34): Gly at position 34 is amidated
YXEGTXTSDYSIXLDEKAQXEFIXYLIEGGPSSG

SEQ ID NO: 229 - protein, 30 aa, Artificial Sequence
  Synthetic Construct
  MISC_FEATURE (2)..(2): Xaa at position 2 is Aib
  MISC_FEATURE (6)..(6): Xaa at position 6 is alpha-methyl-Phe(2F)
  MISC_FEATURE (13)..(13): Xaa at position 13 is alpha-methyl-Leu
  MOD_RES (17)..(17): Lys at position 17 is chemically modified by conjugation of the epsilon-amino group of the Lys side chain with (2-[2-(2-amino-ethoxy)-ethoxy]-acetyl)2-(gamma-Glu)-CO-(CH2)16-CO 2H
  MISC_FEATURE (20)..(20): Xaa at position 20 is Aib
  MISC_FEATURE (24)..(24): Xaa at position 24 is D-Glu
  MOD_RES (30)..(30): Gly at position 30 is amidated
YXEGTXTSDYSIXLDEKAQXEFIXYLIEGG

SEQ ID NO: 230 - protein, 39 aa, Artificial Sequence; identical to SEQ ID NO: 10
  Synthetic Construct
  MISC_FEATURE (2)..(2): Xaa at position 2 is Aib
  MISC_FEATURE (6)..(6): Xaa at position 6 is alpha-methyl-Phe(2F)
  MISC_FEATURE (13)..(13): Xaa at position 13 is alpha-methyl-Leu
  MOD_RES (17)..(17): Lys at position 17 is chemically modified by conjugation of the epsilon-amino group of the Lys side chain with (2-[2-(2-amino-ethoxy)-ethoxy]-acetyl)2-(gamma-Glu)-CO-(CH2)16-CO 2H
  MISC_FEATURE (20)..(20): Xaa at position 20 is Aib
  MISC_FEATURE (24)..(24): Xaa at position 24 is D-Glu
  MOD_RES (39)..(39): Ser at position 39 is amidated

SEQ ID NO: 231 - protein, 39 aa, Artificial Sequence
  Synthetic Construct
  MISC_FEATURE (2)..(2): Xaa at position 2 is Aib
  MISC_FEATURE (6)..(6): Xaa at position 6 is alpha-methyl-Phe(2F)
  MISC_FEATURE (13)..(13): Xaa at position 13 is alpha-methyl-Leu
  MOD_RES (17)..(17): Lys at position 17 is chemically modified by conjugation of the epsilon-amino group of the Lys side chain with (2-[2-(2-amino-ethoxy)-ethoxy]-acetyl)2-(gamma-Glu)-CO-(CH2)18-CO 2H
  MISC_FEATURE (20)..(20): Xaa at position 20 is Aib
  MISC_FEATURE (24)..(24): Xaa at position 24 is D-Glu
  MISC_FEATURE (25)..(25): Xaa at position 25 alpha-methyl-Tyr
  MOD_RES (39)..(39): Ser at position 39 is amidated
YXEGTXTSDYSIXLDEKAQXEFIXXLIEGGPSSGAPPPS

SEQ ID NO: 232 - protein, 39 aa, Artificial Sequence
  Synthetic Construct
  MISC_FEATURE (2)..(2): Xaa at position 2 is Aib
  MISC_FEATURE (6)..(6): Xaa at position 6 is alpha-methyl-Phe(2F)
  MISC_FEATURE (13)..(13): Xaa at position 13 is alpha-methyl-Leu
  MOD_RES (17)..(17): Lys at position 17 is chemically modified by conjugation of the epsilon-amino group of the Lys side chain with (2-[2-(2-amino-ethoxy)-ethoxy]-acetyl)2-(gamma-Glu)-CO-(CH2)18-CO 2H
  MISC_FEATURE (20)..(20): Xaa at position 20 is Aib
  MISC_FEATURE (25)..(25): Xaa at position 25 is alpha-methyl-Tyr
  MOD_RES (39)..(39): Ser at position 39 is amidated
YXEGTXTSDYSIXLDEKAQXEFIEXLIEGGPSSGAPPPS

SEQ ID NO: 233 - protein, 39 aa, Artificial Sequence; identical to SEQ ID NO: 10
  Synthetic Construct
  MISC_FEATURE (2)..(2): Xaa at position 2 is Aib
  MISC_FEATURE (6)..(6): Xaa at position 6 is alpha-methyl-Phe(2F)
  MISC_FEATURE (13)..(13): Xaa at position 13 is Aib
  MOD_RES (17)..(17): Lys at position 17 is chemically modified by conjugation of the epsilon-amino group of the Lys side chain with (2-[2-(2-amino-ethoxy)-ethoxy]-acetyl)2-(gamma-Glu)-CO-(CH2)18-CO 2H
  MISC_FEATURE (20)..(20): Xaa at position 20 is Aib
  MISC_FEATURE (24)..(24): Xaa at position 24 is D-Glu
  MOD_RES (39)..(39): Ser at position 39 is amidated

SEQ ID NO: 234 - protein, 39 aa, Artificial Sequence; identical to SEQ ID NO: 10
  Synthetic Construct
  MISC_FEATURE (2)..(2): Xaa at position 2 is Aib
  MISC_FEATURE (6)..(6): Xaa at position 6 is alpha-methyl-Phe
  MISC_FEATURE (13)..(13): Xaa at position 13 is Aib
  MOD_RES (17)..(17): Lys at position 17 is chemically modified by conjugation of the epsilon-amino group of the Lys side chain with (2-[2-(2-amino-ethoxy)-ethoxy]-acetyl)2-(gamma-Glu)-CO-(CH2)18-CO 2H
  MISC_FEATURE (20)..(20): Xaa at position 20 is Aib
  MISC_FEATURE (24)..(24): Xaa at position 24 is D-Glu
  MOD_RES (39)..(39): Ser at position 39 is amidated

SEQ ID NO: 235 - protein, 39 aa, Artificial Sequence
  Synthetic Construct
  MISC_FEATURE (2)..(2): Xaa at position 2 is Aib
  MISC_FEATURE (6)..(6): Xaa at position 6 is alpha-methyl-Phe(2F)
  MOD_RES (17)..(17): Lys at position 17 is chemically modified by conjugation of the epsilon-amino group of the Lys side chain with (2-[2-(2-amino-ethoxy)-ethoxy]-acetyl)2-(gamma-Glu)-CO-(CH2)18-CO 2H
  MISC_FEATURE (20)..(20): Xaa at position 20 is Aib
  MISC_FEATURE (24)..(24): Xaa at position 24 is D-Glu
  MOD_RES (39)..(39): Ser at position 39 is amidated
YXEGTXTSDYSILLDEKAQXEFIXYLIEGGPSSGAPPPS

SEQ ID NO: 236 - protein, 39 aa, Artificial Sequence; identical to SEQ ID NO: 10
  Synthetic Construct
  MISC_FEATURE (2)..(2): Xaa at position 2 is Aib
  MISC_FEATURE (6)..(6): Xaa at position 6 is alpha-methyl-Phe
  MISC_FEATURE (13)..(13): Xaa at position 13 is alpha-methyl-Leu
  MOD_RES (17)..(17): Lys at position 17 is chemically modified by conjugation of the epsilon-amino group of the Lys side chain with (2-[2-(2-amino-ethoxy)-ethoxy]-acetyl)2-(gamma-Glu)-CO-(CH2)18-CO 2H
  MISC_FEATURE (20)..(20): Xaa at position 20 is Aib
  MISC_FEATURE (24)..(24): Xaa at position 24 is D-Glu
  MOD_RES (39)..(39): Ser at position 39 is amidated

SEQ ID NO: 237 - protein, 34 aa, Artificial Sequence
  Synthetic Construct
  MISC_FEATURE (2)..(2): Xaa at position 2 is Aib
  MISC_FEATURE (6)..(6): Xaa at position 6 is alpha-methyl-Phe
  MISC_FEATURE (13)..(13): Xaa at position 13 is alpha-methyl-Leu
  MOD_RES (17)..(17): Lys at position 17 is chemically modified by conjugation of the epsilon-amino group of the Lys side chain with (2-[2-(2-amino-ethoxy)-ethoxy]-acetyl)2-(gamma-Glu)-CO-(CH2)18-CO 2H
  MISC_FEATURE (20)..(20): Xaa at position 20 is Aib
  MISC_FEATURE (24)..(24): Xaa at position 24 is D-Glu
  MOD_RES (34)..(34): Gly at position 34 is amidated
YXEGTXTSDYSIXLDKKAQXEFIXYLIEGGPSSG

SEQ ID NO: 238 - protein, 38 aa, Artificial Sequence
  Synthetic Construct
  MISC_FEATURE (2)..(2): Xaa at position 2 is Aib
  MISC_FEATURE (6)..(6): Xaa at position 6 is alpha-methyl-Phe(2F)
  MISC_FEATURE (12)..(12): Xaa at position 12 is alpha-methyl-Leu
  MOD_RES (16)..(16): Lys at position 16 is chemically modified by conjugation of the epsilon-amino group of the Lys side chain with (2-[2-(2-amino-ethoxy)-ethoxy]-acetyl)2-(gamma-Glu)-CO-(CH2)18-CO 2H
  MISC_FEATURE (19)..(19): Xaa at position 19 is Aib
  MISC_FEATURE (23)..(23): Xaa at position 23 is D-Glu
  MOD_RES (38)..(38): Ser at position 39 is amidated
YXEGTXTSDYSXLDEKAQXEFIXYLIEGGPSSGAPPPS

SEQ ID NO: 239 - protein, 39 aa, Artificial Sequence
  Synthetic Construct
  MISC_FEATURE (2)..(2): Xaa at position 2 is Aib
  MISC_FEATURE (6)..(6): Xaa at position 6 is alpha-methyl-Phe(2F)
  MISC_FEATURE (13)..(13): Xaa at position 13 is alpha-methyl-Leu
  MOD_RES (17)..(17): Lys at position 17 is chemically modified by conjugation of the epsilon-amino group of the Lys side chain with (2-[2-(2-amino-ethoxy)-ethoxy]-acetyl)2-(gamma-Glu)-CO-(CH2)18-CO 2H
  MISC_FEATURE (20)..(20): Xaa at position 20 is Aib
  MISC_FEATURE (24)..(24): Xaa at position 24 is D-Glu
  MOD_RES (39)..(39): Ser at position 39 is amidated
YXEGTXTSDYSIXLDHKAQXEFIXYLIEGGPSSGAPPPS

SEQ ID NO: 240 - protein, 39 aa, Artificial Sequence; identical to SEQ ID NO: 220
  Synthetic Construct
  MISC_FEATURE (2)..(2): Xaa at position 2 is Aib
  MISC_FEATURE (6)..(6): Xaa at position 6 is alpha-methyl-Phe(2F)
  MISC_FEATURE (13)..(13): Xaa at position 13 is alpha-methyl-Leu
  MOD_RES (17)..(17): Lys at position 17 is chemically modified by conjugation of the epsilon-amino group of the Lys side chain with (2-[2-(2-amino-ethoxy)-ethoxy]-acetyl)2-(gamma-Glu)-CO-(CH2)16-CO 2H
  MISC_FEATURE (20)..(20): Xaa at position 20 is Aib
  MISC_FEATURE (24)..(24): Xaa at position 24 is D-Glu
  MOD_RES (39)..(39): Ser at position 39 is amidated

SEQ ID NO: 241 - protein, 39 aa, Artificial Sequence
  Synthetic Construct
  MISC_FEATURE (2)..(2): Xaa at position 2 is Aib
  MISC_FEATURE (6)..(6): Xaa at position 6 is alpha-methyl-Phe(2F)
  MISC_FEATURE (10)..(10): Xaa at position 10 is 4Pal
  MISC_FEATURE (13)..(13): Xaa at position 13 is alpha-methyl-Leu
  MISC_FEATURE (16)..(16): Xaa at position 16 is Orn
  MOD_RES (17)..(17): Lys at position 17 is chemically modified by conjugation of the epsilon-amino group of the Lys side chain with (2-[2-(2-amino-ethoxy)-ethoxy]-acetyl)2-(gamma-Glu)-CO-(CH2)16-CO 2H
  MISC_FEATURE (20)..(20): Xaa at position 20 is Aib
  MISC_FEATURE (24)..(24): Xaa at position 24 is D-Glu
  MOD_RES (39)..(39): Ser at position 39 is amidated
YXEGTXTSDXSIXLDXKAQXEFIXYLIEGGPSSGAPPPS

SEQ ID NO: 242 - protein, 39 aa, Artificial Sequence; identical to SEQ ID NO: 241
  Synthetic Construct
  MISC_FEATURE (2)..(2): Xaa at position 2 is Aib
  MISC_FEATURE (6)..(6): Xaa at position 6 is alpha-methyl-Phe(2F)
  MISC_FEATURE (10)..(10): Xaa at position 10 is 4Pal
  MISC_FEATURE (13)..(13): Xaa at position 13 is alpha-methyl-Leu
  MISC_FEATURE (16)..(16): Xaa at position 16 is Dab
  MOD_RES (17)..(17): Lys at position 17 is chemically modified by conjugation of the epsilon-amino group of the Lys side chain with (2-[2-(2-amino-ethoxy)-ethoxy]-acetyl)2-(gamma-Glu)-CO-(CH2)16-CO 2H
  MISC_FEATURE (20)..(20): Xaa at position 20 is Aib
  MISC_FEATURE (24)..(24): Xaa at position 24 is D-Glu
  MOD_RES (39)..(39): Ser at position 39 is amidated

SEQ ID NO: 243 - protein, 39 aa, Artificial Sequence
  Synthetic Construct
  MISC_FEATURE (2)..(2): Xaa at position 2 is Aib
  MISC_FEATURE (6)..(6): Xaa at position 6 is alpha-methyl-Phe(2F)
  MISC_FEATURE (10)..(10): Xaa at position 10 is 4Pal
  MISC_FEATURE (16)..(16): Xaa at position 16 is Dab
  MOD_RES (17)..(17): Lys at position 17 is chemically modified by conjugation of the epsilon-amino group of the Lys side chain with (2-[2-(2-amino-ethoxy)-ethoxy]-acetyl)2-(gamma-Glu)-CO-(CH2)16-CO 2H
  MISC_FEATURE (20)..(20): Xaa at position 20 is Aib
  MISC_FEATURE (24)..(24): Xaa at position 24 is D-Glu
  MOD_RES (39)..(39): Ser at position 39 is amidated
YXEGTXTSDXSILLDXKAQXEFIXYLIEGGPSSGAPPPS

SEQ ID NO: 244 - protein, 39 aa, Artificial Sequence; identical to SEQ ID NO: 241
  Synthetic Construct
  MISC_FEATURE (2)..(2): Xaa at position 2 is Aib
  MISC_FEATURE (6)..(6): Xaa at position 6 is alpha-methyl-Phe
  MISC_FEATURE (10)..(10): Xaa at position 10 is 4Pal
  MISC_FEATURE (13)..(13): Xaa at position 13 is alpha-methyl-Leu
  MISC_FEATURE (16)..(16): Xaa at position 16 is Dab
  MOD_RES (17)..(17): Lys at position 17 is chemically modified by conjugation of the epsilon-amino group of the Lys side chain with (2-[2-(2-amino-ethoxy)-ethoxy]-acetyl)2-(gamma-Glu)-CO-(CH2)16-CO 2H
  MISC_FEATURE (20)..(20): Xaa at position 20 is Aib
  MISC_FEATURE (24)..(24): Xaa at position 24 is D-Glu
  MOD_RES (39)..(39): Ser at position 39 is amidated

SEQ ID NO: 245 - protein, 39 aa, Artificial Sequence
  Synthetic Construct
  MISC_FEATURE (2)..(2): Xaa at position 2 is Aib
  MISC_FEATURE (6)..(6): Xaa at position 6 is alpha-methyl-Phe(2F)
  MISC_FEATURE (13)..(13): Xaa at position 13 is alpha-methyl-Leu
  MISC_FEATURE (16)..(16): Xaa at position 16 is Orn
  MOD_RES (17)..(17): Lys at position 17 is chemically modified by conjugation of the epsilon-amino group of the Lys side chain with (2-[2-(2-amino-ethoxy)-ethoxy]-acetyl)2-(gamma-Glu)-CO-(CH2)16-CO 2H
  MISC_FEATURE (20)..(20): Xaa at position 20 is Aib
  MISC_FEATURE (24)..(24): Xaa at position 24 is D-Glu
  MISC_FEATURE (25)..(25): Xaa at position 25 is alpha-methyl-Tyr
  MOD_RES (39)..(39): Ser at position 39 is amidated
YXEGTXTSDYSIXLDXKAQXEFIXXLIEGGPSSGAPPPS

SEQ ID NO: 246 - protein, 39 aa, Artificial Sequence
  Synthetic Construct
  MISC_FEATURE (2)..(2): Xaa at position 2 is Aib
  MISC_FEATURE (6)..(6): Xaa at position 6 is alpha-methyl-Phe(2F)
  MISC_FEATURE (13)..(13): Xaa at position 13 is alpha-methyl-Leu
  MISC_FEATURE (16)..(16): Xaa at position 16 is Orn
  MOD_RES (17)..(17): Lys at position 17 is chemically modified by conjugation of the epsilon-amino group of the Lys side chain with (2-[2-(2-amino-ethoxy)-ethoxy]-acetyl)2-(gamma-Glu)-CO-(CH2)16-CO 2H
  MISC_FEATURE (20)..(20): Xaa at position 20 is Aib
  MISC_FEATURE (24)..(24): Xaa at position 24 is D-Glu
  MISC_FEATURE (25)..(25): Xaa at position 25 alpha-methyl-Tyr
  MOD_RES (39)..(39): Ser at position 39 is amidated
YXEGTXTSDASIXLDXKAQXEFIXXLIEGGPSSGAPPPS

SEQ ID NO: 247 - protein, 39 aa, Artificial Sequence
  Synthetic Construct
  MISC_FEATURE (2)..(2): Xaa at position 2 is Aib
  MISC_FEATURE (6)..(6): Xaa at position 6 is alpha-methyl-Phe(2F)
  MISC_FEATURE (13)..(13): Xaa at position 13 is alpha-methyl-Leu
  MISC_FEATURE (16)..(16): Xaa at position 16 is Orn
  MOD_RES (17)..(17): Lys at position 17 is chemically modified by conjugation of the epsilon-amino group of the Lys side chain with (2-[2-(2-amino-ethoxy)-ethoxy]-acetyl)2-(gamma-Glu)-CO-(CH2)16-CO 2H
  MISC_FEATURE (20)..(20): Xaa at position 20 is Aib
  MISC_FEATURE (24)..(24): Xaa at position 24 is D-Glu
  MISC_FEATURE (25)..(25): Xaa at position 25 is alpha-methyl-Tyr
  MOD_RES (39)..(39): Ser at position 39 is amidated
YXEGTXTSDLSIXLDXKAQXEFIXXLIEGGPSSGAPPPS

SEQ ID NO: 248 - protein, 39 aa, Artificial Sequence
  Synthetic Construct
  MISC_FEATURE (2)..(2): Xaa at position 2 is Aib
  MISC_FEATURE (6)..(6): Xaa at position 6 is alpha-methyl-Phe(2F)
  MISC_FEATURE (10)..(10): Xaa at position 10 is 4Pal
  MISC_FEATURE (13)..(13): Xaa at position 13 is alpha-methyl-Leu
  MISC_FEATURE (16)..(16): Xaa at position 16 is Orn
  MOD_RES (17)..(17): Lys at position 17 is chemically modified by conjugation of the epsilon-amino group of the Lys side chain with (2-[2-(2-amino-ethoxy)-ethoxy]-acetyl)2-(gamma-Glu)-CO-(CH2)16-CO 2H
  MISC_FEATURE (20)..(20): Xaa at position 20 is Aib
  MISC_FEATURE (24)..(24): Xaa at position 24 is D-Glu
  MISC_FEATURE (25)..(25): Xaa at position 25 is alpha-methyl-Tyr
  MOD_RES (39)..(39): Ser at position 39 is amidated
YXEGTXTSDXSIXLDXKAQXTFIXXLIEGGPSSGAPPPS

SEQ ID NO: 249 - protein, 39 aa, Artificial Sequence
  Synthetic Construct
  MISC_FEATURE (2)..(2): Xaa at position 2 is Aib
  MISC_FEATURE (6)..(6): Xaa at position 6 is alpha-methyl-Phe(2F)
  MISC_FEATURE (10)..(10): Xaa at position 10 is 4Pal
  MISC_FEATURE (13)..(13): Xaa at position 13 is alpha-methyl-Leu
  MISC_FEATURE (16)..(16): Xaa at position 16 is Orn
  MOD_RES (17)..(17): Lys at position 17 is chemically modified by conjugation of the epsilon-amino group of the Lys side chain with (2-[2-(2-amino-ethoxy)-ethoxy]-acetyl)2-(gamma-Glu)-CO-(CH2)16-CO 2H
  MISC_FEATURE (20)..(20): Xaa at position 20 is Aib
  MISC_FEATURE (24)..(24): Xaa at position 24 is D-Glu
  MISC_FEATURE (25)..(25): Xaa at position 25 is alpha-methyl-Tyr
  MOD_RES (39)..(39): Ser at position 39 is amidated
YXEGTXTSDXSIXLDXKAQXAFIXXLIEGGPSSGAPPPS

SEQ ID NO: 250 - protein, 39 aa, Artificial Sequence
  Synthetic Construct
  MISC_FEATURE (2)..(2): Xaa at position 2 is Aib
  MISC_FEATURE (6)..(6): Xaa at position 6 is alpha-methyl-Phe(2F)
  MISC_FEATURE (13)..(13): Xaa at position 13 is alpha-methyl-Leu
  MISC_FEATURE (16)..(16): Xaa at position 16 is Orn
  MOD_RES (17)..(17): Lys at position 17 is chemically modified by conjugation of the epsilon-amino group of the Lys side chain with (2-[2-(2-amino-ethoxy)-ethoxy]-acetyl)2-(gamma-Glu)-CO-(CH2)16-CO 2H
  MISC_FEATURE (20)..(20): Xaa at position 20 is Aib
  MISC_FEATURE (24)..(24): Xaa at position 24 is D-Glu
  MISC_FEATURE (25)..(25): Xaa at position 25 is alpha-methyl-Tyr
  MOD_RES (39)..(39): Ser at position 39 is amidated
YXEGTXTSDVSIXLDXKAQXTFIXXLIEGGPSSGAPPPS

SEQ ID NO: 251 - protein, 39 aa, Artificial Sequence
  Synthetic Construct
  MISC_FEATURE (2)..(2): Xaa at position 2 is Aib
  MISC_FEATURE (6)..(6): Xaa at position 6 is alpha-methyl-Phe(2F)
  MISC_FEATURE (13)..(13): Xaa at position 13 is alpha-methyl-Leu
  MISC_FEATURE (16)..(16): Xaa at position 16 is Orn
  MOD_RES (17)..(17): Lys at position 17 is chemically modified by conjugation of the epsilon-amino group of the Lys side chain with (2-[2-(2-amino-ethoxy)-ethoxy]-acetyl)2-(gamma-Glu)-CO-(CH2)16-CO 2H
  MISC_FEATURE (20)..(20): Xaa at position 20 is Aib
  MISC_FEATURE (24)..(24): Xaa at position 24 is D-Glu
  MISC_FEATURE (25)..(25): Xaa at position 25 is alpha-methyl-Tyr
  MOD_RES (39)..(39): Ser at position 39 is amidated
YXEGTXTSDVSIXLDXKAQXAFIXXLIEGGPSSGAPPPS

SEQ ID NO: 252 - protein, 39 aa, Artificial Sequence
  Synthetic Construct
  MISC_FEATURE (2)..(2): Xaa at position 2 is Aib
  MISC_FEATURE (6)..(6): Xaa at position 6 is alpha-methyl-Phe(2F)
  MISC_FEATURE (13)..(13): Xaa at position 13 is alpha-methyl-Leu
  MISC_FEATURE (16)..(16): Xaa at position 16 is Orn
  MOD_RES (17)..(17): Lys at position 17 is chemically modified by conjugation of the epsilon-amino group of the Lys side chain with (2-[2-(2-amino-ethoxy)-ethoxy]-acetyl)2-(gamma-Glu)-CO-(CH2)16-CO 2H
  MISC_FEATURE (20)..(20): Xaa at position 20 is Aib
  MISC_FEATURE (24)..(24): Xaa at position 24 is D-Glu
  MISC_FEATURE (25)..(25): Xaa at position 25 is alpha-methyl-Tyr
  MOD_RES (39)..(39): Ser at position 39 is amidated
YXEGTXTSDLSIXLDXKAQXTFIXXLIEGGPSSGAPPPS

SEQ ID NO: 253 - protein, 39 aa, Artificial Sequence
  Synthetic Construct
  MISC_FEATURE (2)..(2): Xaa at position 2 is Aib
  MISC_FEATURE (6)..(6): Xaa at position 6 is alpha-methyl-Phe(2F)
  MISC_FEATURE (13)..(13): Xaa at position 13 is alpha-methyl-Leu
  MISC_FEATURE (16)..(16): Xaa at position 16 is Orn
  MOD_RES (17)..(17): Lys at position 17 is chemically modified by conjugation of the epsilon-amino group of the Lys side chain with (2-[2-(2-amino-ethoxy)-ethoxy]-acetyl)2-(gamma-Glu)-CO-(CH2)16-CO 2H
  MISC_FEATURE (20)..(20): Xaa at position 20 is Aib
  MISC_FEATURE (24)..(24): Xaa at position 24 is D-Glu
  MISC_FEATURE (25)..(25): Xaa at position 25 is alpha-methyl-Tyr
  MOD_RES (39)..(39): Ser at position 39 is amidated
YXEGTXTSDLSIXLDXKAQXAFIXXLIEGGPSSGAPPPS

SEQ ID NO: 254 - protein, 39 aa, Artificial Sequence
  Synthetic Construct
  MISC_FEATURE (2)..(2): Xaa at position 2 is Aib
  MISC_FEATURE (6)..(6): Xaa at position 6 is alpha-methyl-Phe(2F)
  MISC_FEATURE (13)..(13): Xaa at position 13 is alpha-methyl-Leu
  MISC_FEATURE (16)..(16): Xaa at position 16 is Orn
  MOD_RES (17)..(17): Lys at position 17 is chemically modified by conjugation of the epsilon-amino group of the Lys side chain with (2-[2-(2-amino-ethoxy)-ethoxy]-acetyl)2-(gamma-Glu)-CO-(CH2)16-CO 2H
  MISC_FEATURE (20)..(20): Xaa at position 20 is Aib
  MISC_FEATURE (24)..(24): Xaa at position 24 is D-Glu
  MISC_FEATURE (25)..(25): Xaa at position 25 is alpha-methyl-Tyr
  MOD_RES (39)..(39): Ser at position 39 is amidated
YXEGTXTSDASIXLDXKAQXTFIXXLIEGGPSSGAPPPS

SEQ ID NO: 255 - protein, 39 aa, Artificial Sequence
  Synthetic Construct
  MISC_FEATURE (2)..(2): Xaa at position 2 is Aib
  MISC_FEATURE (6)..(6): Xaa at position 6 is alpha-methyl-Phe(2F)
  MISC_FEATURE (13)..(13): Xaa at position 13 is alpha-methyl-Leu
  MISC_FEATURE (16)..(16): Xaa at position 16 is Orn
  MOD_RES (17)..(17): Lys at position 17 is chemically modified by conjugation of the epsilon-amino group of the Lys side chain with (2-[2-(2-amino-ethoxy)-ethoxy]-acetyl)2-(gamma-Glu)-CO-(CH2)16-CO 2H
  MISC_FEATURE (20)..(20): Xaa at position 20 is Aib
  MISC_FEATURE (24)..(24): Xaa at position 24 is D-Glu
  MISC_FEATURE (25)..(25): Xaa at position 25 is alpha-methyl-Tyr
  MOD_RES (39)..(39): Ser at position 39 is amidated
YXEGTXTSDASIXLDXKAQXAFIXXLIEGGPSSGAPPPS

SEQ ID NO: 256 - protein, 39 aa, Artificial Sequence; identical to SEQ ID NO: 11
  Synthetic Construct
  MISC_FEATURE (2)..(2): Xaa at position 2 is Aib
  MISC_FEATURE (6)..(6): Xaa at position 6 is alpha-methyl-Phe(2F)
  MISC_FEATURE (13)..(13): Xaa at position 13 is Aib
  MISC_FEATURE (16)..(16): Xaa at position 16 is Orn
  MOD_RES (17)..(17): Lys at position 17 is chemically modified by conjugation of the epsilon-amino group of the Lys side chain with (2-[2-(2-amino-ethoxy)-ethoxy]-acetyl)2-(gamma-Glu)-CO-(CH2)16-CO 2H
  MISC_FEATURE (20)..(20): Xaa at position 20 is Aib
  MISC_FEATURE (24)..(24): Xaa at position 24 is D-Glu
  MOD_RES (39)..(39): Ser at position 39 is amidated

SEQ ID NO: 257 - protein, 39 aa, Artificial Sequence
  Synthetic Construct
  MISC_FEATURE (2)..(2): Xaa at position 2 is Aib
  MISC_FEATURE (6)..(6): Xaa at position 6 is alpha-methyl-Phe(2F)
  MISC_FEATURE (16)..(16): Xaa at position 16 is Orn
  MOD_RES (17)..(17): Lys at position 17 is chemically modified by conjugation of the epsilon-amino group of the Lys side chain with (2-[2-(2-amino-ethoxy)-ethoxy]-acetyl)2-(gamma-Glu)-CO-(CH2)16-CO 2H
  MISC_FEATURE (20)..(20): Xaa at position 20 is Aib
  MISC_FEATURE (24)..(24): Xaa at position 24 is D-Glu
  MOD_RES (39)..(39): Ser at position 39 is amidated
YXEGTXTSDYSILLDXKAQXEFIXYLIEGGPSSGAPPPS

SEQ ID NO: 258 - protein, 39 aa, Artificial Sequence; identical to SEQ ID NO: 11
  Synthetic Construct
  MISC_FEATURE (2)..(2): Xaa at position 2 is Aib
  MISC_FEATURE (6)..(6): Xaa at position 6 is alpha-methyl-Phe(2F)
  MISC_FEATURE (13)..(13): Xaa at position 13 is Nle
  MISC_FEATURE (16)..(16): Xaa at position 16 is Orn
  MOD_RES (17)..(17): Lys at position 17 is chemically modified by conjugation of the epsilon-amino group of the Lys side chain with (2-[2-(2-amino-ethoxy)-ethoxy]-acetyl)2-(gamma-Glu)-CO-(CH2)16-CO 2H
  MISC_FEATURE (20)..(20): Xaa at position 20 is Aib
  MISC_FEATURE (24)..(24): Xaa at position 24 is D-Glu
  MOD_RES (39)..(39): Ser at position 39 is amidated

SEQ ID NO: 259 - protein, 39 aa, Artificial Sequence; identical to SEQ ID NO: 11
  Synthetic Construct
  MISC_FEATURE (2)..(2): Xaa at position 2 is Aib
  MISC_FEATURE (6)..(6): Xaa at position 6 is alpha-methyl-Phe(2F)
  MISC_FEATURE (13)..(13): Xaa at position 13 is Aib
  MISC_FEATURE (16)..(16): Xaa at position 16 is Orn
  MOD_RES (17)..(17): Lys at position 17 is chemically modified by conjugation of the epsilon-amino group of the Lys side chain with (2-[2-(2-amino-ethoxy)-ethoxy]-acetyl)2-(gamma-Glu)-CO-(CH2)18-CO 2H
  MISC_FEATURE (20)..(20): Xaa at position 20 is Aib
  MISC_FEATURE (24)..(24): Xaa at position 24 is D-Glu
  MOD_RES (39)..(39): Ser at position 39 is amidated

SEQ ID NO: 260 - protein, 39 aa, Artificial Sequence; identical to SEQ ID NO: 249
  Synthetic Construct
  MISC_FEATURE (2)..(2): Xaa at position 2 is Aib
  MISC_FEATURE (6)..(6): Xaa at position 6 is alpha-methyl-Phe(2F)
  MISC_FEATURE (10)..(10): Xaa at position 10 is 4Pal
  MISC_FEATURE (13)..(13): Xaa at position 13 is alpha-methyl-Leu
  MISC_FEATURE (16)..(16): Xaa at position 16 is Orn
  MOD_RES (17)..(17): Lys at position 17 is chemically modified by conjugation of the epsilon-amino group of the Lys side chain with (2-[2-(2-amino-ethoxy)-ethoxy]-acetyl)2-(epsilon-Lys)-CO-(CH2)18- CO2H
  MISC_FEATURE (20)..(20): Xaa at position 20 is Aib
  MISC_FEATURE (24)..(24): Xaa at position 24 is D-Glu
  MISC_FEATURE (25)..(25): Xaa at position 25 is alpha-methyl-Tyr
  MOD_RES (39)..(39): Ser at position 39 is amidated

SEQ ID NO: 261 - protein, 39 aa, Artificial Sequence
  Synthetic Construct
  MISC_FEATURE (2)..(2): Xaa at position 2 is Aib
  MISC_FEATURE (6)..(6): Xaa at position 6 is alpha-methyl-Phe(2F)
  MISC_FEATURE (10)..(10): Xaa at position 10 is 4Pal
  MISC_FEATURE (13)..(13): Xaa at position 13 is alpha-methyl-Leu
  MISC_FEATURE (16)..(16): Xaa at position 16 is Orn
  MOD_RES (17)..(17): Lys at position 17 is chemically modified by conjugation of the epsilon-amino group of the Lys side chain with (2-[2-(2-amino-ethoxy)-ethoxy]-acetyl)2-(epsilon-Lys)-CO-(CH2)18- CO2H
  MISC_FEATURE (20)..(20): Xaa at position 20 is Aib
  MISC_FEATURE (24)..(24): Xaa at position 24 is D-Glu
  MISC_FEATURE (25)..(25): Xaa at position 25 is alpha-methyl-Tyr
  MOD_RES (39)..(39): Ser at position 39 is amidated
YXEGTXTSDXSIXLDXKAQXAFIXXLIAGGPSSGAPPPS

SEQ ID NO: 262 - protein, 39 aa, Artificial Sequence
  Synthetic Construct
  MISC_FEATURE (2)..(2): Xaa at position 2 is Aib
  MOD_RES (17)..(17): Lys at position 17 is chemically modified by conjugation of the epsilon-amino group of the Lys side chain with (2-[2-(2-amino-ethoxy)-ethoxy]-acetyl)2-(gamma-Glu)-CO-(CH2)18-CO 2H
  MOD_RES (39)..(39): Ser at position 39 is amidated
YXEGTFTSDYSILLDKKAQAAFIEYLIEGGPSSGAPPPS

SEQ ID NO: 263 - protein, 39 aa, Artificial Sequence
  Synthetic Construct
  MISC_FEATURE (2)..(2): Xaa at position 2 is Aib
  MOD_RES (17)..(17): Lys at position 17 is chemically modified by conjugation of the epsilon-amino group of the Lys side chain with (2-[2-(2-amino-ethoxy)-ethoxy]-acetyl)2-(gamma-Glu)-CO-(CH2)18-CO 2H
  MOD_RES (39)..(39): Ser at position 39 is amidated
YXEGTFTSDYSILLDKKAQQAFIEYLIEGGPSSGAPPPS

SEQ ID NO: 264 - protein, 39 aa, Artificial Sequence
  Synthetic Construct
  MISC_FEATURE (2)..(2): Xaa at position 2 is Aib
  MOD_RES (17)..(17): Lys at position 17 is chemically modified by conjugation of the epsilon-amino group of the Lys side chain with (2-[2-(2-amino-ethoxy)-ethoxy]-acetyl)2-(gamma-Glu)-CO-(CH2)18-CO 2H
  MOD_RES (39)..(39): Ser at position 39 is amidated
YXEGTFTSDYSILLDKKAQHAFIEYLIEGGPSSGAPPPS

SEQ ID NO: 265 - protein, 39 aa, Artificial Sequence
  Synthetic Construct
  MISC_FEATURE (2)..(2): Xaa at position 2 is Aib
  MOD_RES (17)..(17): Lys at position 17 is chemically modified by conjugation of the epsilon-amino group of the Lys side chain with (2-[2-(2-amino-ethoxy)-ethoxy]-acetyl)2-(gamma-Glu)-CO-(CH2)18-CO 2H
  MOD_RES (39)..(39): Ser at position 39 is amidated
YXEGTFTSDYSILLDKKAQKAFIEYLIEGGPSSGAPPPS

SEQ ID NO: 266 - protein, 39 aa, Artificial Sequence
  Synthetic Construct
  MISC_FEATURE (2)..(2): Xaa at position 2 is Aib
  MOD_RES (17)..(17): Lys at position 17 is chemically modified by conjugation of the epsilon-amino group of the Lys side chain with (2-[2-(2-amino-ethoxy)-ethoxy]-acetyl)2-(gamma-Glu)-CO-(CH2)18-CO 2H
  MOD_RES (39)..(39): Ser at position 39 is amidated
YXEGTFTSDYSILLDKKAQRAFIEYLIEGGPSSGAPPPS

SEQ ID NO: 267 - protein, 39 aa, Artificial Sequence
  Synthetic Construct
  MISC_FEATURE (2)..(2): Xaa at position 2 is Aib
  MOD_RES (17)..(17): Lys at position 17 is chemically modified by conjugation of the epsilon-amino group of the Lys side chain with (2-[2-(2-amino-ethoxy)-ethoxy]-acetyl)2-(gamma-Glu)-CO-(CH2)18-CO 2H
  MOD_RES (39)..(39): Ser at position 39 is amidated
YXEGTFTSDYSILLDEKAQKAFIEYLIEGGPSSGAPPPS

SEQ ID NO: 268 - protein, 39 aa, Artificial Sequence
  Synthetic Construct
  MISC_FEATURE (2)..(2): Xaa at position 2 is Aib
  MOD_RES (17)..(17): Lys at position 17 is chemically modified by conjugation of the epsilon-amino group of the Lys side chain with (2-[2-(2-amino-ethoxy)-ethoxy]-acetyl)2-(gamma-Glu)-CO-(CH2)18-CO 2H
  MISC_FEATURE (20)..(20): Xaa at position 20 is Aib
  MOD_RES (39)..(39): Ser at position 39 is amidated
YXEGTFTSDYSILLDEKAQXAFIEYLIEGGPSSGAPPPS

SEQ ID NO: 269 - protein, 39 aa, Artificial Sequence
  Synthetic Construct
  MISC_FEATURE (2)..(2): Xaa at position 2 is Aib
  MOD_RES (17)..(17): Lys at position 17 is chemically modified by conjugation of the epsilon-amino group of the Lys side chain with (2-[2-(2-amino-ethoxy)-ethoxy]-acetyl)2-(gamma-Glu)-CO-(CH2)18-CO 2H
  MISC_FEATURE (20)..(20): Xaa at position 20 is Aib
  MISC_FEATURE (39)..(39): Ser at position 39 is amidated
YXEGTFTSDHSILLDKKAQXAFIEYLIEGGPSSGAPPPS

SEQ ID NO: 270 - protein, 39 aa, Artificial Sequence
  Synthetic Construct
  MISC_FEATURE (2)..(2): Xaa at position 2 is Aib
  MOD_RES (17)..(17): Lys at position 17 is chemically modified by conjugation of the epsilon-amino group of the Lys side chain with (2-[2-(2-amino-ethoxy)-ethoxy]-acetyl)2-(gamma-Glu)-CO-(CH2)18-CO 2H
  MOD_RES (39)..(39): Ser at position 39 is amidated
YXEGTFTSDYSILLDKKAQEAFIEYLIEGGPSSGAPPPS

SEQ ID NO: 271 - protein, 39 aa, Artificial Sequence
  Synthetic Construct
  MISC_FEATURE (2)..(2): Xaa at position 2 is Aib
  MOD_RES (17)..(17): Lys at position 17 is chemically modified by conjugation of the epsilon-amino group of the Lys side chain with (2-[2-(2-amino-ethoxy)-ethoxy]-acetyl)2-(gamma-Glu)-CO-(CH2)18-CO 2H
  MOD_RES (39)..(39): Ser at position 39 is amidated
YXEGTFTSDYSILLDKKAQTAFIEYLIEGGPSSGAPPPS

SEQ ID NO: 272 - protein, 39 aa, Artificial Sequence
  Synthetic Construct
  MISC_FEATURE (2)..(2): Xaa at position 2 is Aib
  MOD_RES (17)..(17): Lys at position 17 is chemically modified by conjugation of the epsilon-amino group of the Lys side chain with (2-[2-(2-amino-ethoxy)-ethoxy]-acetyl)2-(gamma-Glu)-CO-(CH2)18-CO 2H
  MOD_RES (39)..(39): Ser at position 39 is amidated
YXEGTFTSDYSILLDKKAQSAFIEYLIEGGPSSGAPPPS

SEQ ID NO: 273 - protein, 34 aa, Artificial Sequence
  Synthetic Construct
  MISC_FEATURE (2)..(2): Xaa at position 2 is Aib
  MISC_FEATURE (6)..(6): Xaa at position 6 is alpha-methyl-Phe(2F)
  MISC_FEATURE (10)..(10): Xaa at position 10 is 4Pal
  MISC_FEATURE (13)..(13): Xaa at position 13 is alpha-methyl-Leu
  MISC_FEATURE (16)..(16): Xaa at position 16 is Orn
  MOD_RES (17)..(17): Lys at position 17 is chemically modified by conjugation of the epsilon-amino group of the Lys side chain with (2-[2-(2-amino-ethoxy)-ethoxy]-acetyl)2-(gamma-Glu)-CO-(CH2)16-CO 2H
  MISC_FEATURE (20)..(20): Xaa at position 20 is Aib
  MISC_FEATURE (24)..(24): Xaa at position 24 is D-Glu
  MISC_FEATURE (25)..(25): Xaa at position 25 is alpha-methyl-Tyr
  MOD_RES (34)..(34): Gly at position 34 is amidated
YXEGTXTSDXSIXLDXKAQXEFIXXLIEGGPSSG

SEQ ID NO: 274 - protein, 30 aa, Artificial Sequence
  Synthetic Construct
  MISC_FEATURE (2)..(2): Xaa at position 2 is Aib
  MISC_FEATURE (6)..(6): Xaa at position 6 is alpha-methyl-Phe(2F)
  MISC_FEATURE (10)..(10): Xaa at position 10 is 4Pal
  MISC_FEATURE (13)..(13): Xaa at position 13 is alpha-methyl-Leu
  MISC_FEATURE (16)..(16): Xaa at position 13 is Orn
  MOD_RES (17)..(17): Lys at position 17 is chemically modified by conjugation of the epsilon-amino group of the Lys side chain with (2-[2-(2-amino-ethoxy)-ethoxy]-acetyl)2-(gamma-Glu)-CO-(CH2)16-CO 2H
  MISC_FEATURE (20)..(20): Xaa at position 20 is Aib
  MISC_FEATURE (24)..(24): Xaa at position 24 is D-Glu
  MISC_FEATURE (25)..(25): Xaa at position 25 is alpha-methyl-Tyr
  MOD_RES (30)..(30): Gly at position 30 is amidated
YXEGTXTSDXSIXLDXKAQXEFIXXLIEGG

SEQ ID NO: 275 - protein, 34 aa, Artificial Sequence; identical to SEQ ID NO: 59
  Synthetic Construct
  MISC_FEATURE (2)..(2): Xaa at position 2 is Aib
  MOD_RES (17)..(17): Lys at position 17 is chemically modified by conjugation of the epsilon-amino group of the Lys side chain with (2-[2-(2-amino-ethoxy)-ethoxy]-acetyl)2-(gamma-Glu)-CO-(CH2)16-CO 2H
  MISC_FEATURE (20)..(20): Xaa at position 20 is Aib
  MOD_RES (34)..(34): Gly at position 34 is amidated

SEQ ID NO: 276 - protein, 30 aa, Artificial Sequence; identical to SEQ ID NO: 60
  Synthetic Construct
  MISC_FEATURE (2)..(2): Xaa at position 2 is Aib
  MOD_RES (17)..(17): Lys at position 17 is chemically modified by conjugation of the epsilon-amino group of the Lys side chain with (2-[2-(2-amino-ethoxy)-ethoxy]-acetyl)2-(gamma-Glu)-CO-(CH2)16-CO 2H
  MISC_FEATURE (20)..(20): Xaa at position 20 is Aib
  MOD_RES (30)..(30): Gly at position 30 is amidated

SEQ ID NO: 277 - protein, 34 aa, Artificial Sequence
  Synthetic Construct
  MISC_FEATURE (2)..(2): Xaa at position 2 is Aib
  MOD_RES (17)..(17): Lys at position 17 is chemically modified by conjugation of the epsilon-amino group of the Lys side chain with (2-[2-(2-amino-ethoxy)-ethoxy]-acetyl)2-(gamma-Glu)-CO-(CH2)16-CO 2H
  MISC_FEATURE (20)..(20): Xaa at position 20 is Aib
  MOD_RES (34)..(34): Gly at position 34 is amidated
YXEGTFTSDYSILLDEKAQXAFIEYLIEGGPSSG

SEQ ID NO: 278 - protein, 30 aa, Artificial Sequence
  Synthetic Construct
  MISC_FEATURE (2)..(2): Xaa at position 2 is Aib
  MOD_RES (17)..(17): Lys at position 17 is chemically modified by conjugation of the epsilon-amino group of the Lys side chain with (2-[2-(2-amino-ethoxy)-ethoxy]-acetyl)2-(gamma-Glu)-CO-(CH2)16-CO 2H
  MISC_FEATURE (20)..(20): Xaa at position 20 is Aib
  MISC_FEATURE (30)..(30): Gly at position 30 is amidated
YXEGTFTSDYSILLDEKAQXAFIEYLIEGG

SEQ ID NO: 279 - protein, 34 aa, Artificial Sequence
  Synthetic Construct
  MISC_FEATURE (2)..(2): Xaa at position 2 is Aib
  MOD_RES (17)..(17): Lys at position 17 is chemically modified by conjugation of the epsilon-amino group of the Lys side chain with (2-[2-(2-amino-ethoxy)-ethoxy]-acetyl)2-(gamma-Glu)-CO-(CH2)16-CO 2H
  MISC_FEATURE (20)..(20): Xaa at position 20 is Aib
  MOD_RES (34)..(34): Gly at position 34 is amidated
YXEGTFTSDYSILLDKKAQXEFIEYLIEGGPSSG

SEQ ID NO: 280 - protein, 30 aa, Artificial Sequence
  Synthetic Construct
  MISC_FEATURE (2)..(2): Xaa at position 2 is Aib
  MOD_RES (17)..(17): Lys at position 17 is chemically modified by conjugation of the epsilon-amino group of the Lys side chain with (2-[2-(2-amino-ethoxy)-ethoxy]-acetyl)2-(gamma-Glu)-CO-(CH2)16-CO 2H
  MISC_FEATURE (20)..(20): Xaa at position 20 is Aib
  MOD_RES (30)..(30): Gly at position 30 is amidated
YXEGTFTSDYSILLDKKAQXEFIEYLIEGG

SEQ ID NO: 281 - protein, 34 aa, Artificial Sequence
  Synthetic Construct
  MISC_FEATURE (2)..(2): Xaa at position 2 is Aib
  MOD_RES (17)..(17): Lys at position 17 is chemically modified by conjugation of the epsilon-amino group of the Lys side chain with (2-[2-(2-amino-ethoxy)-ethoxy]-acetyl)2-(gamma-Glu)-CO-(CH2)16-CO 2H
  MISC_FEATURE (20)..(20): Xaa at position 20 is Aib
  MOD_RES (34)..(34): Gly at position 34 is amidated
YXEGTFTSDYSILLDKKAQXAFIEYLIAGGPSSG

SEQ ID NO: 282 - protein, 30 aa, Artificial Sequence
  Synthetic Construct
  MISC_FEATURE (2)..(2): Xaa at position 2 is Aib
  MOD_RES (17)..(17): Lys at position 17 is chemically modified by conjugation of the epsilon-amino group of the Lys side chain with (2-[2-(2-amino-ethoxy)-ethoxy]-acetyl)2-(gamma-Glu)-CO-(CH2)16-CO 2H
  MISC_FEATURE (20)..(20): Xaa at position 20 is Aib
  MOD_RES (30)..(30): Gly at position 30 is amidated
YXEGTFTSDYSILLDKKAQXAFIEYLIAGG

SEQ ID NO: 283 - protein, 34 aa, Artificial Sequence
  Synthetic Construct
  MISC_FEATURE (2)..(2): Xaa at position 2 is Aib
  MOD_RES (17)..(17): Lys at position 17 is chemically modified by conjugation of the epsilon-amino group of the Lys side chain with (2-[2-(2-amino-ethoxy)-ethoxy]-acetyl)2-(gamma-Glu)-CO-(CH2)16-CO 2H
  MOD_RES (34)..(34): Gly at position 34 is amidated
YXEGTFTSDYSILLDKKAQPAFIEYLIEGGPSSG

SEQ ID NO: 284 - protein, 30 aa, Artificial Sequence
  Synthetic Construct
  MISC_FEATURE (2)..(2): Xaa at position 2 is Aib
  MOD_RES (17)..(17): Lys at position 17 is chemically modified by conjugation of the epsilon-amino group of the Lys side chain with (2-[2-(2-amino-ethoxy)-ethoxy]-acetyl)2-(gamma-Glu)-CO-(CH2)16-CO 2H
  MOD_RES (30)..(30): Gly at position 30 is amidated
YXEGTFTSDYSILLDKKAQPAFIEYLIEGG

SEQ ID NO: 285 - protein, 39 aa, Artificial Sequence; identical to SEQ ID NO: 10
  Synthetic Construct
  MISC_FEATURE (2)..(2): Xaa at position 2 is Aib
  MISC_FEATURE (6)..(6): Xaa at position 6 is alpha-methyl-Phe(2F)
  MISC_FEATURE (13)..(13): Xaa at position 13 is alpha-methyl-Leu
  MISC_FEATURE (20)..(20): Xaa at position 20 is Aib
  MISC_FEATURE (24)..(24): Xaa at position 24 is D-Glu
  MOD_RES (39)..(39): Ser at position 39 is amidated

SEQ ID NO: 286 - protein, 39 aa, Artificial Sequence
  Synthetic Construct
  MISC_FEATURE (2)..(2): Xaa at position 2 is Aib
  MISC_FEATURE (6)..(6): Xaa at position 6 is alpha-methyl-Phe(2F)
  MISC_FEATURE (13)..(13): Xaa at position 13 is alpha-methyl-Leu
  MISC_FEATURE (20)..(20): Xaa at position 20 is Aib
  MISC_FEATURE (24)..(24): Xaa at position 24 is D-Glu
  MOD_RES (39)..(39): Ser at position 39 is amidated
YXEGTXTSDYSIXLDEQAQXEFIXYLIEGGPSSGAPPPS

SEQ ID NO: 287 - protein, 40 aa, Artificial Sequence
  Synthetic Construct
  MISC_FEATURE (2)..(2): Xaa at position 2 is Aib
  MISC_FEATURE (6)..(6): Xaa at position 6 is alpha-methyl-Phe(2F)
  MISC_FEATURE (13)..(13): Xaa at position 13 is alpha-methyl-Leu
  MISC_FEATURE (20)..(20): Xaa at position 20 is Aib
  MISC_FEATURE (24)..(24): Xaa at position 24 is D-Glu
  MOD_RES (40)..(40): Cys at position 40 is amidated
YXEGTXTSDYSIXLDEKAQXEFIXYLIEGGPSSGAPPPSC

SEQ ID NO: 288 - protein, 40 aa, Artificial Sequence
  Synthetic Construct
  MISC_FEATURE (2)..(2): Xaa at position 2 is Aib
  MISC_FEATURE (6)..(6): Xaa at position 6 is alpha-methyl-Phe(2F)
  MISC_FEATURE (13)..(13): Xaa at position 13 is alpha-methyl-Leu
  MISC_FEATURE (20)..(20): Xaa at position 20 is Aib
  MISC_FEATURE (24)..(24): Xaa at position 24 is D-Glu
  MOD_RES (40)..(40): Cys at position 40 is amidated
YXEGTXTSDYSIXLDEQAQXEFIXYLIEGGPSSGAPPPSC

SEQ ID NO: 289 - protein, 39 aa, Artificial Sequence; identical to SEQ ID NO: 11
  Synthetic Construct
  MISC_FEATURE (2)..(2): Xaa at position 2 is Aib
  MISC_FEATURE (6)..(6): Xaa at position 6 is alpha-methyl-Phe(2F)
  MISC_FEATURE (13)..(13): Xaa at position 13 is alpha-methyl-Leu
  MISC_FEATURE (16)..(16): Xaa at position 16 is Orn
  MISC_FEATURE (20)..(20): Xaa at position 20 is Aib
  MISC_FEATURE (24)..(24): Xaa at position 24 is D-Glu
  MOD_RES (39)..(39): Ser at position 39 is amidated

SEQ ID NO: 290 - protein, 39 aa, Artificial Sequence
  Synthetic Construct
  MISC_FEATURE (2)..(2): Xaa at position 2 is Aib
  MISC_FEATURE (6)..(6): Xaa at position 6 is alpha-methyl-Phe(2F)
  MISC_FEATURE (13)..(13): Xaa at position 13 is alpha-methyl-Leu
  MISC_FEATURE (16)..(16): Xaa at position 16 is Orn
  MISC_FEATURE (20)..(20): Xaa at position 20 is Aib
  MISC_FEATURE (24)..(24): Xaa at position 24 is D-Glu
  MOD_RES (39)..(39): Ser at position 39 is amidated
YXEGTXTSDYSIXLDXQAQXEFIXYLIEGGPSSGAPPPS

SEQ ID NO: 291 - protein, 40 aa, Artificial Sequence
  Synthetic Construct
  MISC_FEATURE (2)..(2): Xaa at position 2 is Aib
  MISC_FEATURE (6)..(6): Xaa at position 6 is alpha-methyl-Phe(2F)
  MISC_FEATURE (13)..(13): Xaa at position 13 is alpha-methyl-Leu
  MISC_FEATURE (16)..(16): Xaa at position 16 is Orn
  MISC_FEATURE (20)..(20): Xaa at position 20 is Aib
  MISC_FEATURE (24)..(24): Xaa at position 24 is D-Glu
  MOD_RES (40)..(40): Cys at position 40 is amidated
YXEGTXTSDYSIXLDXKAQXEFIXYLIEGGPSSGAPPPSC

SEQ ID NO: 292 - protein, 40 aa, Artificial Sequence
  Synthetic Construct
  MISC_FEATURE (2)..(2): Xaa at position 2 is Aib
  MISC_FEATURE (6)..(6): Xaa at position 6 is alpha-methyl-Phe(2F)
  MISC_FEATURE (13)..(13): Xaa at position 13 is alpha-methyl-Leu
  MISC_FEATURE (16)..(16): Xaa at position 16 is Orn
  MISC_FEATURE (20)..(20): Xaa at position 20 is Aib
  MISC_FEATURE (24)..(24): Xaa at position 24 is D-Glu
  MOD_RES (40)..(40): Cys at position 40 is amidated
YXEGTXTSDYSIXLDXQAQXEFIXYLIEGGPSSGAPPPSC

SEQ ID NO: 293 - protein, 39 aa, Artificial Sequence; identical to SEQ ID NO: 13
  Synthetic Construct
  MISC_FEATURE (2)..(2): Xaa at position 2 is Aib
  MISC_FEATURE (6)..(6): Xaa at position 6 is alpha-methyl-Phe(2F)
  MISC_FEATURE (10)..(10): Xaa at position 10 is 4Pal
  MISC_FEATURE (13)..(13): Xaa at position 13 is alpha-methyl-Leu
  MISC_FEATURE (16)..(16): Xaa at position 16 is Orn
  MISC_FEATURE (20)..(20): Xaa at position 20 is Aib
  MISC_FEATURE (24)..(24): Xaa at position 24 is D-Glu
  MISC_FEATURE (25)..(25): Xaa at position 25 is alpha-methyl-Tyr
  MOD_RES (39)..(39): Ser at position 39 is amidated

SEQ ID NO: 294 - protein, 39 aa, Artificial Sequence
  Synthetic Construct
  MISC_FEATURE (2)..(2): Xaa at position 2 is Aib
  MISC_FEATURE (6)..(6): Xaa at position 6 is alpha-methyl-Phe(2F)
  MISC_FEATURE (10)..(10): Xaa at position 10 is 4Pal
  MISC_FEATURE (13)..(13): Xaa at position 13 is alpha-methyl-Leu
  MISC_FEATURE (16)..(16): Xaa at position 16 is Orn
  MISC_FEATURE (20)..(20): Xaa at position 20 is Aib
  MISC_FEATURE (24)..(24): Xaa at position 24 is D-Glu
  MISC_FEATURE (25)..(25): Xaa at position 25 is alpha-methyl-Tyr
  mod (39)..(39): Ser at position 39 is amidated
YXEGTXTSDXSIXLDXQAQXEFIXXLIEGGPSSGAPPPS

SEQ ID NO: 295 - protein, 40 aa, Artificial Sequence
  Synthetic Construct
  MISC_FEATURE (2)..(2): Xaa at position 2 is Aib
  MISC_FEATURE (6)..(6): Xaa at position 6 is alpha-methyl-Phe(2F)
  MISC_FEATURE (10)..(10): Xaa at position 10 is 4Pal
  MISC_FEATURE (13)..(13): Xaa at position 13 is alpha-methyl-Leu
  MISC_FEATURE (16)..(16): Xaa at position 16 is Orn
  MISC_FEATURE (20)..(20): Xaa at position 20 is Aib
  MISC_FEATURE (24)..(24): Xaa at position 24 is D-Glu
  MISC_FEATURE (25)..(25): Xaa at position 25 is alpha-methyl-Tyr
  MOD_RES (40)..(40): Cys at position 40 is amidated
YXEGTXTSDXSIXLDXKAQXEFIXXLIEGGPSSGAPPPSC

SEQ ID NO: 296 - protein, 40 aa, Artificial Sequence
  Synthetic Construct
  MISC_FEATURE (2)..(2): Xaa at position 2 is Aib
  MISC_FEATURE (6)..(6): Xaa at position 6 is alpha-methyl-Phe(2F)
  MISC_FEATURE (10)..(10): Xaa at position 10 is 4Pal
  MISC_FEATURE (13)..(13): Xaa at position 13 is alpha-methyl-Leu
  MISC_FEATURE (16)..(16): Xaa at position 16 is Orn
  MISC_FEATURE (20)..(20): Xaa at position 20 is Aib
  MISC_FEATURE (24)..(24): Xaa at position 24 is D-Glu
  MISC_FEATURE (25)..(25): Xaa at position 25 is alpha-methyl-Tyr
  MOD_RES (40)..(40): Cys at position 40 is amidated
YXEGTXTSDXSIXLDXQAQXEFIXXLIEGGPSSGAPPPSC

SEQ ID NO: 297 - protein, 4 aa, Artificial Sequence
  Synthetic Construct
  MOD_RES (4)..(4): The C-terminal Gly is modified with R2 to provide PSSG-R2, wherein the modification is NH2 or absent.
PSSG

SEQ ID NO: 298 - protein, 9 aa, Artificial Sequence
  Synthetic Construct
  MOD_RES (9)..(9): The C-terminal Ser is modified with R2 to provide PSSGAPPPS-R2, wherein the modification is NH2 or absent.
PSSGAPPPS

SEQ ID NO: 299 - protein, 4 aa, Artificial Sequence
  Synthetic Construct
PSSG

SEQ ID NO: 300 - protein, 4 aa, Artificial Sequence
  Synthetic Construct
  MOD_RES (4)..(4): Gly at position 4 is amidated
PSSG

SEQ ID NO: 301 - protein, 9 aa, Artificial Sequence
  Synthetic Construct
PSSGAPPPS

SEQ ID NO: 302 - protein, 9 aa, Artificial Sequence
  Synthetic Construct
  MOD_RES (9)..(9): Ser at position 9 is amidated
PSSGAPPPS

SEQ ID NO: 303 - protein, 39 aa, Artificial Sequence
  Synthetic Construct
  MISC_FEATURE (2)..(2): Xaa at position 2 is Aib
  MOD_RES (17)..(17): Lys at position 17 is chemically modified by conjugation of the epsilon-amino group of the Lys side chain with (2-[2-(2-amino-ethoxy)-ethoxy]-acetyl)2-(gamma-Glu)-CO-(CH2)18-CO 2H
  MISC_FEATURE (20)..(20): Xaa at position 20 is Aib
  MOD_RES (39)..(39): Ser at position 39 is amidated
YXEGTFTSDYSILLDKKAQXAFIEYLIAGGPSSGAPPPS

SEQ ID NO: 304 - protein, 39 aa, Artificial Sequence
  Synthetic Construct
  MISC_FEATURE (2)..(2): Xaa at position 2 is Aib
  MISC_FEATURE (13)..(13): Xaa at position 13 is alpha-methyl-Leu
  MOD_RES (17)..(17): Lys at position 17 is chemically modified by conjugation of the epsilon-amino group of the Lys side chain with (2-[2-(2-amino-ethoxy)-ethoxy]-acetyl)2-(gamma-Glu)-CO-(CH2)18-CO 2H
  MISC_FEATURE (20)..(20): Xaa at position 20 is Aib
  MOD_RES (39)..(39): Ser at position 39 is amidated
YXEGTFTSDYSIXLDKKAQXEFIEYLIAGGPSSGAPPPS

SEQ ID NO: 305 - protein, 39 aa, Artificial Sequence
  Synthetic Construct
  MISC_FEATURE (1)..(1): Xaa at position 1 is D-Tyr
  MISC_FEATURE (2)..(2): Xaa at position 2 is Aib
  MISC_FEATURE (13)..(13): Xaa at position 13 is alpha-methyl-Leu
  MOD_RES (17)..(17): Lys at position 17 is chemically modified by conjugation of the epsilon-amino group of the Lys side chain with (2-[2-(2-amino-ethoxy)-ethoxy]-acetyl)2-(gamma-Glu)-CO-(CH2)18-CO 2H
  MISC_FEATURE (20)..(20): Xaa at position 20 is Aib
  MOD_RES (39)..(39): Ser at position 39 is amidated
XXEGTFTSDYSIXLDKKAQXEFIEYLIAGGPSSGAPPPS

SEQ ID NO: 306 - protein, 39 aa, Artificial Sequence
  Synthetic Construct
  MISC_FEATURE (1)..(1): Xaa at position 1 is D-Tyr
  MISC_FEATURE (2)..(2): Xaa at position 2 is Aib
  MISC_FEATURE (13)..(13): Xaa at position 13 is alpha-methyl-Leu
  MISC_FEATURE (16)..(16): Xaa at position 16 is Orn
  MOD_RES (17)..(17): Lys at position 17 is chemically modified by conjugation of the epsilon-amino group of the Lys side chain with (2-[2-(2-amino-ethoxy)-ethoxy]-acetyl)2-(gamma-Glu)-CO-(CH2)18-CO 2H
  MISC_FEATURE (20)..(20): Xaa at position 20 is Aib
  MISC_FEATURE (24)..(24): Xaa at position 24 is D-Glu
  MOD_RES (39)..(39): Ser at position 39 is amidated
XXEGTFTSDYSIXLDXKAQXAFIXYLIAGGPSSGAPPPS

SEQ ID NO: 307 - protein, 39 aa, Artificial Sequence
  Synthetic Construct
  MISC_FEATURE (1)..(1): Xaa at position 1 is D-Tyr
  MISC_FEATURE (2)..(2): Xaa at position 2 is Aib
  MISC_FEATURE (13)..(13): Xaa at position 13 is alpha-methyl-Leu
  MOD_RES (17)..(17): Lys at position 17 is chemically modified by conjugation of the epsilon-amino group of the Lys side chain with (2-[2-(2-amino-ethoxy)-ethoxy]-acetyl)2-(gamma-Glu)-CO-(CH2)18-CO 2H
  MISC_FEATURE (20)..(20): Xaa at position 20 is Aib
  MISC_FEATURE (25)..(25): Xaa at position 25 is alpha-methyl-Tyr
  MOD_RES (39)..(39): Ser at position 39 is amidated
XXEGTFTSDYSIXLDKKAQXEFIEXLIAGGPSSGAPPPS

SEQ ID NO: 308 - protein, 39 aa, Artificial Sequence
  Synthetic Construct
  MISC_FEATURE (1)..(1): Xaa at position 1 is D-Tyr
  MISC_FEATURE (2)..(2): Xaa at position 2 is Aib
  MISC_FEATURE (13)..(13): Xaa at position 13 is alpha-methyl-Leu
  MISC_FEATURE (16)..(16): Xaa at position 16 is Orn
  MOD_RES (17)..(17): Lys at position 17 is chemically modified by conjugation of the epsilon-amino group of the Lys side chain with (2-[2-(2-amino-ethoxy)-ethoxy]-acetyl)2-(gamma-Glu)-CO-(CH2)18-CO 2H
  MISC_FEATURE (20)..(20): Xaa at position 20 is Aib
  MISC_FEATURE (25)..(25): Xaa at position 25 is alpha-methyl-Tyr
  MOD_RES (39)..(39): Ser at position 39 is amidated
XXEGTFTSDYSIXLDXKAQXEFIEXLIAGGPSSGAPPPS

SEQ ID NO: 309 - protein, 30 aa, Artificial Sequence
  Synthetic Construct
  MISC_FEATURE (2)..(2): Xaa at position 2 is Aib
  MOD_RES (17)..(17): Lys at position 17 is chemically modified by conjugation of the epsilon-amino group of the Lys side chain with (2-[2-(2-amino-ethoxy)-ethoxy]-acetyl)2-(gamma-Glu)-CO-(CH2)16-CO 2H
  MOD_RES (30)..(30): Gly at position 30 is amidated
YXEGTFTSDYSILLDKKAQQAFIEYLIEGG

SEQ ID NO: 310 - protein, 30 aa, Artificial Sequence
  Synthetic Construct
  MISC_FEATURE (2)..(2): Xaa at position 2 is Aib
  MOD_RES (17)..(17): Lys at position 17 is chemically modified by conjugation of the epsilon-amino group of the Lys side chain with (2-[2-(2-amino-ethoxy)-ethoxy]-acetyl)2-(gamma-Glu)-CO-(CH2)16-CO 2H
  MOD_RES (30)..(30): Gly at position 30 is amidated
YXEGTFTSDYSILLDKKAQHAFIEYLIEGG

SEQ ID NO: 311 - protein, 34 aa, Artificial Sequence
  Synthetic Construct
  MISC_FEATURE (2)..(2): Xaa at position 2 is Aib
  MOD_RES (17)..(17): Lys at position 17 is chemically modified by conjugation of the epsilon-amino group of the Lys side chain with (2-[2-(2-amino-ethoxy)-ethoxy]-acetyl)2-(gamma-Glu)-CO-(CH2)16-CO 2H
  MOD_RES (34)..(34): Gly at position 34 is amidated
YXEGTFTSDYSILLDKKAQKAFIEYLIEGGPSSG

SEQ ID NO: 312 - protein, 30 aa, Artificial Sequence
  Synthetic Construct
  MISC_FEATURE (2)..(2): Xaa at position 2 is Aib
  MOD_RES (17)..(17): Lys at position 17 is chemically modified by conjugation of the epsilon-amino group of the Lys side chain with (2-[2-(2-amino-ethoxy)-ethoxy]-acetyl)2-(gamma-Glu)-CO-(CH2)16-CO 2H
  MISC_FEATURE (20)..(20): Xaa at position 20 is Aib
  MOD_RES (30)..(30): Gly at position 30 is amidated
YXEGTFTSDYSILLDKKAQXEFIEYLIAGG

SEQ ID NO: 313 - protein, 34 aa, Artificial Sequence
  Synthetic Construct
  MISC_FEATURE (2)..(2): Xaa at position 2 is Aib
  MOD_RES (17)..(17): Lys at position 17 is chemically modified by conjugation of the epsilon-amino group of the Lys side chain with (2-[2-(2-amino-ethoxy)-ethoxy]-acetyl)2-(gamma-Glu)-CO-(CH2)16-CO 2H
  MISC_FEATURE (20)..(20): Xaa at position 20 is Aib
  MOD_RES (34)..(34): Gly at position 34 is amidated
YXEGTFTSDYSILLDKKAQXAFVEYLIEGGPSSG

SEQ ID NO: 314 - protein, 34 aa, Artificial Sequence
  Synthetic Construct
  MISC_FEATURE (2)..(2): Xaa at position 2 is Aib
  MOD_RES (17)..(17): Lys at position 17 is chemically modified by conjugation of the epsilon-amino group of the Lys side chain with (2-[2-(2-amino-ethoxy)-ethoxy]-acetyl)2-(gamma-Glu)-CO-(CH2)16-CO 2H
  MISC_FEATURE (20)..(20): Xaa at position 20 is Aib
  MOD_RES (34)..(34): Gly at position 34 is amidated
YXEGTFTSDYSILLDKKAQXAFLEYLIEGGPSSG

SEQ ID NO: 315 - protein, 34 aa, Artificial Sequence
  Synthetic Construct
  MISC_FEATURE (2)..(2): Xaa at position 2 is Aib
  MISC_FEATURE (13)..(13): Xaa at position 13 is alpha-methyl-Leu
  MOD_RES (17)..(17): Lys at position 17 is chemically modified by conjugation of the epsilon-amino group of the Lys side chain with (2-[2-(2-amino-ethoxy)-ethoxy]-acetyl)2-(gamma-Glu)-CO-(CH2)16-CO 2H
  MISC_FEATURE (20)..(20): Xaa at position 20 is Aib
  MOD_RES (34)..(34): Gly at position 34 is amidated
YXEGTFTSDYSIXLDKKAQXAFIEYLIEGGPSSG

SEQ ID NO: 316 - protein, 34 aa, Artificial Sequence
  Synthetic Construct
  MISC_FEATURE (2)..(2): Xaa at position 2 is Aib
  MISC_FEATURE (6)..(6): Xaa at position 6 is alpha-methyl-Phe
  MOD_RES (17)..(17): Lys at position 17 is chemically modified by conjugation of the epsilon-amino group of the Lys side chain with (2-[2-(2-amino-ethoxy)-ethoxy]-acetyl)2-(gamma-Glu)-CO-(CH2)16-CO 2H
  MISC_FEATURE (20)..(20): Xaa at position 20 is Aib
  MOD_RES (34)..(34): Gly at position 34 is amidated
YXEGTXTSDYSILLDKKAQXAFIEYLIEGGPSSG

SEQ ID NO: 317 - protein, 34 aa, Artificial Sequence; identical to SEQ ID NO: 316
  Synthetic Construct
  MISC_FEATURE (2)..(2): Xaa at position 2 is Aib
  MISC_FEATURE (6)..(6): Xaa at position 6 is alpha-methyl-Phe(2F)
  MOD_RES (17)..(17): Lys at position 17 is chemically modified by conjugation of the epsilon-amino group of the Lys side chain with (2-[2-(2-amino-ethoxy)-ethoxy]-acetyl)2-(gamma-Glu)-CO-(CH2)16-CO 2H
  MISC_FEATURE (20)..(20): Xaa at position 20 is Aib
  MOD_RES (34)..(34): Gly at position 34 is amidated

SEQ ID NO: 318 - protein, 34 aa, Artificial Sequence
  Synthetic Construct
  MISC_FEATURE (2)..(2): Xaa at position 2 is Aib
  MISC_FEATURE (13)..(13): Xaa at position 13 is alpha-methyl-Leu
  MOD_RES (17)..(17): Lys at position 17 is chemically modified by conjugation of the epsilon-amino group of the Lys side chain with (2-[2-(2-amino-ethoxy)-ethoxy]-acetyl)2-(gamma-Glu)-CO-(CH2)16-CO 2H
  MISC_FEATURE (20)..(20): Xaa at position 20 is Aib
  MOD_RES (34)..(34): Gly at position 34 is amidated
YXEGTFTSDYSIXLDEKAQXAFIEYLIEGGPSSG

SEQ ID NO: 319 - protein, 34 aa, Artificial Sequence
  Synthetic Construct
  MISC_FEATURE (2)..(2): Xaa at position 2 is Aib
  MISC_FEATURE (13)..(13): Xaa at position 13 is alpha-methyl-Leu
  MOD_RES (17)..(17): Lys at position 17 is chemically modified by conjugation of the epsilon-amino group of the Lys side chain with (2-[2-(2-amino-ethoxy)-ethoxy]-acetyl)2-(gamma-Glu)-CO-(CH2)16-CO 2H
  MISC_FEATURE (20)..(20): Xaa at position 20 is Aib
  MOD_RES (34)..(34): Gly at position 34 is amidated
YXEGTFTSDYSIXLDKKAQXEFIEYLIEGGPSSG

SEQ ID NO: 320 - protein, 34 aa, Artificial Sequence
  Synthetic Construct
  MISC_FEATURE (2)..(2): Xaa at position 2 is Aib
  MISC_FEATURE (13)..(13): Xaa at position 13 is alpha-methyl-Leu
  MOD_RES (17)..(17): Lys at position 17 is chemically modified by conjugation of the epsilon-amino group of the Lys side chain with (2-[2-(2-amino-ethoxy)-ethoxy]-acetyl)2-(gamma-Glu)-CO-(CH2)16-CO 2H
  MISC_FEATURE (20)..(20): Xaa at position 20 is Aib
  MOD_RES (34)..(34): Gly at position 34 is amidated
YXEGTFTSDYSIXLDKKAQXAFIEYLIAGGPSSG

SEQ ID NO: 321 - protein, 34 aa, Artificial Sequence
  Synthetic Construct
  MISC_FEATURE (2)..(2): Xaa at position 2 is Aib
  MISC_FEATURE (13)..(13): Xaa at position 13 is alpha-methyl-Leu
  MOD_RES (17)..(17): Lys at position 17 is chemically modified by conjugation of the epsilon-amino group of the Lys side chain with (2-[2-(2-amino-ethoxy)-ethoxy]-acetyl)2-(gamma-Glu)-CO-(CH2)16-CO 2H
  MISC_FEATURE (20)..(20): Xaa at position 20 is Aib
  MOD_RES (34)..(34): Gly at position 34 is amidated
YXEGTFTSDYSIXLDKKAQXEFIEYLIAGGPSSG

SEQ ID NO: 322 - protein, 34 aa, Artificial Sequence
  Synthetic Construct
  MISC_FEATURE (2)..(2): Xaa at position 2 is Aib
  MISC_FEATURE (6)..(6): Xaa at position 6 is alpha-methyl-Phe
  MOD_RES (17)..(17): Lys at position 17 is chemically modified by conjugation of the epsilon-amino group of the Lys side chain with (2-[2-(2-amino-ethoxy)-ethoxy]-acetyl)2-(gamma-Glu)-CO-(CH2)16-CO 2H
  MISC_FEATURE (20)..(20): Xaa at position 20 is Aib
  MOD_RES (34)..(34): Gly at position 34 is amidated
YXEGTXTSDYSILLDEKAQXAFIEYLIEGGPSSG

SEQ ID NO: 323 - protein, 34 aa, Artificial Sequence
  Synthetic Construct
  MISC_FEATURE (2)..(2): Xaa at position 2 is Aib
  MISC_FEATURE (6)..(6): Xaa at position 6 is alpha-methyl-Phe
  MOD_RES (17)..(17): Lys at position 17 is chemically modified by conjugation of the epsilon-amino group of the Lys side chain with (2-[2-(2-amino-ethoxy)-ethoxy]-acetyl)2-(gamma-Glu)-CO-(CH2)16-CO 2H
  MISC_FEATURE (20)..(20): Xaa at position 20 is Aib
  MOD_RES (34)..(34): Gly at position 34 is amidated
YXEGTXTSDYSILLDKKAQXEFIEYLIEGGPSSG

SEQ ID NO: 324 - protein, 34 aa, Artificial Sequence
  Synthetic Construct
  MISC_FEATURE (2)..(2): Xaa at position 2 is Aib
  MISC_FEATURE (6)..(6): Xaa at position 6 is alpha-methyl-Phe
  MOD_RES (17)..(17): Lys at position 17 is chemically modified by conjugation of the epsilon-amino group of the Lys side chain with (2-[2-(2-amino-ethoxy)-ethoxy]-acetyl)2-(gamma-Glu)-CO-(CH2)16-CO 2H
  MISC_FEATURE (20)..(20): Xaa at position 20 is Aib
  MOD_RES (34)..(34): Gly at position 34 is amidated
YXEGTXTSDYSILLDKKAQXAFIEYLIAGGPSSG

SEQ ID NO: 325 - protein, 34 aa, Artificial Sequence
  Synthetic Construct
  MISC_FEATURE (2)..(2): Xaa at position 2 is Aib
  MISC_FEATURE (6)..(6): Xaa at position 6 is alpha-methyl-Phe
  MOD_RES (17)..(17): Lys at position 17 is chemically modified by conjugation of the epsilon-amino group of the Lys side chain with (2-[2-(2-amino-ethoxy)-ethoxy]-acetyl)2-(gamma-Glu)-CO-(CH2)16-CO 2H
  MISC_FEATURE (20)..(20): Xaa at position 20 is Aib
  MOD_RES (34)..(34): Gly at position 34 is amidated
YXEGTXTSDYSILLDKKAQXEFIEYLIAGGPSSG

SEQ ID NO: 326 - protein, 34 aa, Artificial Sequence; identical to SEQ ID NO: 322
  Synthetic Construct
  MISC_FEATURE (2)..(2): Xaa at position 2 is Aib
  MISC_FEATURE (6)..(6): Xaa at position 6 is alpha-methyl-Phe(2F)
  MOD_RES (17)..(17): Lys at position 17 is chemically modified by conjugation of the epsilon-amino group of the Lys side chain with (2-[2-(2-amino-ethoxy)-ethoxy]-acetyl)2-(gamma-Glu)-CO-(CH2)16-CO 2H
  MISC_FEATURE (20)..(20): Xaa at position 20 is Aib
  MOD_RES (34)..(34): Gly at position 34 is amidated

SEQ ID NO: 327 - protein, 34 aa, Artificial Sequence; identical to SEQ ID NO: 323
  Synthetic Construct
  MISC_FEATURE (2)..(2): Xaa at position 2 is Aib
  MISC_FEATURE (6)..(6): Xaa at position 6 is alpha-methyl-Phe(2F)
  MOD_RES (17)..(17): Lys at position 17 is chemically modified by conjugation of the epsilon-amino group of the Lys side chain with (2-[2-(2-amino-ethoxy)-ethoxy]-acetyl)2-(gamma-Glu)-CO-(CH2)16-CO 2H
  MISC_FEATURE (20)..(20): Xaa at position 20 is Aib
  MOD_RES (34)..(34): Gly at position 34 is amidated

SEQ ID NO: 328 - protein, 34 aa, Artificial Sequence; identical to SEQ ID NO: 324
  Synthetic Construct
  MISC_FEATURE (2)..(2): Xaa at position 2 is Aib
  MISC_FEATURE (6)..(6): Xaa at position 6 is alpha-methyl-Phe(2F)
  MOD_RES (17)..(17): Lys at position 17 is chemically modified by conjugation of the epsilon-amino group of the Lys side chain with (2-[2-(2-amino-ethoxy)-ethoxy]-acetyl)2-(gamma-Glu)-CO-(CH2)16-CO 2H
  MISC_FEATURE (20)..(20): Xaa at position 20 is Aib
  MOD_RES (34)..(34): Gly at position 34 is amidated

SEQ ID NO: 329 - protein, 34 aa, Artificial Sequence; identical to SEQ ID NO: 325
  Synthetic Construct
  MISC_FEATURE (2)..(2): Xaa at position 2 is Aib
  MISC_FEATURE (6)..(6): Xaa at position 6 is alpha-methyl-Phe(2F)
  MOD_RES (17)..(17): Lys at position 17 is chemically modified by conjugation of the epsilon-amino group of the Lys side chain with (2-[2-(2-amino-ethoxy)-ethoxy]-acetyl)2-(gamma-Glu)-CO-(CH2)16-CO 2H
  MISC_FEATURE (20)..(20): Xaa at position 20 is Aib
  MOD_RES (34)..(34): Gly at position 34 is amidated

SEQ ID NO: 330 - protein, 39 aa, Artificial Sequence; identical to SEQ ID NO: 17
  Synthetic Construct
  MISC_FEATURE (2)..(2): Xaa at position 2 is Aib
  MOD_RES (17)..(17): Lys at position 17 is chemically modified by conjugation of the epsilon-amino group of the Lys side chain with (2-[2-(2-amino-ethoxy)-ethoxy]-acetyl)2-(gamma-Glu)-CO-(CH2)16-CO 2H
  MISC_FEATURE (20)..(20): Xaa at position 20 is Aib
  MOD_RES (39)..(39): Ser at position 39 is amidated

SEQ ID NO: 331 - protein, 39 aa, Artificial Sequence; identical to SEQ ID NO: 303
  Synthetic Construct
  MISC_FEATURE (2)..(2): Xaa at position 2 is Aib
  MOD_RES (17)..(17): Lys at position 17 is chemically modified by conjugation of the epsilon-amino group of the Lys side chain with (2-[2-(2-amino-ethoxy)-ethoxy]-acetyl)2-(gamma-Glu)-CO-(CH2)16-CO 2H
  MISC_FEATURE (20)..(20): Xaa at position 20 is Aib
  MOD_RES (39)..(39): Ser at position 39 is amidated

SEQ ID NO: 332 - protein, 34 aa, Artificial Sequence; identical to SEQ ID NO: 281
  Synthetic Construct
  MISC_FEATURE (2)..(2): Xaa at position 2 is Aib
  MOD_RES (17)..(17): Lys at position 17 is chemically modified by conjugation of the epsilon-amino group of the Lys side chain with (2-[2-(2-amino-ethoxy)-ethoxy]-acetyl)2-(gamma-Glu)-CO-(CH2)18-CO 2H
  MISC_FEATURE (20)..(20): Xaa at position 20 is Aib
  MOD_RES (34)..(34): Gly at position 34 is amidated

SEQ ID NO: 333 - protein, 34 aa, Artificial Sequence
  Synthetic Construct
  MISC_FEATURE (2)..(2): Xaa at position 2 is Aib
  MOD_RES (17)..(17): Lys at position 17 is chemically modified by conjugation of the epsilon-amino group of the Lys side chain with (2-[2-(2-amino-ethoxy)-ethoxy]-acetyl)2-(gamma-Glu)-CO-(CH2)18-CO 2H
  MISC_FEATURE (20)..(20): Xaa at position 20 is Aib
  MOD_RES (34)..(34): Gly at position 34 is amidated
YXEGTFTSDYSILLDKKAQXEFIEYLIAGGPSSG

SEQ ID NO: 334 - protein, 39 aa, Artificial Sequence
  Synthetic Construct
  MISC_FEATURE (2)..(2): Xaa at position 2 is Aib
  MOD_RES (17)..(17): Lys at position 17 is chemically modified by conjugation of the epsilon-amino group of the Lys side chain with (2-[2-(2-amino-ethoxy)-ethoxy]-acetyl)2-(gamma-Glu)-CO-(CH2)18-CO 2H
  MISC_FEATURE (20)..(20): Xaa at position 20 is Aib
  MOD_RES (39)..(39): Ser at position 39 is amidated
YXEGTFTSDYSILLDKKAQXEFIEYLIAGGPSSGAPPPS

SEQ ID NO: 335 - protein, 34 aa, Artificial Sequence
  Synthetic Construct
  MISC_FEATURE (2)..(2): Xaa at position 2 is Aib
  MOD_RES (17)..(17): Lys at position 17 is chemically modified by conjugation of the epsilon-amino group of the Lys side chain with (2-[2-(2-amino-ethoxy)-ethoxy]-acetyl)2-(gamma-Glu)-CO-(CH2)16-CO 2H
  MISC_FEATURE (20)..(20): Xaa at position 20 is Aib
  MOD_RES (34)..(34): Gly at position 34 is amidated
YXEGTFTSDYSILLDKKAQXDFIEYLIEGGPSSG

SEQ ID NO: 336 - protein, 34 aa, Artificial Sequence
  Synthetic Construct
  MISC_FEATURE (2)..(2): Xaa at position 2 is Aib
  MOD_RES (17)..(17): Lys at position 17 is chemically modified by conjugation of the epsilon-amino group of the Lys side chain with (2-[2-(2-amino-ethoxy)-ethoxy]-acetyl)2-(gamma-Glu)-CO-(CH2)16-CO 2H
  MISC_FEATURE (20)..(20): Xaa at position 20 is Aib
  MOD_RES (34)..(34): Gly at position 34 is amidated
YXEGTFTSDYSILLDKKAQXTFIEYLIEGGPSSG

SEQ ID NO: 337 - protein, 34 aa, Artificial Sequence
  Synthetic Construct
  MISC_FEATURE (2)..(2): Xaa at position 2 is Aib
  MOD_RES (17)..(17): Lys at position 17 is chemically modified by conjugation of the epsilon-amino group of the Lys side chain with (2-[2-(2-amino-ethoxy)-ethoxy]-acetyl)2-(gamma-Glu)-CO-(CH2)16-CO 2H
  MISC_FEATURE (20)..(20): Xaa at position 20 is Aib
  MOD_RES (34)..(34): Gly at position 34 is amidated
YXEGTFTSDYSILLDKKAQXHFIEYLIEGGPSSG

SEQ ID NO: 338 - protein, 39 aa, Artificial Sequence; identical to SEQ ID NO: 68
  Synthetic Construct
  MISC_FEATURE (2)..(2): Xaa at position 2 is Aib
  MISC_FEATURE (13)..(13): Xaa at position 13 is alpha-methyl-Leu
  MOD_RES (17)..(17): Lys at position 17 is chemically modified by conjugation of the epsilon-amino group of the Lys side chain with (2-[2-(2-amino-ethoxy)-ethoxy]-acetyl)2-(gamma-Glu)-CO-(CH2)16-CO 2H
  MISC_FEATURE (20)..(20): Xaa at position 20 is Aib
  MOD_RES (39)..(39): Ser at position 39 is amidated

SEQ ID NO: 339 - protein, 39 aa, Artificial Sequence
  Synthetic Construct
  MISC_FEATURE (2)..(2): Xaa at position 2 is Aib
  MISC_FEATURE (13)..(13): Xaa at position 13 is alpha-methyl-Leu
  MOD_RES (17)..(17): Lys at position 17 is chemically modified by conjugation of the epsilon-amino group of the Lys side chain with (2-[2-(2-amino-ethoxy)-ethoxy]-acetyl)2-(gamma-Glu)-CO-(CH2)18-CO 2H
  MISC_FEATURE (20)..(20): Xaa at position 20 is Aib
  MOD_RES (39)..(39): Ser at position 39 is amidated
YXEGTFTSDYSIXLDKKAQXAFIEYLIAGGPSSGAPPPS

SEQ ID NO: 340 - protein, 39 aa, Artificial Sequence; identical to SEQ ID NO: 66
  Synthetic Construct
  MISC_FEATURE (2)..(2): Xaa at position 2 is Aib
  MISC_FEATURE (6)..(6): Xaa at position 6 is alpha-methyl-Phe(2F)
  MOD_RES (17)..(17): Lys at position 17 is chemically modified by conjugation of the epsilon-amino group of the Lys side chain with (2-[2-(2-amino-ethoxy)-ethoxy]-acetyl)2-(gamma-Glu)-CO-(CH2)18-CO 2H
  MISC_FEATURE (20)..(20): Xaa at position 20 is Aib
  MOD_RES (39)..(39): Ser at position 39 is amidated

SEQ ID NO: 341 - protein, 39 aa, Artificial Sequence
  Synthetic Construct
  MISC_FEATURE (2)..(2): Xaa at position 2 is Aib
  MOD_RES (17)..(17): Lys at position 17 is chemically modified by conjugation of the epsilon-amino group of the Lys side chain with (2-[2-(2-amino-ethoxy)-ethoxy]-acetyl)2-(gamma-Glu)-CO-(CH2)18-CO 2H
  MISC_FEATURE (20)..(20): Xaa at position 20 is Aib
  MOD_RES (39)..(39): Ser at position 39 is amidated
FXEGTFTSDYSILLDKKAQXAFIEYLIEGGPSSGAPPPS

SEQ ID NO: 342 - protein, 39 aa, Artificial Sequence
  Synthetic Construct
  MISC_FEATURE (2)..(2): Xaa at position 2 is Aib
  MISC_FEATURE (13)..(13): Xaa at position 13 is alpha-methyl-Leu
  MOD_RES (17)..(17): Lys at position 17 is chemically modified by conjugation of the epsilon-amino group of the Lys side chain with (2-[2-(2-amino-ethoxy)-ethoxy]-acetyl)2-(gamma-Glu)-CO-(CH2)18-CO 2H
  MISC_FEATURE (20)..(20): Xaa at position 20 is Aib
  MOD_RES (39)..(39): Ser at position 39 is amidated
FXEGTFTSDYSIXLDKKAQXAFIEYLIEGGPSSGAPPPS

SEQ ID NO: 343 - protein, 39 aa, Artificial Sequence
  Synthetic Construct
  MISC_FEATURE (2)..(2): Xaa at position 2 is Aib
  MISC_FEATURE (13)..(13): Xaa at position 13 is alpha-methyl-Leu
  MOD_RES (17)..(17): Lys at position 17 is chemically modified by conjugation of the epsilon-amino group of the Lys side chain with (2-[2-(2-amino-ethoxy)-ethoxy]-acetyl)2-(gamma-Glu)-CO-(CH2)16-CO 2H
  MISC_FEATURE (20)..(20): Xaa at position 20 is Aib
  MOD_RES (39)..(39): Ser at position 39 is amidated
FXEGTFTSDYSIXLDKKAQXAFIEYLIEAGPSSGAPPPS

SEQ ID NO: 344 - protein, 39 aa, Artificial Sequence
  Synthetic Construct
  MISC_FEATURE (1)..(1): Xaa at position 1 is D-Tyr
  MISC_FEATURE (2)..(2): Xaa at position 2 is Aib
  MISC_FEATURE (6)..(6): Xaa at position 6 is alpha-methyl-Phe
  MOD_RES (17)..(17): Lys at position 17 is chemically modified by conjugation of the epsilon-amino group of the Lys side chain with (2-[2-(2-amino-ethoxy)-ethoxy]-acetyl)2-(gamma-Glu)-CO-(CH2)18-CO 2H
  MISC_FEATURE (20)..(20): Xaa at position 20 is Aib
  MOD_RES (39)..(39): Ser at position 39 is amidated
XXEGTXTSDYSILLDKKAQXAFIEYLIEGGPSSGAPPPS

SEQ ID NO: 345 - protein, 39 aa, Artificial Sequence
  Synthetic Construct
  MISC_FEATURE (2)..(2): Xaa at position 2 is Aib
  MOD_RES (17)..(17): Lys at position 17 is chemically modified by conjugation of the epsilon-amino group of the Lys side chain with (2-[2-(2-amino-ethoxy)-ethoxy]-acetyl)2-(gamma-Glu)-CO-(CH2)18-CO 2H
  MISC_FEATURE (20)..(20): Xaa at position 20 is Aib
  MOD_RES (39)..(39): Ser at position 39 is amidated
YXEGTFTSDYSILLDEKAQXAFIEYLIAGGPSSGAPPPS

SEQ ID NO: 346 - protein, 39 aa, Artificial Sequence
  Synthetic Construct
  MISC_FEATURE (2)..(2): Xaa at position 2 is Aib
  MISC_FEATURE (13)..(13): Xaa at position 13 is alpha-methyl-Leu
  MOD_RES (17)..(17): Lys at position 17 is chemically modified by conjugation of the epsilon-amino group of the Lys side chain with (2-[2-(2-amino-ethoxy)-ethoxy]-acetyl)2-(gamma-Glu)-CO-(CH2)18-CO 2H
  MISC_FEATURE (20)..(20): Xaa at position 20 is Aib
  MOD_RES (39)..(39): Ser at position 39 is amidated
YXEGTFTSDYSIXLDEKAQXEFIEYLIAGGPSSGAPPPS

SEQ ID NO: 347 - protein, 39 aa, Artificial Sequence
  Synthetic Construct
  MISC_FEATURE (2)..(2): Xaa at position 2 is Aib
  MISC_FEATURE (13)..(13): Xaa at position 13 is alpha-methyl-Leu
  MOD_RES (17)..(17): Lys at position 17 is chemically modified by conjugation of the epsilon-amino group of the Lys side chain with (2-[2-(2-amino-ethoxy)-ethoxy]-acetyl)2-(gamma-Glu)-CO-(CH2)18-CO 2H
  MISC_FEATURE (20)..(20): Xaa at position 2 is Aib
  MOD_RES (39)..(39): Ser at position 39 is amidated
YXEGTFTSDYSIXLDEKAQXAFIEYLIAGGPSSGAPPPS

SEQ ID NO: 348 - protein, 39 aa, Artificial Sequence
  Synthetic Construct
  MISC_FEATURE (2)..(2): Xaa at position 2 is Aib
  MISC_FEATURE (13)..(13): Xaa at position 13 is alpha-methyl-Leu
  MOD_RES (17)..(17): Lys at position 17 is chemically modified by conjugation of the epsilon-amino group of the Lys side chain with (2-[2-(2-amino-ethoxy)-ethoxy]-acetyl)2-(gamma-Glu)-CO-(CH2)18-CO 2H
  MISC_FEATURE (20)..(20): Xaa at position 20 is Aib
  MOD_RES (39)..(39): Ser at position 39 is amidated
YXEGTFTSDYSIXLDKKAQXEFIEYLIEGGPSSGAPPPS

SEQ ID NO: 349 - protein, 39 aa, Artificial Sequence
  Synthetic Construct
  MISC_FEATURE (1)..(1): Xaa at position 1 is D-Tyr
  MISC_FEATURE (2)..(2): Xaa at position 2 is Aib
  MISC_FEATURE (13)..(13): Xaa at position 13 is alpha-methyl-Leu
  MOD_RES (17)..(17): Lys at position 17 is chemically modified by conjugation of the epsilon-amino group of the Lys side chain with (2-[2-(2-amino-ethoxy)-ethoxy]-acetyl)2-(gamma-Glu)-CO-(CH2)18-CO 2H
  MISC_FEATURE (20)..(20): Xaa at position 20 is Aib
  MOD_RES (39)..(39): Ser at position 39 is amidated
XXEGTFTSDYSIXLDKKAQXAFIEYLIEGGPSSGAPPPS

SEQ ID NO: 350 - protein, 39 aa, Artificial Sequence
  Synthetic Construct
  MISC_FEATURE (1)..(1): Xaa at position 1 is D-Tyr
  MISC_FEATURE (2)..(2): Xaa at position 2 is Aib
  MISC_FEATURE (6)..(6): Xaa at position 6 is alpha-methyl-Phe
  MISC_FEATURE (13)..(13): Xaa at position 13 is alpha-methyl-Leu
  MOD_RES (17)..(17): Lys at position 17 is chemically modified by conjugation of the epsilon-amino group of the Lys side chain with (2-[2-(2-amino-ethoxy)-ethoxy]-acetyl)2-(gamma-Glu)-CO-(CH2)18-CO 2H
  MISC_FEATURE (20)..(20): Xaa at position 20 is Aib
  MOD_RES (39)..(39): Ser at position 39 is amidated
XXEGTXTSDYSIXLDKKAQXAFIEYLIEGGPSSGAPPPS

SEQ ID NO: 351 - protein, 39 aa, Artificial Sequence; identical to SEQ ID NO: 350
  Synthetic Construct
  MISC_FEATURE (1)..(1): Xaa at position 1 is D-Tyr
  MISC_FEATURE (2)..(2): Xaa at position 2 is Aib
  MISC_FEATURE (6)..(6): Xaa at position 6 is alpha-methyl-Phe(2F)
  MISC_FEATURE (13)..(13): Xaa at position 13 is alpha-methyl-Leu
  MOD_RES (17)..(17): Lys at position 17 is chemically modified by conjugation of the epsilon-amino group of the Lys side chain with (2-[2-(2-amino-ethoxy)-ethoxy]-acetyl)2-(gamma-Glu)-CO-(CH2)18-CO 2H
  MISC_FEATURE (20)..(20): Xaa at position 20 is Aib
  MOD_RES (39)..(39): Ser at position 39 is amidated

SEQ ID NO: 352 - protein, 39 aa, Artificial Sequence
  Synthetic Construct
  MISC_FEATURE (2)..(2): Xaa at position 2 is Aib
  MISC_FEATURE (13)..(13): Xaa at position 13 is alpha-methyl-Leu
  MOD_RES (17)..(17): Lys at position 17 is chemically modified by conjugation of the epsilon-amino group of the Lys side chain with (2-[2-(2-amino-ethoxy)-ethoxy]-acetyl)2-(gamma-Glu)-CO-(CH2)18-CO 2H
  MISC_FEATURE (20)..(20): Xaa at position 20 is Aib
  MOD_RES (39)..(39): Ser at position 39 is amidated
FXEGTFTSDYSIXLDKKAQXAFIEYLIAGGPSSGAPPPS

SEQ ID NO: 353 - protein, 39 aa, Artificial Sequence
  Synthetic Construct
  MISC_FEATURE (2)..(2): Xaa at position 2 is Aib
  MISC_FEATURE (13)..(13): Xaa at position 13 is alpha-methyl-Leu
  MOD_RES (17)..(17): Lys at position 17 is chemically modified by conjugation of the epsilon-amino group of the Lys side chain with (2-[2-(2-amino-ethoxy)-ethoxy]-acetyl)2-(gamma-Glu)-CO-(CH2)18-CO 2H
  MISC_FEATURE (20)..(20): Xaa at position 20 is Aib
  MOD_RES (39)..(39): Ser at position 39 is amidated
FXEGTFTSDYSIXLDKKAQXEFIEYLIAGGPSSGAPPPS

SEQ ID NO: 354 - protein, 39 aa, Artificial Sequence; identical to SEQ ID NO: 304
  Synthetic Construct
  MISC_FEATURE (2)..(2): Xaa at position 2 is Aib
  MISC_FEATURE (13)..(13): Xaa at position 13 is alpha-methyl-Leu
  MOD_RES (17)..(17): Lys at position 17 is chemically modified by conjugation of the epsilon-amino group of the Lys side chain with (2-[2-(2-amino-ethoxy)-ethoxy]-acetyl)-(gamma-Glu)-CO-(CH2)18-CO2 H
  MISC_FEATURE (20)..(20): Xaa at position 20 is Aib
  MOD_RES (39)..(39): Ser at position 39 is amidated

SEQ ID NO: 355 - protein, 39 aa, Artificial Sequence
  Synthetic Construct
  MISC_FEATURE (1)..(1): Xaa at position 1 is D-Tyr
  MISC_FEATURE (2)..(2): Xaa at position 2 is Aib
  MISC_FEATURE (13)..(13): Xaa at position 13 is alpha-methyl-Leu
  MOD_RES (17)..(17): Lys at position 17 is chemically modified by conjugation of the epsilon-amino group of the Lys side chain with (2-[2-(2-amino-ethoxy)-ethoxy]-acetyl)2-(gamma-Glu)-CO-(CH2)18-CO 2H
  MISC_FEATURE (20)..(20): Xaa at position 20 is Aib
  MOD_RES (39)..(39): Ser at position 39 is amidated
XXEGTFTSDYSIXLDKKAQXAFIEYLIAGGPSSGAPPPS

SEQ ID NO: 356 - protein, 39 aa, Artificial Sequence
  Synthetic Construct
  MISC_FEATURE (1)..(1): Xaa at position 1 is D-Tyr
  MISC_FEATURE (2)..(2): Xaa at position 2 is Aib
  MISC_FEATURE (13)..(13): Xaa at position 13 is alpha-methyl-Leu
  MOD_RES (17)..(17): Lys at position 17 is chemically modified by conjugation of the epsilon-amino group of the Lys side chain with (2-[2-(2-amino-ethoxy)-ethoxy]-acetyl)2-(gamma-Glu)-CO-(CH2)18-CO 2H
  MISC_FEATURE (20)..(20): Xaa at position 20 is Aib
  MOD_RES (39)..(39): Ser at position 39 is amidated
XXEGTFTSDYSIXLDEKAQXAFIEYLIAGGPSSGAPPPS

SEQ ID NO: 357 - protein, 39 aa, Artificial Sequence
  Synthetic Construct
  MISC_FEATURE (1)..(1): Xaa at position 1 is D-Tyr
  MISC_FEATURE (2)..(2): Xaa at position 2 is Aib
  MISC_FEATURE (13)..(13): Xaa at position 13 is alpha-methyl-Leu
  MOD_RES (17)..(17): Lys at position 17 is chemically modified by conjugation of the epsilon-amino group of the Lys side chain with (2-[2-(2-amino-ethoxy)-ethoxy]-acetyl)2-(gamma-Glu)-CO-(CH2)18-CO 2H
  MISC_FEATURE (20)..(20): Xaa at position 20 is Aib
  MOD_RES (39)..(39): Ser at position 39 is amidated
XXEGTFTSDYSIXLDEKAQXEFIEYLIAGGPSSGAPPPS

SEQ ID NO: 358 - protein, 39 aa, Artificial Sequence
  Synthetic Construct
  MISC_FEATURE (2)..(2): Xaa at position 2 is Aib
  MISC_FEATURE (13)..(13): Xaa at position 13 is alpha-methyl-Leu
  MOD_RES (17)..(17): Lys at position 17 is chemically modified by conjugation of the epsilon-amino group of the Lys side chain with (2-[2-(2-amino-ethoxy)-ethoxy]-acetyl)2-(gamma-Glu)-CO-(CH2)18-CO 2H
  MISC_FEATURE (20)..(20): Xaa at position 20 is Aib
  MISC_FEATURE (24)..(24): Xaa at position 24 is D-Glu
  MOD_RES (39)..(39): Ser at position 39 is amidated
YXEGTFTSDYSIXLDEKAQXAFIXYLIAGGPSSGAPPPS

SEQ ID NO: 359 - protein, 39 aa, Artificial Sequence
  Synthetic Construct
  MISC_FEATURE (2)..(2): Xaa at position 2 is Aib
  MISC_FEATURE (13)..(13): Xaa at position 13 is alpha-methyl-Leu
  MOD_RES (17)..(17): Lys at position 17 is chemically modified by conjugation of the epsilon-amino group of the Lys side chain with (2-[2-(2-amino-ethoxy)-ethoxy]-acetyl)2-(gamma-Glu)-CO-(CH2)18-CO 2H
  MISC_FEATURE (20)..(20): Xaa at position 20 is Aib
  MOD_RES (39)..(39): Ser at position 39 is amidated
YXEGTFTSDYSIXLDEKAQXDFIEYLIAGGPSSGAPPPS

SEQ ID NO: 360 - protein, 39 aa, Artificial Sequence
  Synthetic Construct
  MISC_FEATURE (1)..(1): Xaa at position 1 is D-Tyr
  MISC_FEATURE (2)..(2): Xaa at position 2 is Aib
  MISC_FEATURE (6)..(6): Xaa at position 6 is alpha-methyl-Phe
  MISC_FEATURE (13)..(13): Xaa at position 13 is alpha-methyl-Leu
  MOD_RES (17)..(17): Lys at position 17 is chemically modified by conjugation of the epsilon-amino group of the Lys side chain with (2-[2-(2-amino-ethoxy)-ethoxy]-acetyl)2-(gamma-Glu)-CO-(CH2)18-CO 2H
  MISC_FEATURE (20)..(20): Xaa at position 20 is Aib
  MOD_RES (39)..(39): Ser at position 39 is amidated
XXEGTXTSDYSIXLDKKAQXEFIEYLIAGGPSSGAPPPS

SEQ ID NO: 361 - protein, 39 aa, Artificial Sequence
  Synthetic Construct
  MISC_FEATURE (1)..(1): Xaa at position 1 is D-Tyr
  MISC_FEATURE (2)..(2): Xaa at position 2 is Aib
  MISC_FEATURE (13)..(13): Xaa at position 13 is alpha-methyl-Leu
  MISC_FEATURE (16)..(16): Xaa at position 16 is Orn
  MOD_RES (17)..(17): Lys at position 17 is chemically modified by conjugation of the epsilon-amino group of the Lys side chain with (2-[2-(2-amino-ethoxy)-ethoxy]-acetyl)2-(gamma-Glu)-CO-(CH2)18-CO 2H
  MISC_FEATURE (20)..(20): Xaa at position 20 is Aib
  MOD_RES (39)..(39): Ser at position 39 is amidated
XXEGTFTSDYSIXLDXKAQXAFIEYLIAGGPSSGAPPPS

SEQ ID NO: 362 - protein, 39 aa, Artificial Sequence; identical to SEQ ID NO: 361
  Synthetic Construct
  MISC_FEATURE (1)..(1): Xaa at position 1 is D-Tyr
  MISC_FEATURE (2)..(2): Xaa at position 2 is Aib
  MISC_FEATURE (13)..(13): Xaa at position 13 is alpha-methyl-Leu
  MISC_FEATURE (16)..(16): Xaa at position 16 is Dab
  MOD_RES (17)..(17): Lys at position 17 is chemically modified by conjugation of the epsilon-amino group of the Lys side chain with (2-[2-(2-amino-ethoxy)-ethoxy]-acetyl)2-(gamma-Glu)-CO-(CH2)18-CO 2H
  MISC_FEATURE (20)..(20): Xaa at position 20 is Aib
  MOD_RES (39)..(39): Ser at position 39 is amidated

SEQ ID NO: 363 - protein, 39 aa, Artificial Sequence; identical to SEQ ID NO: 361
  Synthetic Construct
  MISC_FEATURE (1)..(1): Xaa at position 1 is D-Tyr
  MISC_FEATURE (2)..(2): Xaa at position 2 is Aib
  MISC_FEATURE (13)..(13): Xaa at position 13 is alpha-methyl-Leu
  MISC_FEATURE (16)..(16): Xaa at position 16 is Dap
  MOD_RES (17)..(17): Lys at position 17 is chemically modified by conjugation of the epsilon-amino group of the Lys side chain with (2-[2-(2-amino-ethoxy)-ethoxy]-acetyl)2-(gamma-Glu)-CO-(CH2)18-CO 2H
  MISC_FEATURE (20)..(20): Xaa at position 20 is Aib
  MOD_RES (39)..(39): Ser at position 39 is amidated

SEQ ID NO: 364 - protein, 39 aa, Artificial Sequence
  Synthetic Construct
  MISC_FEATURE (1)..(1): Xaa at position 1 is D-Tyr
  MISC_FEATURE (2)..(2): Xaa at position 2 is Aib
  MISC_FEATURE (13)..(13): Xaa at position 13 is alpha-methyl-Leu
  MISC_FEATURE (16)..(16): Xaa at position 16 is Orn
  MOD_RES (17)..(17): Lys at position 17 is chemically modified by conjugation of the epsilon-amino group of the Lys side chain with (2-[2-(2-amino-ethoxy)-ethoxy]-acetyl)2-(gamma-Glu)-CO-(CH2)18-CO 2H
  MISC_FEATURE (20)..(20): Xaa at position 20 is Aib
  MOD_RES (39)..(39): Ser at position 39 is amidated
XXEGTFTSDYSIXLDXKAQXEFIEYLIAGGPSSGAPPPS

SEQ ID NO: 365 - protein, 39 aa, Artificial Sequence; identical to SEQ ID NO: 364
  Synthetic Construct
  MISC_FEATURE (1)..(1): Xaa at position 1 is D-Tyr
  MISC_FEATURE (2)..(2): Xaa at position 2 is Aib
  MISC_FEATURE (13)..(13): Xaa at position 13 is alpha-methyl-Leu
  MISC_FEATURE (16)..(16): Xaa at position 16 is Dab
  MOD_RES (17)..(17): Lys at position 17 is chemically modified by conjugation of the epsilon-amino group of the Lys side chain with (2-[2-(2-amino-ethoxy)-ethoxy]-acetyl)2-(gamma-Glu)-CO-(CH2)18-CO 2H
  MISC_FEATURE (20)..(20): Xaa at position 20 is Aib
  MOD_RES (39)..(39): Ser at position 39 is amidated

SEQ ID NO: 366 - protein, 39 aa, Artificial Sequence; identical to SEQ ID NO: 364
  Synthetic Construct
  MISC_FEATURE (1)..(1): Xaa at position 1 is D-Tyr
  MISC_FEATURE (2)..(2): Xaa at position 2 is Aib
  MISC_FEATURE (13)..(13): Xaa at position 13 is alpha-methyl-Leu
  MISC_FEATURE (16)..(16): Xaa at position 16 is Dap
  MOD_RES (17)..(17): Lys at position 17 is chemically modified by conjugation of the epsilon-amino group of the Lys side chain with (2-[2-(2-amino-ethoxy)-ethoxy]-acetyl)2-(gamma-Glu)-CO-(CH2)18-CO 2H
  MISC_FEATURE (20)..(20): Xaa at position 20 is Aib
  MOD_RES (39)..(39): Ser at position 39 is amidated

SEQ ID NO: 367 - protein, 39 aa, Artificial Sequence
  Synthetic Construct
  MISC_FEATURE (1)..(1): Xaa at position 1 is D-Tyr
  MISC_FEATURE (2)..(2): Xaa at position 2 is Aib
  MISC_FEATURE (13)..(13): Xaa at position 13 is alpha-methyl-Leu
  MOD_RES (17)..(17): Lys at position 17 is chemically modified by conjugation of the epsilon-amino group of the Lys side chain with (2-[2-(2-amino-ethoxy)-ethoxy]-acetyl)2-(gamma-Glu)-CO-(CH2)18-CO 2H
  MISC_FEATURE (20)..(20): Xaa at position 20 is Aib
  MISC_FEATURE (24)..(24): Xaa at position 24 is D-Glu
  MOD_RES (39)..(39): Ser at position 39 is amidated
XXEGTFTSDYSIXLDKKAQXAFIXYLIAGGPSSGAPPPS

SEQ ID NO: 368 - protein, 39 aa, Artificial Sequence
  Synthetic Construct
  MISC_FEATURE (1)..(1): Xaa at position 1 is D-Tyr
  MISC_FEATURE (2)..(2): Xaa at position 2 is Aib
  MISC_FEATURE (13)..(13): Xaa at position 13 is alpha-methyl-Leu
  MOD_RES (17)..(17): Lys at position 17 is chemically modified by conjugation of the epsilon-amino group of the Lys side chain with (2-[2-(2-amino-ethoxy)-ethoxy]-acetyl)2-(gamma-Glu)-CO-(CH2)18-CO 2H
  MISC_FEATURE (20)..(20): Xaa at position 20 is Aib
  MISC_FEATURE (24)..(24): Xaa at position 24 is D-Glu
  MOD_RES (39)..(39): Ser at position 39 is amidated
XXEGTFTSDYSIXLDKKAQXEFIXYLIEGGPSSGAPPPS

SEQ ID NO: 369 - protein, 39 aa, Artificial Sequence
  Synthetic Construct
  MISC_FEATURE (1)..(1): Xaa at position 1 is D-Tyr
  MISC_FEATURE (2)..(2): Xaa at position 2 is Aib
  MISC_FEATURE (13)..(13): Xaa at position 13 is alpha-methyl-Leu
  MISC_FEATURE (16)..(16): Xaa at position 16 is Orn
  MOD_RES (17)..(17): Lys at position 17 is chemically modified by conjugation of the epsilon-amino group of the Lys side chain with (2-[2-(2-amino-ethoxy)-ethoxy]-acetyl)2-(gamma-Glu)-CO-(CH2)18-CO 2H
  MISC_FEATURE (20)..(20): Xaa at position 20 is Aib
  MISC_FEATURE (24)..(24): Xaa at position 24 is D-Glu
  MOD_RES (39)..(39): Ser at position 39 is amidated
XXEGTFTSDYSIXLDXKAQXEFIXYLIAGGPSSGAPPPS

SEQ ID NO: 370 - protein, 39 aa, Artificial Sequence
  Synthetic Construct
  MISC_FEATURE (1)..(1): Xaa at position 1 is D-Tyr
  MISC_FEATURE (2)..(2): Xaa at position 2 is Aib
  MISC_FEATURE (13)..(13): Xaa at position 13 is alpha-methyl-Leu
  MISC_FEATURE (16)..(16): Xaa at position 16 is Orn
  MOD_RES (17)..(17): Lys at position 17 is chemically modified by conjugation of the epsilon-amino group of the Lys side chain with (2-[2-(2-amino-ethoxy)-ethoxy]-acetyl)2-(gamma-Glu)-CO-(CH2)18-CO 2H
  MISC_FEATURE (20)..(20): Xaa at position 20 is Aib
  MISC_FEATURE (24)..(24): Xaa at position 24 is D-Glu
  MOD_RES (39)..(39): Ser at position 39 is amidated
XXEGTFTSDYSIXLDXKAQXEFIXYLIEGGPSSGAPPPS

SEQ ID NO: 371 - protein, 39 aa, Artificial Sequence
  Synthetic Construct
  MISC_FEATURE (1)..(1): Xaa at position 1 is D-Tyr
  MISC_FEATURE (2)..(2): Xaa at position 2 is Aib
  MISC_FEATURE (13)..(13): Xaa at position 13 is alpha-methyl-Leu
  MOD_RES (17)..(17): Lys at position 17 is chemically modified by conjugation of the epsilon-amino group of the Lys side chain with (2-[2-(2-amino-ethoxy)-ethoxy]-acetyl)2-(gamma-Glu)-CO-(CH2)18-CO 2H
  MISC_FEATURE (20)..(20): Xaa at position 20 is Aib
  MISC_FEATURE (24)..(24): Xaa at position 24 is D-Glu
  MOD_RES (39)..(39): Ser at position 39 is amidated
XXEGTFTSDYSIXLDKKAQXAFIXYLIEGGPSSGAPPPS

SEQ ID NO: 372 - protein, 39 aa, Artificial Sequence
  Synthetic Construct
  MISC_FEATURE (1)..(1): Xaa at position 1 is D-Tyr
  MISC_FEATURE (2)..(2): Xaa at position 2 is Aib
  MISC_FEATURE (13)..(13): Xaa at position 13 is alpha-methyl-Leu
  MISC_FEATURE (16)..(16): Xaa at position 16 is Orn
  MOD_RES (17)..(17): Lys at position 17 is chemically modified by conjugation of the epsilon-amino group of the Lys side chain with (2-[2-(2-amino-ethoxy)-ethoxy]-acetyl)2-(gamma-Glu)-CO-(CH2)18-CO 2H
  MISC_FEATURE (20)..(20): Xaa at position 20 is Aib
  MISC_FEATURE (24)..(24): Xaa at position 24 is D-Glu
  MOD_RES (39)..(39): Ser at position 39 is amidated
XXEGTFTSDYSIXLDXKAQXAFIXYLIEGGPSSGAPPPS

SEQ ID NO: 373 - protein, 39 aa, Artificial Sequence
  Synthetic Construct
  MISC_FEATURE (1)..(1): Xaa at position 1 is D-Tyr
  MISC_FEATURE (2)..(2): Xaa at position 2 is Aib
  MISC_FEATURE (13)..(13): Xaa at position 13 is alpha-methyl-Leu
  MISC_FEATURE (16)..(16): Xaa at position 16 is Orn
  MOD_RES (17)..(17): Lys at position 17 is chemically modified by conjugation of the epsilon-amino group of the Lys side chain with (2-[2-(2-amino-ethoxy)-ethoxy]-acetyl)2-(gamma-Glu)-CO-(CH2)18-CO 2H
  MISC_FEATURE (20)..(20): Xaa at position 20 is Aib
  MOD_RES (39)..(39): Ser at position 39 is amidated
XXEGTFTSDYSIXLDXKAQXAFVEYLIAGGPSSGAPPPS

SEQ ID NO: 374 - protein, 39 aa, Artificial Sequence
  Synthetic Construct
  MISC_FEATURE (1)..(1): Xaa at position 1 is D-Tyr
  MISC_FEATURE (2)..(2): Xaa at position 2 is Aib
  MISC_FEATURE (13)..(13): Xaa at position 13 is alpha-methyl-Leu
  MISC_FEATURE (16)..(16): Xaa at position 16 is Orn
  MOD_RES (17)..(17): Lys at position 17 is chemically modified by conjugation of the epsilon-amino group of the Lys side chain with (2-[2-(2-amino-ethoxy)-ethoxy]-acetyl)2-(gamma-Glu)-CO-(CH2)18-CO 2H
  MISC_FEATURE (20)..(20): Xaa at position 20 is Aib
  MOD_RES (39)..(39): Ser at position 39 is amidated
XXEGTFTSDYSIXLDXKAQXEFVEYLIAGGPSSGAPPPS

SEQ ID NO: 375 - protein, 39 aa, Artificial Sequence
  Synthetic Construct
  MISC_FEATURE (1)..(1): Xaa at position 1 is D-Tyr
  MISC_FEATURE (2)..(2): Xaa at position 2 is Aib
  MISC_FEATURE (13)..(13): Xaa at position 13 is alpha-methyl-Leu
  MISC_FEATURE (16)..(16): Xaa at position 16 is Orn
  MOD_RES (17)..(17): Lys at position 17 is chemically modified by conjugation of the epsilon-amino group of the Lys side chain with (2-[2-(2-amino-ethoxy)-ethoxy]-acetyl)2-(gamma-Glu)-CO-(CH2)18-CO 2H
  MISC_FEATURE (20)..(20): Xaa at position 20 is Aib
  MOD_RES (39)..(39): Ser at position 39 is amidated
XXEGTFTSDYSIXLDXKAQXAFVEYLIEGGPSSGAPPPS

SEQ ID NO: 376 - protein, 39 aa, Artificial Sequence
  Synthetic Construct
  MISC_FEATURE (1)..(1): Xaa at position 1 is D-Tyr
  MISC_FEATURE (2)..(2): Xaa at position 2 is Aib
  MISC_FEATURE (13)..(13): Xaa at position 13 is alpha-methyl-Leu
  MOD_RES (17)..(17): Lys at position 17 is chemically modified by conjugation of the epsilon-amino group of the Lys side chain with (2-[2-(2-amino-ethoxy)-ethoxy]-acetyl)2-(gamma-Glu)-CO-(CH2)18-CO 2H
  MISC_FEATURE (20)..(20): Xaa at position 20 is Aib
  MISC_FEATURE (24)..(24): Xaa at position 24 is D-Glu
  MOD_RES (39)..(39): Ser at position 39 is amidated
XXEGTFTSDYSIXLDKKAQXAFVXYLIAGGPSSGAPPPS

SEQ ID NO: 377 - protein, 39 aa, Artificial Sequence
  Synthetic Construct
  MISC_FEATURE (1)..(1): Xaa at position 1 is D-Tyr
  MISC_FEATURE (2)..(2): Xaa at position 2 is Aib
  MISC_FEATURE (13)..(13): Xaa at position 13 is alpha-methyl-Leu
  MISC_FEATURE (16)..(16): Xaa at position 16 is Orn
  MOD_RES (17)..(17): Lys at position 17 is chemically modified by conjugation of the epsilon-amino group of the Lys side chain with (2-[2-(2-amino-ethoxy)-ethoxy]-acetyl)2-(gamma-Glu)-CO-(CH2)18-CO 2H
  MISC_FEATURE (20)..(20): Xaa at position 20 is Aib
  MISC_FEATURE (24)..(24): Xaa at position 24 is D-Glu
  MOD_RES (39)..(39): Ser at position 39 is amidated
XXEGTFTSDYSIXLDXKAQXAFVXYLIAGGPSSGAPPPS

SEQ ID NO: 378 - protein, 39 aa, Artificial Sequence; identical to SEQ ID NO: 306
  Synthetic Construct
  MISC_FEATURE (1)..(1): Xaa at position 1 is D-Tyr
  MISC_FEATURE (2)..(2): Xaa at position 2 is Aib
  MISC_FEATURE (13)..(13): Xaa at position 13 is alpha-methyl-Leu
  MISC_FEATURE (16)..(16): Xaa at position 16 is Orn
  MOD_RES (17)..(17): Lys at position 17 is chemically modified by conjugation of the epsilon-amino group of the Lys side chain with (2-[2-(2-amino-ethoxy)-ethoxy]-acetyl)2-(gamma-Glu)-CO-(CH2)16-CO 2H
  MISC_FEATURE (20)..(20): Xaa at position 20 is Aib
  MISC_FEATURE (24)..(24): Xaa at position 24 is D-Glu
  MOD_RES (39)..(39): Ser at position 39 is amidated

SEQ ID NO: 379 - protein, 39 aa, Artificial Sequence; identical to SEQ ID NO: 377
  Synthetic Construct
  MISC_FEATURE (1)..(1): Xaa at position 1 is D-Tyr
  MISC_FEATURE (2)..(2): Xaa at position 2 is Aib
  MISC_FEATURE (13)..(13): Xaa at position 13 is alpha-methyl-Leu
  MISC_FEATURE (16)..(16): Xaa at position 16 is Orn
  MOD_RES (17)..(17): Lys at position 17 is chemically modified by conjugation of the epsilon-amino group of the Lys side chain with (2-[2-(2-amino-ethoxy)-ethoxy]-acetyl)2-(gamma-Glu)-CO-(CH2)16-CO 2H
  MISC_FEATURE (20)..(20): Xaa at position 20 is Aib
  MISC_FEATURE (24)..(24): Xaa at position 24 is D-Glu
  MOD_RES (39)..(39): Ser at position 39 is amidated

SEQ ID NO: 380 - protein, 39 aa, Artificial Sequence
  Synthetic Construct
  MISC_FEATURE (1)..(1): Xaa at position 1 is D-Tyr
  MISC_FEATURE (2)..(2): Xaa at position 2 is Aib
  MISC_FEATURE (13)..(13): Xaa at position 13 is alpha-methyl-Leu
  MOD_RES (17)..(17): Lys at position 17 is chemically modified by conjugation of the epsilon-amino group of the Lys side chain with (2-[2-(2-amino-ethoxy)-ethoxy]-acetyl)2-(gamma-Glu)-CO-(CH2)18-CO 2H
  MISC_FEATURE (20)..(20): Xaa at position 20 is Aib
  MISC_FEATURE (25)..(25): Xaa at position 25 is alpha-methyl-Tyr
  MOD_RES (39)..(39): Ser at position 39 is amidated
XXEGTFTSDYSIXLDKKAQXAFIEXLIAGGPSSGAPPPS

SEQ ID NO: 381 - protein, 39 aa, Artificial Sequence
  Synthetic Construct
  MISC_FEATURE (1)..(1): Xaa at position 1 is D-Tyr
  MISC_FEATURE (2)..(2): Xaa at position 2 is Aib
  MISC_FEATURE (13)..(13): Xaa at position 13 is alpha-methyl-Leu
  MISC_FEATURE (16)..(16): Xaa at position 16 is Orn
  MOD_RES (17)..(17): Lys at position 17 is chemically modified by conjugation of the epsilon-amino group of the Lys side chain with (2-[2-(2-amino-ethoxy)-ethoxy]-acetyl)2-(gamma-Glu)-CO-(CH2)18-CO 2H
  MISC_FEATURE (20)..(20): Xaa at position 20 is Aib
  MISC_FEATURE (25)..(25): Xaa at position 25 is alpha-methyl-Tyr
  MOD_RES (39)..(39): Ser at position 39 is amidated
XXEGTFTSDYSIXLDXKAQXAFIEXLIAGGPSSGAPPPS

SEQ ID NO: 382 - protein, 39 aa, Artificial Sequence
  Synthetic Construct
  MISC_FEATURE (2)..(2): Xaa at position 2 is Aib
  MISC_FEATURE (13)..(13): Xaa at position 13 is alpha-methyl-Leu
  MOD_RES (17)..(17): Lys at position 17 is chemically modified by conjugation of the epsilon-amino group of the Lys side chain with (2-[2-(2-amino-ethoxy)-ethoxy]-acetyl)2-(gamma-Glu)-CO-(CH2)18-CO 2H
  MISC_FEATURE (20)..(20): Xaa at position 20 is Aib
  MISC_FEATURE (25)..(25): Xaa at position 25 is alpha-methyl-Tyr
  MOD_RES (39)..(39): Ser at position 39 is amidated
YXEGTFTSDYSIXLDKKAQXEFIEXLIAGGPSSGAPPPS

SEQ ID NO: 383 - protein, 39 aa, Artificial Sequence; identical to SEQ ID NO: 364
  Synthetic Construct
  MISC_FEATURE (1)..(1): Xaa at position 1 is D-Tyr
  MISC_FEATURE (2)..(2): Xaa at position 2 is Aib
  MISC_FEATURE (13)..(13): Xaa at position 13 is alpha-methyl-Leu
  MISC_FEATURE (16)..(16): Xaa at position 16 is Orn
  MOD_RES (17)..(17): Lys at position 17 is chemically modified by conjugation of the epsilon-amino group of the Lys side chain with (2-[2-(2-amino-ethoxy)-ethoxy]-acetyl)2-(gamma-Glu)-CO-(CH2)16-CO 2H
  MISC_FEATURE (20)..(20): Xaa at position 20 is Aib
  MOD_RES (39)..(39): Ser at position 39 is amidated

SEQ ID NO: 384 - protein, 39 aa, Artificial Sequence
  Synthetic Construct
  MISC_FEATURE (1)..(1): Xaa at position 1 is D-Tyr
  MISC_FEATURE (2)..(2): Xaa at position 2 is Aib
  MISC_FEATURE (13)..(13): Xaa at position 13 is alpha-methyl-Leu
  MISC_FEATURE (16)..(16): Xaa at position 16 is Orn
  MOD_RES (17)..(17): Lys at position 17 is chemically modified by conjugation of the epsilon-amino group of the Lys side chain with (2-[2-(2-amino-ethoxy)-ethoxy]-acetyl)2-(gamma-Glu)-CO-(CH2)18-CO 2H
  MISC_FEATURE (20)..(20): Xaa at position 20 is Aib
  MOD_RES (39)..(39): Ser at position 39 is amidated
XXEGTFTSDYSIXLDXKAQXDFIEYLIAGGPSSGAPPPS

SEQ ID NO: 385 - protein, 34 aa, Artificial Sequence
  Synthetic Construct
  MISC_FEATURE (1)..(1): Xaa at position 1 is D-Tyr
  MISC_FEATURE (2)..(2): Xaa at position 2 is Aib
  MISC_FEATURE (13)..(13): Xaa at position 13 is alpha-methyl-Leu
  MISC_FEATURE (16)..(16): Xaa at position 16 is Orn
  MOD_RES (17)..(17): Lys at position 17 is chemically modified by conjugation of the epsilon-amino group of the Lys side chain with (2-[2-(2-amino-ethoxy)-ethoxy]-acetyl)2-(gamma-Glu)-CO-(CH2)18-CO 2H
  MISC_FEATURE (20)..(20): Xaa at position 20 is Aib
  MOD_RES (34)..(34): Gly at position 34 is amidated
XXEGTFTSDYSIXLDXKAQXEFIEYLIAGGPSSG

SEQ ID NO: 386 - protein, 39 aa, Artificial Sequence; identical to SEQ ID NO: 364
  Synthetic Construct
  MISC_FEATURE (1)..(1): Xaa at position 1 is D-Tyr
  MISC_FEATURE (2)..(2): Xaa at position 2 is Aib
  MISC_FEATURE (13)..(13): Xaa at position 13 is alpha-methyl-Leu
  MISC_FEATURE (16)..(16): Xaa at position 16 is Orn
  MOD_RES (17)..(17): Lys at position 17 is chemically modified by conjugation of the epsilon-amino group of the Lys side chain with (2-[2-(2-amino-ethoxy)-ethoxy]-acetyl)-(gamma-Glu)-CO-(CH2)18-CO2 H
  MISC_FEATURE (20)..(20): Xaa at position 20 is Aib
  MOD_RES (39)..(39): Ser at position 39 is amidated

SEQ ID NO: 387 - protein, 39 aa, Artificial Sequence; identical to SEQ ID NO: 307
  Synthetic Construct
  MISC_FEATURE (1)..(1): Xaa at position 1 is D-Tyr
  MISC_FEATURE (2)..(2): Xaa at position 2 is Aib
  MISC_FEATURE (13)..(13): Xaa at position 13 is alpha-methyl-Leu
  MOD_RES (17)..(17): Lys at position 17 is chemically modified by conjugation of the epsilon-amino group of the Lys side chain with (2-[2-(2-amino-ethoxy)-ethoxy]-acetyl)-(gamma-Glu)-CO-(CH2)18-CO2 H
  MISC_FEATURE (20)..(20): Xaa at position 20 is Aib
  MISC_FEATURE (25)..(25): Xaa at position 25 is alpha-methyl-Tyr
  MOD_RES (39)..(39): Ser at position 39 is amidated

SEQ ID NO: 388 - protein, 39 aa, Artificial Sequence; identical to SEQ ID NO: 380
  Synthetic Construct
  MISC_FEATURE (1)..(1): Xaa at position 1 is D-Tyr
  MISC_FEATURE (2)..(2): Xaa at position 2 is Aib
  MISC_FEATURE (13)..(13): Xaa at position 13 is alpha-methyl-Leu
  MOD_RES (17)..(17): Lys at position 17 is chemically modified by conjugation of the epsilon-amino group of the Lys side chain with (2-[2-(2-amino-ethoxy)-ethoxy]-acetyl)-(gamma-Glu)-CO-(CH2)18-CO2 H
  MISC_FEATURE (20)..(20): Xaa at position 20 is Aib
  MISC_FEATURE (25)..(25): Xaa at position 25 is alpha-methyl-Tyr
  MOD_RES (39)..(39): Ser at position 39 is amidated

SEQ ID NO: 389 - protein, 39 aa, Artificial Sequence; identical to SEQ ID NO: 307
  Synthetic Construct
  MISC_FEATURE (1)..(1): Xaa at position 1 is D-Tyr
  MISC_FEATURE (2)..(2): Xaa at position 2 is Aib
  MISC_FEATURE (13)..(13): Xaa at position 13 is alpha-methyl-Leu
  MOD_RES (17)..(17): Lys at position 17 is chemically modified by conjugation of the epsilon-amino group of the Lys side chain with (2-[2-(2-amino-ethoxy)-ethoxy]-acetyl)2-(gamma-Glu)-CO-(CH2)16-CO 2H
  MISC_FEATURE (20)..(20): Xaa at position 20 is Aib
  MISC_FEATURE (25)..(25): Xaa at position 25 is alpha-methyl-Tyr
  MOD_RES (39)..(39): Ser at position 39 is amidated

SEQ ID NO: 390 - protein, 39 aa, Artificial Sequence; identical to SEQ ID NO: 308
  Synthetic Construct
  MISC_FEATURE (1)..(1): Xaa at position 1 is D-Tyr
  MISC_FEATURE (2)..(2): Xaa at position 2 is Aib
  MISC_FEATURE (13)..(13): Xaa at position 13 is alpha-methyl-Leu
  MISC_FEATURE (16)..(16): Xaa at position 16 is Orn
  MOD_RES (17)..(17): Lys at position 17 is chemically modified by conjugation of the epsilon-amino group of the Lys side chain with (2-[2-(2-amino-ethoxy)-ethoxy]-acetyl)2-(gamma-Glu)-CO-(CH2)16-CO 2H
  MISC_FEATURE (20)..(20): Xaa at position 20 is Aib
  MISC_FEATURE (25)..(25): Xaa at position 25 is alpha-methyl-Tyr
  MOD_RES (39)..(39): Ser at position 39 is amidated

SEQ ID NO: 391 - protein, 39 aa, Artificial Sequence; identical to SEQ ID NO: 380
  Synthetic Construct
  MISC_FEATURE (1)..(1): Xaa at position 1 is D-Tyr
  MISC_FEATURE (2)..(2): Xaa at position 2 is Aib
  MISC_FEATURE (13)..(13): Xaa at position 13 is alpha-methyl-Leu
  MOD_RES (17)..(17): Lys at position 17 is chemically modified by conjugation of the epsilon-amino group of the Lys side chain with (2-[2-(2-amino-ethoxy)-ethoxy]-acetyl)2-(gamma-Glu)-CO-(CH2)16-CO 2H
  MISC_FEATURE (20)..(20): Xaa at position 20 is Aib
  MISC_FEATURE (25)..(25): Xaa at position 25 is alpha-methyl-Tyr
  MOD_RES (39)..(39): Ser at position 39 is amidated

SEQ ID NO: 392 - protein, 39 aa, Artificial Sequence; identical to SEQ ID NO: 381
  Synthetic Construct
  MISC_FEATURE (1)..(1): Xaa at position 1 is D-Tyr
  MISC_FEATURE (2)..(2): Xaa at position 2 is Aib
  MISC_FEATURE (13)..(13): Xaa at position 13 is alpha-methyl-Leu
  MISC_FEATURE (16)..(16): Xaa at position 16 is Orn
  MOD_RES (17)..(17): Lys at position 17 is chemically modified by conjugation of the epsilon-amino group of the Lys side chain with (2-[2-(2-amino-ethoxy)-ethoxy]-acetyl)2-(gamma-Glu)-CO-(CH2)16-CO 2H
  MISC_FEATURE (20)..(20): Xaa at position 20 is Aib
  MISC_FEATURE (25)..(25): Xaa at position 25 is alpha-methyl-Tyr
  MOD_RES (39)..(39): Ser at position 39 is amidated

SEQ ID NO: 393 - protein, 39 aa, Artificial Sequence; identical to SEQ ID NO: 305
  Synthetic Construct
  MISC_FEATURE (1)..(1): Xaa at position 1 is D-Tyr
  MISC_FEATURE (2)..(2): Xaa at position 2 is Aib
  MISC_FEATURE (13)..(13): Xaa at position 13 is alpha-methyl-Leu
  MOD_RES (17)..(17): Lys at position 17 is chemically modified by conjugation of the epsilon-amino group of the Lys side chain with (2-[2-(2-amino-ethoxy)-ethoxy]-acetyl)-(gamma-Glu)-CO-(CH2)18-CO2 H
  MISC_FEATURE (20)..(20): Xaa at position 20 is Aib
  MOD_RES (39)..(39): Ser at position 39 is amidated

SEQ ID NO: 394 - protein, 39 aa, Artificial Sequence
  Synthetic Construct
  MISC_FEATURE (1)..(1): Xaa at position 1 is D-Tyr
  MISC_FEATURE (2)..(2): Xaa at position 2 is Aib
  MISC_FEATURE (13)..(13): Xaa at position 13 is alpha-methyl-Leu
  MOD_RES (17)..(17): Lys at position 17 is chemically modified by conjugation of the epsilon-amino group of the Lys side chain with (2-[2-(2-amino-ethoxy)-ethoxy]-acetyl)2-(gamma-Glu)-CO-(CH2)18-CO 2H
  MISC_FEATURE (20)..(20): Xaa at position 20 is Aib
  MISC_FEATURE (25)..(25): Xaa at position 25 is alpha-methyl-Tyr
  MOD_RES (39)..(39): Ser at position 39 is amidated
XXEGTFTSDYSIXLDKKAQXEFIEXLIEGGPSSGAPPPS

SEQ ID NO: 395 - protein, 39 aa, Artificial Sequence
  Synthetic Construct
  MISC_FEATURE (1)..(1): Xaa at position 1 is D-Tyr
  MISC_FEATURE (2)..(2): Xaa at position 2 is Aib
  MISC_FEATURE (13)..(13): Xaa at position 13 is alpha-methyl-Leu
  MISC_FEATURE (16)..(16): Xaa at position 16 is Orn
  MOD_RES (17)..(17): Lys at position 17 is chemically modified by conjugation of the epsilon-amino group of the Lys side chain with (2-[2-(2-amino-ethoxy)-ethoxy]-acetyl)2-(gamma-Glu)-CO-(CH2)18-CO 2H
  MISC_FEATURE (20)..(20): Xaa at position 20 is Aib
  MISC_FEATURE (25)..(25): Xaa at position 25 is alpha-methyl-Tyr
  MOD_RES (39)..(39): Ser at position 39 is amidated
XXEGTFTSDYSIXLDXKAQXEFIEXLIEGGPSSGAPPPS

SEQ ID NO: 396 - protein, 39 aa, Artificial Sequence
  Synthetic Construct
  MISC_FEATURE (1)..(1): Xaa at position 1 is D-Tyr
  MISC_FEATURE (2)..(2): Xaa at position 2 is Aib
  MISC_FEATURE (13)..(13): Xaa at position 13 is alpha-methyl-Leu
  MOD_RES (17)..(17): Lys at position 17 is chemically modified by conjugation of the epsilon-amino group of the Lys side chain with (2-[2-(2-amino-ethoxy)-ethoxy]-acetyl)2-(gamma-Glu)-CO-(CH2)18-CO 2H
  MISC_FEATURE (20)..(20): Xaa at position 20 is Aib
  MISC_FEATURE (25)..(25): Xaa at position 25 is alpha-methyl-Tyr
  MOD_RES (39)..(39): Ser at position 39 is amidated
XXEGTFTSDYSIXLDEKAQXAFIEXLIAGGPSSGAPPPS